European Patent Application EP 4 563 701 A1, published June 4, 2025. Title: ペプチド合成酵素ライブラリー構築法. Applicant: 国立大学法人神戸大学. Application JP. The sequence listing filed with the application follows.

SEQUENCE LISTING (65 sequences)

SEQ ID NO: 1 - DNA, 41 bp, synthetic construct
  misc_feature 1..41: note = primer 00-F
  source 1..41: mol_type = other DNA
cgacttggccgatgtggcccgggagacctgttttccaagag

SEQ ID NO: 2 - DNA, 48 bp, synthetic construct
  misc_feature 1..48: note = primer 00-R
  source 1..48: mol_type = other DNA
tttaggggccgccacggccgtcttgttaaactcatacaacaatttttg

SEQ ID NO: 3 - DNA, 38 bp, synthetic construct
  misc_feature 1..38: note = primer 01-F
  source 1..38: mol_type = other DNA
caagacggccgtggcggcccctaaagctttcaccctgc

SEQ ID NO: 4 - DNA, 50 bp, synthetic construct
  misc_feature 1..50: note = primer 01-R
  source 1..50: mol_type = other DNA
ttgagcggcctcaacggccgttttgttaaattcaaagactattttttgtt

SEQ ID NO: 5 - DNA, 46 bp, synthetic construct
  misc_feature 1..46: note = primer 02-F
  source 1..46: mol_type = other DNA
caaaacggccgttgaggccgctcaaaaagatattccttttcatcgc

SEQ ID NO: 6 - DNA, 48 bp, synthetic construct
  misc_feature 1..48: note = primer 02-R
  source 1..48: mol_type = other DNA
gttcacggccggacgggccgtttcgttaaacaattggataacctgttg

SEQ ID NO: 7 - DNA, 43 bp, synthetic construct
  misc_feature 1..43: note = primer 03-F
  source 1..43: mol_type = other DNA
cgaaacggcccgtccggccgtgaacaaaacgataccccaattg

SEQ ID NO: 8 - DNA, 43 bp, synthetic construct
  misc_feature 1..43: note = primer 03-R
  source 1..43: mol_type = other DNA
tctcggggccagggcggcctgccccattttttcaaggagtaac

SEQ ID NO: 9 - DNA, 43 bp, synthetic construct
  misc_feature 1..43: note = primer 04-F
  source 1..43: mol_type = other DNA
ggggcaggccgccctggccccgagaaatgaaaacatagtaagc

SEQ ID NO: 10 - DNA, 47 bp, synthetic construct
  misc_feature 1..47: note = primer 04-R
  source 1..47: mol_type = other DNA
ttcaggggccacactggccgtcctgttattttgagaaacgattttcc

SEQ ID NO: 11 - DNA, 34 bp, synthetic construct
  misc_feature 1..34: note = primer 05-F
  source 1..34: mol_type = other DNA
caggacggccagtgtggcccctgaagccccaacc

SEQ ID NO: 12 - DNA, 37 bp, synthetic construct
  misc_feature 1..37: note = primer 05-R
  source 1..37: mol_type = other DNA
tcttggggcctctatggccgtacgattgagctcgtgg

SEQ ID NO: 13 - DNA, 42 bp, synthetic construct
  misc_feature 1..42: note = primer 06-F
  source 1..42: mol_type = other DNA
tcgtacggccatagaggccccaagaaatgaaaccatcagcag

SEQ ID NO: 14 - DNA, 43 bp, synthetic construct
  misc_feature 1..43: note = primer 06-R
  source 1..43: mol_type = other DNA
ggtttcggccactggggcctgatctgtgatttctccaatcagc

SEQ ID NO: 15 - DNA, 41 bp, synthetic construct
  misc_feature 1..41: note = primer 07-F
  source 1..41: mol_type = other DNA
agatcaggccccagtggccgaaaccatccatgccatgtttg

SEQ ID NO: 16 - DNA, 47 bp, synthetic construct
  misc_feature 1..47: note = primer 07-R
  source 1..47: mol_type = other DNA
tgaataggccgtcacggccaacagatggcatgattcaatgaaatctc

SEQ ID NO: 17 - DNA, 47 bp, synthetic construct
  misc_feature 1..47: note = primer 08-F
  source 1..47: mol_type = other DNA
tctgttggccgtgacggcctattcaatgaatcaaacgctccactatg

SEQ ID NO: 18 - DNA, 42 bp, synthetic construct
  misc_feature 1..42: note = primer 08-R
  source 1..42: mol_type = other DNA
tccgtaggccttcgcggccccggtgttaaactcattaagcag

SEQ ID NO: 19 - DNA, 46 bp, synthetic construct
  misc_feature 1..46: note = primer 09-F
  source 1..46: mol_type = other DNA
caccggggccgcgaaggcctacggagttcaaacaatcagtcaattg

SEQ ID NO: 20 - DNA, 45 bp, synthetic construct
  misc_feature 1..45: note = primer 09-R
  source 1..45: mol_type = other DNA
ctttggggcctccgtggccgtattgttgaactgtgtgacaatctg

SEQ ID NO: 21 - DNA, 50 bp, synthetic construct
  misc_feature 1..50: note = primer 10-F
  source 1..50: mol_type = other DNA
caatacggccacggaggccccaaagaatcatacaattatcgatttatttc

SEQ ID NO: 22 - DNA, 49 bp, synthetic construct
  misc_feature 1..49: note = primer 10-R
  source 1..49: mol_type = other DNA
aagcttggccaagacggccatacaaaaagaaagacggacagagaatggc

SEQ ID NO: 23 - DNA, 50699 bp, synthetic construct
  misc_feature 1..50699: note = linked construct ppsW03
  source 1..50699: mol_type = other DNA
atgtggcccgggagacctgttttccaagagaaaacaggtttttttatgtctgtaataacgctttgtcgaaccttccaacaattagaagaatgatgcacaaaagaaaattagtccgattaaaaagtagtgtataagaccttatgtaaaacaatacttttatcactttatatccggaaatttgataaaaaaagaaacgaaaaataaagaaataatactatattcaaaaaaaatgttataaaaatttaatgttttttattgtactttaaaaaatatccgttaatatagtgcatatatggattatatagtcatataatttcttttattgtcatttttctgcttttttctacattttcttatcctcttattatgagaactggagggaatccgttgagcgaacatacttattctttaacccatgcccaaaggagagtgtggtttaccgaactgctggagccagataccagcatttgcaatcttacagcttgtgtgaaatttaaaggcaatattgagcttgatactctggagggagcactgaatcattccatctcccgcaacgacgccattagatttcagctgttagaaggagaagagcttgagcctcgattgcaccttactgaatataaatattatccacttagaataattgatttttcaaatgttgaaatgatagaaatagagcaatggattcaggatcaagcgagcattccatttaaactgttcaactcgcctctttttcaattttacctccttagaattgactctcatgaagtttggctatttgcgaaattccatcatatcataatggatggaatctctttaaatgtgatgggaaatcaaattatagatctttatcaaaaaatgaaaaagaaagatcctttacctgatcagccggaaccttcttacttgagctacatcgaaaaagagagtcaatatctacaatctccacggtttgcaaaggaccgtttattttggacgcaaacctttgagcacccgttggaataccactcgttagccgaccagacgtccttacaaaaacagagcacatctgcatccagagacaccatcattctttcacctgatctagagcaaacgattcgaatcttctgcgaagaacacaagatcaatatcatttccttatttatggcttcattttacatatgcatcagccgaatcacttctaaaaaagatcttgccattggcacctactatggcaacagaggttcaaaggctgaaaaagaaatgctcggcatgttcgttagttcccttccaatcagaataacggttgatcctgacacagattttctttcctttgtccgcacaataggcagggaacagctttctgttatgcgtcatcaacggtttccttataatttgcttgtaaatgaattaagaaatgaacagaaggatttacacaaccttatcggtatatctatgcagtatcagccacttcagtggcacaatgcagatgattttgactatgaaacagcgctttatttcagcggatacaccgcgaacgaactttcagttcaaatacaagaacggatagacaatggaaccattcaattaaatttcgactatcaaaataccttgttttctcttgaggatattaaacgaatacaatctcatctgcttaccatactggaaaacgcccttaaacatccgcacagctttataagagaattagatatgacgaatacaagagaaaagcaaaaattgttgtatgagtttaacaagacggccgtggcggcccctaaagctttcaccctgcatgggctgtttgagcgacaggcagctttcacaccggagcggctggccattcgcttttcaggcggttcgctgacatacgctgagcttgatatgtacgccagccggctggctgcgcaccttgcggcacgcggcgtcacaaacgaaagtatcgtcggtgtcctgtctgaacgctcacctgacatgctgatcgctgtccttgctgtattgaaggccggcggggcgtatttgccgcttgatcctgcgtatccaaaggagcggctgagctacatgctgaaagacagcggggcatcgctcttgctgacacagccgggatgctccgcaccaaacttttctggcgaaacgcttgaagtggacatgacatctcttgcgagcgaaaaagcagaaaaccatgagtttactcctgctgacggcggatctctcgcctatgtcatctatacatcgggctctaccgggcagccgaaaggagtggccgttgagcaccgtcaggctgtttcctttctgaccggcatgcagcaccagtttccgctttcggaagatgacattgtcatggtgaaaacctctttttcctttgatgcgtctgtgtggcagctgttttggtggtcgctttccggtgcttcggcgtatctgcttccgcccggctgggagaaagactccgcattgatcgtacaagccattcatcaggaaaacgtgacaacggctcattttattccggctatgctgaacagctttctcgatcaagcggaaatcgaaaggctgagtgacaggacaagcctaaagcgtgtattcgccggaggtgaaccgcttgcgccgcgtacggcagcccgttttgcttctgtattgccgcaggtatcattaatccatggttacgggccgacagaagcaacggtagacgcggcattttacgtattggatccagaacgggacagggatcgtttgcggattccgattgggaagcccgtacctggtgcgcgtttgtatgttttagatccgcatttagccgtacagccttccggtgtcgccggcgaactgtacattgccggagcgggtgttgccagaggttatttgaatcggccggcattaacggaggagcgttttcttgaagacccgttttacccgggggaacgcatgtacaaaaccggggatgtggcgcgctggctccctgacgggaatgttgaattcctcgggcgcacggatgatcaggtaaaaatccgcggctaccggattgagccgggagaaattgaagcggcactaagaagcatagaaggcgtaagagaggcggctgttaccgtacggacagacagcggggagccggaattatgcgcttatgtagaagggctccaaagaaacgaagtgcgtgcacagcttgagagactgttgccgggctacatggtcccagcctatatgatagagatggaacagtggccggttacgccaagcggaaagctcgaccgaaacgccctgccagctcctggcggagcggcagatgcggagacctacacggcgccgagaaacgtgactgagatgaagctttctcagctgtgggaggacgtgctgaaaaatggccctgtcgggattcacgacaacttttttgaccgcgggggacattccttaaaagcaacggcgcttgtctcacggatcgccaaagaattcgatgtacaggtgccgctaaaagatgtgtttgcccatccgacagtagaaggactggctaccgttatccgtgaaggaacggacagtccatatgaagcgattaagcccgctgaaaaacaggaaacctatccggtttcctctgcccaaaagcggatttatgtccttcagcagctggaggacggagggacaggctacaatatgccggctgtgttagagctcgaagggaagctcaaccctgaaaggatggagagagctttcaaagagctgatcaagcgccacgagtcgcttcggacctccttcgaacaggacgcaggaggcgatccggtgcagcgcatccatgacgaggtgccgtttacgttacagactacagttctcggcgaacgaaccgaacaggaggccgcagccgcatttatcaaaccgtttgatctcagccaagcgccgctgttccgtgcccaaatcgtaaagatatcagatgagcggcacctgttgctggttgatatgcatcacatcatttcagacggtgtttccgtcaacattctgattcgggaattcggcgagctgtacaataatcggaatcttccggcactgcgcattcaatataaagattatgccgtatggcgagaaggattcaaaacaggagacgcgtacaaaacgcaagaggcgtactggctgaagcagctcgagggcgagctgcctgtgctggatcttccggctgatcatgcccgcccgccggtgcgaagcttcgcgggtgacaaggtctcatttacgctggatcaagaggttgcatcaggccttcacaagctggcacgtgaaaacggaagcacactgtacatggtgcttcttgcggcttacaccgcgttcttgtcacgcttaagcggacaggaagatatcatcgtcggctcgccaattgccggccggccgcacaaggatcttgagccgatactcggcatgtttgtgaacacgctggcgcttcggacgcgcccggagggcgggaagccattcgtacagtatttgcaggaagtgcgtgagacagcattggaagcctttgagcaccaggattacccgttcgaagagcttgtcgataagcttgaattgacacgagatatgagccggaacccagtgtttgatgcgatgtttatccttcaaaatgtggaaaaacaagacatagatctgagagaaataaaagtccggcctgccaatttcgcacatcacatttccttatttgatatcacattaatagctacggaaataagtggatctatttgctgcgaaatggaatttagtacagaagtattcctgaaagctacgattgaacgctgggctgatcattttatcgaatttctgcatgaggcactttcaactcctgaaacaagccttgcacaaataaacatacttagtgataaagaaaaacaaaaaatagtctttgaatttaacaaaacggccgttgaggccgctcaaaaagatattccttttcatcgcatatttgaagcgaaagctgaagaaaatccagaacatatagctgttattgataacgaaacagagattagctatcgccttctaaatgaaagagccaatcgtctggcacgaacattgcaaaacagaaaaggaccgaagccaactgtggctgttttagccaagcggtccatcgatgcaattgttggagttctggcagtgatgaaagctggcggagtgtatatcccaatcgatgcacattatccaaaagctcgtattgaatacattcttcgtgatagcggggcagatattcttcttttacagagagagttgaagcatttgatttcgaactcgcctgaatctgagatgtctcacatcttccttgacgatgagggctcttttgaagaaagtaactgcaaccttaacttatctcctgctcctgaagagccggtatatatcatttatacgtcaggaacgacgggtgcgcctaaaggtgttattgtcacctatcagaactttactcatgctgctcttgcttggcgtcaaatttatgaactggatcggaagcctgtcagactgcttcaaatcgcgagcttttcattcgatgtcttctcaggagatttggcgagaacattgaccaacggcgggactctaatcgtttgcccagatgaaacacggctggaacctgctgaaatatataaaatcattaaatctcagagaatcacggtgatggagtcgacaccggctctcattatcccggtgatggagtatgtataccgtaaccagttcaagcttcctgacttagacatactgattcttggttccgacatggtgaaagctcaagatttcaaaacattgacagatcgctttggccaaagcatgcgcatcattaatagctatggtgtcacagaggcaaccattgattcgagtttctatgaaaccagtatgggtggagagtgtacgggagataacgtaccaatcggcagcccgctgccgaatgtacacatgtacgtactcagccagactgatcaaattcagccgatcggtgttgccggcgagctgtgcatcggcggggcaggtgttgcgaaaggctatcatcataaacctgacttaacgcaaatgaaatttacagaaaatccatttgtctctggagaaaggctgtacagaaccggtgatcgagcatgctggcttccaaacggaacgatccggcttcttggccgaatggattatcaagtaaagataaatggatacagaattgaaacagaagaaattgaaagtgttctgcttcaaacggggcttgtcagagaagctgctgttgccgttcagcatgataaaaatggacaggctggtttggcagcatatattgtgccttcagacgtcaatacgaatgctctccgtgctgctttaacaaaggaactgccagcgtatatgattcctgcatatctgattcctttagtaaacatgccgctgaccctaaacggaaagctggacagaaatgccttgccggctccaaataatgtgttatcgcgtccatataccgcaccagttaacgacttacaaaaaacgatggcgtatatatgggaagatgtactgagcatgtcacgagtcggcattcacgattccttttttgagcttggcggagactcaattaaagcattacaagtggcagcacgtctggcagctgaaggctggagcatgacaatacgcgacttattccgttattcaacgattcaggaactatgcggacatatcacaccattggcatctcaagcggaccagggacctgcggaaggtgaagctgaactcaccccgattcagcgaagatttttcggacaggtacatgcttttcactatcattacaaccagtccgtcatgcttttcagtgaaaaaggattcaatgctaacgcgcttcatctagcgctgcgtaaaataaccgagcatcatgatgccattcgcatgattttccaacgtgaccaaaacggccatgtcattcagtttaatcgcggaatcaatcacaaggatcatgaactgtttggcctttatatttcagattggacaaaagcatcgctggaaagggctcatcttgatgaaaaacttgccgctgaggaaaccgtcattcaaagcaaaatgaatgtagaaaaagggcccttactgcaagcaggtttgtttaaaacggcagaaggggatcatttgctgattgcacttcatcatcttgtgatagatggcgtttcttggagaattctgcttgaggatttagctgcagcatatcaacaggctttagaaaagaaagaaatccaattaccgccaaaaacggattcttatttatcctacgccgatggtcttacccaaatagctgaaagtaaacaattgctttcagagaaaacgtattggcaaacgattttagacgctcacactgcttttcttcctaaggacatagaaaatgtgccagacaaactccaaatgaacagcgacgcagcagcgtttgtactatccggggactggactgaaaaattgctgtttgaaacccagcaagcctatggtactgatgccaacgaacttttgcttacggctttaggaatggcgctttctgaatggactgggcatgaccaaatcgtgatcagcactgagggacacggtagagaagggcatgtgccaaacattgatatttcaaggacagttggatggtttacctccatttatcctattctgctagacatgggtattcccgagcctttcgaggatcagctcgcataccgaattaagacgacaaaagatatgctgagaagagtaccgaacaaaggaactggatacggattgttaacacacataggagaactgcggcataaagagcctgaggtcagctttaattatctcggtcaatttagcgaagagaaggaagttgaaacgtttcaattatcatattaccagccccgttacgaaatagcgggtgagagagaacgagagtatgagctggacatcaatgctctcattacggacggacggcttcacgtaaaagcggtatacacccaagtgttcagcaaacactcaattgagtgctttatggatcgttttcacaggcatcttatcgagacgattgagcattgttcgcagaaaaaagcacgcgaaaaaacattgagcgatttcagcaataaagaattaacgttgtctgcattatctagcatcgaagatctcgtgaaagatctttaacttttgaaaaggtgtgtggaattgatggcacaatcggcacaaattcaagatatttatccgttatcgcacatgcaggaaggaatgctgtttcattcactaatggatttcagctcgaaagcatatatcgaacagacctcgtttacgatcacagggaatctatgcgtcgactcgtttcaaaagagcttaaaccttcttgtttctagatatgatattttcagaacgattttcattaaagaagtaccagatcttacaggtccgcagcaggtagttctatcaaaccgtgaattgacagtatatagagaagatatttctcgcctggctgatcaagaacagcagacgctgattgatgcttttatgactaaggatcgggaaaaaggatttgatttgcaaaaagatcctttaatgcgtcttgccctttttgatagaggagacagccaatatacatgtgtctggacacatcaccatatcatcatggatgggtggtgtctcggcattattcttaaagagtttttcagcatgtatgattcgctcaaaaataactcacctgtacagcttggcagcacggtgccgtacagccgttatattgaatggctcggagaacaagatcaagaagagactgctgcctactggagcgaatatttgaaggagtacggcaatactgcttctattccccgaataaagcgccgcacggcagacgggaattataaagccgaccaggtcagcttttcattagcgccggatatggttgagaaactgacagaggctgcccaaaactggggagtgacattaaacacgctgtttatgagtatttggggcgtgctgctccatcgatataatgctgcagatgatgccgtttttggctccgtcatttcgggacgcccgtcagcgattgacgggattgaatcaatggtcggtttgtttatcaatactgttccagtgcgaatccgatctgcggaaggcataacattttcttcgctggtcaaagccgtgcaggaggatattttatcatctgaacagcatgggtattatccgctttatgagattcaaaaccatagtccattgaagcaagggttgatcgatcatatttttgtttttgaaaattaccctgtacagcttcatcaggcattaagcgtggagagtgaaaatgacgaaggcgctctgaagctgagtgacatttcaatgtcggaacaaaccaattacgactttaatatcgttatcgttccgggagaatcattttatatcaaattcagctacaacgcagacgtttacgagcgggaggagatgctgaggattcaggggcatctaaagcaagcactggattgcattttgacaaatcccgatgttgccgtcagtgacatcaatatcgtgccgccggaggagcaacaggttatccaattgtttaacgaaacggcccgtccggccgtgaacaaaacgataccccaattgtttgaggaacaagctcacaaaacacctgaagctgctgcattgaaaatgggaaacgagtgctggacctatcgccagttacaagtaagagccaatcagattgcgcacgccctgatagaaaaaggcgttggatctggggatatcgttgctgtaatgatgggccggtcaatggaaatgcctgcagctctgcttgggatttggaaagcaggcggcgcttatatgccgcttgatccacattttccagcagaacgtctttcttttcttctgaaggacagtcaagcggctcaattgctgatagaagaagaccttatttccttgatccctccgtcctatgaaggaaatacgataacgatagaacatacagaaagttaccaaacagaagcgccaaatatgccgccaggtgatctagcctacttgatctatacgtcgggaacgacggggcgccctaaaggggttttagttgatcatcacggtattgccaatacattgcaatggagacgggaagagtatagcatgaccgaacaggatatatccctccatttgttttcgtacgtgtttgacggctgtgtaacgagcttatttaccccgcttttatctggtgcgtgcgtactgctgacaacagatgacgaagcgaaggatgtgctggcccttaagcgaaaaatagcccgttataaggtcagccacatgatcattgttccttccctgtacagggtgttattggaagtgatgactgctgacgatgcaaaaagtcttcgtattgtgacatttgcgggtgaagcggtcacgcctgatctgcttgagttgaatcaaataatttgtccttctgctgaactggcaaatgaatacgggcccacagaaaacagtgtggcaacaacaatattgcggcatctgaataaaaaagagaggatcacgatcggacacccgatcagaaacacaaaagtatttgttttgcacggaaatcaaatgcagccgatcggcgcggcgggtgaactgtgtatttccggcgcgggtcttgcgagaggatactacaaacagcaagagctgacacagaaagcattctccgatcatccattccttgaaggggagcgtttataccgaacaggtgatgcaggccgctttttgcctgatggaacgattgaatatattggacgttttgatgatcaagtgaaaattaggggttatcgtattgaactgagagagattgaaacagttcttcgacaagcaccgggggtaaaagaagcagcggtactggcccgtgatgtttctgctgaggaaaaggagctcgttgcttatatcgttccggaaaagggaaacagcctcccagatttgtatcagcatcttgccgggacattgccgtcctatatgatcccagcaagtattatcaacatcagccagatgccattaacatccagcggcaagcttgacaggtttgcgcttcctgaaccagaaaacaatacgagtgtcacatatatggcgccccgaaccttaatcgaagctgatctcgcacatatttgggaagatgtgctgaataaacagcacatcggcattcgtgatgatttctttcagttaggcggacagtccttaaaagcggccgcactggtatcaagaatacataaaaagcttaatgtcgagctgccgctcagtgaggtgttttcttatccgacggttgaaagcatggcggtcaaattgatgagcttaaaagaacacgcttttacacagattgaacctgcggatcaaagagatgtctatccgctgtctttctcgcaaaaacgattatatgctcttcatcagctggcagatgacagcacaggctacaacatgccagctgtacttgaattacgcggaaatctgaatcgccagcggttgagaagcgttctcacagaacttgtgaatcggcatgaagcattacggactgtttttgtgcttgacagagacgagcctgtgcagatcatttatccagagatggcttttgatctaaaagagcttgaaatggaatcagaacaaatgcttgagtctgcaatcgagacctttatcaaaccgttttatctatcatccggtccgctttttagagcatgtgtcattacaatgggcaataatcgcggctttttgctgctcgatatgcaccatattattgccgacggtgtctcgatgagcactcttgtccaagaatttactgacttatattgcggaaaagagttgccagctttaaacctgcattataaggattttgctgtttggcagcaagagaagcacccgaaagagctatacaaaaaacaggaggcctactggctcggtcagcttggcgggagtcttcctacactagaattaccgcttgataaaacaaggccgcgtctccctgatttcaggggtggaacaattgaagtcaacattgataaagacatggctgatgaactgcaccgtttaatggctgaaacgggaacaacattgtatatgattcttctggctgtctattctattttgttatctaagctaagcgggcaagaggatattgttgtcggttcgcctgctgccggaagaccgcacgctgatctggagcgcgtcatcggaatgttcgtcaatacattggcgatgcgcagcaagcccgagggccacaaaacgttcagctcctatttgcatgacattcgccacctggctctgaccgcttacgagcatcaggattatccttttgaggagctggcagataagctcgatacaaatcgagaggtaaatcgcaacccgctgttcgatgcgatgcttgtgcttcaaagcagtgaagatttccggttcgaagtgcctggtctgtcgatttcgtctgtcactcctaaacatgatatatctaaattcgatttaacattacatgctgaggagcatctgagtggaatacgctgccgttttgaatacagcactgctctttttgaagaagaaaccattacgcagtgggcatcctattttattgaattggtaaaaggggtaacggcggatactgagatgagaatttcgaacatgcaattgcttcctgctgcagagcgtaggttactccttgaaaaaatggggcaggccgccctggccccgagaaatgaaaacatagtaagcttatttgaaaagcaagtagctcagtatccggagcatatcgcagtggtgtgcggccattctcagcttacgtatcgagacctgaatgaaaaagccgagcgggcagctgctatgctgatcaaacaaggggtcagaactggcgatatcgtcggtctgatgctcgatcggtcacctgatatgatcattggcgttttatcgattttaaaagctggcggggcctatttgccgattgatcctgaatatcccaaggagcgtattagctttatgctcaatgacagcggagcaaaactgctgctgacagagcgcggtctaaacaaacctgcagactacaccgggcatattttgtatatcgatgaatgtgaaaacaactcaattccggctgatgtaaacattgaagaaatagtaacggatcagcccgcatacgtgatatacacatctggaacgactggtcagccaaagggagtcattgtcgagcaccgcaatgtgatcagtctcttgaagcatcaaaacctgccttttgaatttaaccatgaagacgtctggacgttatttcattcttattgctttgatttctctgtatgggagatgttcggtgcgttattgaacggaagtacattagtcgtggtctctaaagaaacagcccgtgacccccaagcattccgattattgttaaaaaaagagcgcgtcactgtactcaatcagaccccgactgctttttacggcttgatgcttgaagaccaaaatcatacagatcatttaaacatccgctatgtgatttttggcggcgaagccttacagcccggattgcttcaaagctggaatgaaaaatatcctcatactgatttgattaatatgtacggtattacagaaacaacggtccatgtaacattcaaaaaattgtccgcagcagacattgcaaaaaataaaagcaatatcggccggcctctttctactctgcaggctcatgtgatggatgcccatatgaacctgcagccgaccggagttccaggggagctgtatataggcggcgaaggtgtggcacggggatatctcaacagagatgagctgaccgctgaccgttttgtatccaatccttatcttccgggagacagattataccgaacaggagatcttgctaagcgcctgtcaaatggcgagctggaatacttaggccgcattgatgagcaggtgaaagtcagagggcaccgtattgagttaggcgaaatccaagcggcacttcttcagtatccaatgattaaagaggcggctgtcattaccagagcagacgagcaagggcaaacagctatatatgcatatatggtgataaaagatcaacaggctgcgaatatatcagacatccgaacttacctaaaaaacgccttgcctgactttatgctgcctgcccgtatgatacaaattgacagcatcccggtgactgttaatggaaagctcgatcagaaagccctgccagagcctgaaaaacaagcttatacagctgatgatatcagtcctagaaatgagattgaaacggtgatggctgaaatttgggaagagcttcttaatgtagatgagctgggtgtaagcgccaatttctttaagcttggcggagactctattaaagcgctgcaggtttgtgccagactgaagcagcgcggatttgaaacgacagtacgtgagatgtttgaacatcagactcttggtgaactgtccgcccgggttcgaaaagacgtacgcgccattgaccaaggcccggtcgaaggcgagattacttggacacctatccagcagtggtttttctcgcaatctctggaaagccatcattttaaccaatccgttatgatctaccgggctgaacgatttgatgaggctgcgcttagaaaagtactaaaaagccttgtgactcatcatgatgcactgagaatcgtatgccggcatgaagatggcaggcaagtgcagataaacagagggatagatctttcagatgaggagctatatgcacttgaactgtttgatgtaaaggatagcctaacagaagcccggaacacgattgaggaagcagccagccggatgcaagaacatattcgtttggaaaccggccccttacttcacgctggattgtttagaaccgagaatggtgaccatttatttctaacgattcatcacttagttgttgatgcggtttcttggcgcattttgtttgaggatttttcaacagcttacaaacaggcagtctcaggagaatctattaaactgccgcaaaaaacagattcatatttaacgtattcacaaagaatagctgactactctataagccgccaggtgcagcgcgaagcagcgtactgggatgagtgcgagaaccgtcacatccagcctattccaaaagacaatgacgcagcatctaacacattcaaagatacagaagtgattgattttgagctatctcgccatcacacagaattactattaacggctgcacataaagcttacagcacggagatgaatgatatccttctgacagctttaggtcttgctttgcagaaatggacgggaaataaccaatttaaaatcagcatggagggccatggaagggaatcatatcttgaggacatcgatattagcagaactgttggctggttcacctccatttatcctgtgtggcttgatatgagagattccgatcataaggacaaagaagagcggctgggccaccttattaaacagacaaaagatatgctgcaccgtataccgcataaaggcgcgggctacggcgtgctgaaatatatcagcaaaagatggggctctcagaaaaacagcccagaaatcagctttaattatttaggccagtttgatcaggatattcaatcaaatgcctttgaggtgtctgacatcaagccaggaaatgagatcagcccgaactgggagcgtccttatgcactggatatcagcggcgccgtttcttcggggtgcctgaacatgcacatcatctataacaggtttcaatttgaggaaaaaacaatccaaacattttccaggcattttaaacagactctggaaaacatcattgagcattgtaccggcaaagaaaaccaagagtggagcgcatctgatttcactgatgaagacttaacgcttgatgaattgagtgagatcatgggagccgtcaacaaactataggagaggagattcactgatgccgcagcaacctgaaatacaggatatataccctttgtcatttatgcaggaagggatgctttttcactcactgtatgatgaacagtcgagagcttattttgaacaggcttcttttacgatccatggacagcttgacttggagcgtttccaaaaaagtatggatgctgtttttgacaggtacgatatctttcgaacagcattcatctataaaaatgtagccaaacctcgtcaagtcgtgctcaagcaacgtcattgccctattcatattgaagatatttcccatctcaatgaaagggataaagaacattgtaccgaggcattcaaagagcaggacaaatccaaaggctttgatctccaaacggatgtactgatgagaatatctattttaaaatgggcgcctgatcattatgtctgtatctggagccaccatcatattttaatggatggctggtgtttaggcatcgtcattaaagactttctccatatttatcaagcgctgggtaaaggccagcttcctgatttgcctcccgtacagccgtacgggacgtatattaaatggctgatgcagcaagatcgtgaagaagcagctgagtactggaaaaagaggcttcagcatttcgaaaaatctacacccctgccgaaaagaacagatcaaattccgaatgggacactacagcagatcacgtttgccattcccgaaaaagaaaccgccgaattacagaaaatcgcagcagcttctggtgcgacactaaacactgttttccaagctttatgggggattatgcttcaaaaggtcaatcgcagcagcgatgctgtgttcggttcagttatatcaggcagaccttctgagctaaaagatgtggaaaacatggtcgggctttttatcaataccattcctattcgagcccaaagtgattctctgtctttttctgacctagtcaggagaatgcaaaaggacatgaatgaggcagaagcctatagttactttcccttgtatgatattcaggcgcagagtgctctaaagcaagagttgatcgatcatattatcgtctttgaaaatacacctacccagcaagagatcgaagagctgaatcaagcggggtcatttgatttctccgtcaaagattttgagatggaagaggtgaccaattatagttgcagtgtcaaagtgatcccaggccgtaccttgtacgttcggattcattttcagaccagcgcttatcaaccaagcatgatgtccgaaataaaagattatttgctgcacatggtctctgacgtcatctctgatccatctcttcctgtgtcaaagatgacgttgctagatgaggacaaaacacggaaaatcgtttctcaaaataacaggacggccagtgtggcccctgaagccccaaccctgcatgggctgtttgaacgacaggcggcagtcacaccggagcggctggccattcgcttttcaggcggttcgctgacatacgctgagcttgatatgtacgccagccggctggctgcgcaccttgcggcacgcggcgtcacaaacgaaagtatcgtcggtgtcctgtctgaacgctcacctgacatgctgatcgctgtccttgctgtattgaaggccggaggggcgtatttgccgcttgatcctgcgtatccaaaggagcggctgagctacatgctgaaagacagcggggcatcgctcttgctgacacagccgggatgctccgcaccaaacttttctggcgaaacgcttgaagtggacatgacatctcttgagtgtgaagaagtaaaacgtcatgtgtctgcttctgttagcgacggatctctcgcctatgtcatctatacatcgggctctaccgggcagccgaaaggagtggccgttgagcaccgccaggctgtttcctttctgaccggcatgcagcaccagtttcggctttcggaagatgacattgtcatggtgaaaacctctttttcctttgatgcgtctgtgtggcagctgttttggtgggctctttccggtgcttcggcgtatctgcttccgcccggctgggaaaaagactccgcattgatcgtacaagccattcatcaggaaaacgtgacaacggctcattttattccggctatgctgaacagctttctcgatcaagcggaaatcgaaaggctgagtgacaggacaagcctaaagcgtgtattcgccggaggtgaaccgcttgcgccgcgtacggcagcccgttttgcttctgtattgccgcaggtatcattaatccatggctacgggccgacagaagccacggtagacgcggcattttacgtgttagatccagaacgggacagagaccgtttgcggattccgattgggaagcccgtacctggtgcgcgtttgtatgttttagatccgcatttagccgtacagccttccggtgtcgccggcgaactatacattgccggagcgggtgttgccagaggttatttgaatcggccggcattaacggaggagcgttttcttgaagacccgttttacctgggggaacgcatgtacaaaaccggggatgtggcgcgctggctccctgacgggaatgttgaattcctcgggcgcacggatgatcaggtgaaaatccgcggctaccggattgagccgggagagattgaagcggcactaagaagcatagaaggcgtaagggaggcggccgttaccgtacggacagacagcggcgagccggaattatgcgcttatgtagaagggctccaaagaaacgaagtgcgtgcacagcttcagagactgttgccgggctacatggtcccagcctatatgatagaaatggaacagtggccggttacaccaagcggaaagctcgaccgaaacgccctgccagctcctggcggagcggcagatgcggagacctacacggcgccgagaaacgtgactgagatgaagctttctcagctgtgggaggacgtgctgaaaaatggccctgtcgggattcacgacaacttttttgaccgcgggggacattccttaaaagcaacggcgcttgtctcacggatcgccaaagaattcgatgtacaggtgccgctaaaagatgtgtttgcccatccgacggtagaaggactggctaccgttatccgtgaaggaacggacagtccatatgaagcgattaagcccgctgaaaaacaggaaacctatccggtttcctctgcccaaaagcggatttatgtccttcagcagctggaggacggagggacaggctacaatatgccggctgtgttagagctcgaagggaagctcaaccttgaaaggatggacagagctttcaaagagctgatcaagcgccacgagtcgcttcggaccgccttcgaacaggacgcaggaggcgacccggtgcagcgcatccatgacgaggtgccgtttacgttacagactacagttctcggcgcacgaaccgaagaggaggccgcagccgcatttatcaaaccgtttgatctcagccaagcgccgctgttccgtgcccaaatcgtaaaggtatcagatgagcggcacctgttgctggttgatatgcatcacatcatttcagacggtgtttccgtcaacattctgattcgggaattcggcgaactgtacaataatcggaagcttccggcactgcgcattcaatataaagattatgccgtatggcaagaaggattcaaaacaggagacgcgtacaaaacgcagggggcgtactggctgaagcagctcgagggcgagctgcctgtgctggatcttccggctgatcatgcccgcccgccgatgcgaagcttcgcgggtgacaaggtctcatttacgctggatcaagaggttacatcaggcctttacaagctggcacgagaaaacggaagcacactgtacatggtgctccttgcagcttacaccgcgttcttgtcacgcttaagcggacaggaagatatcatcgtcggctcgccaattgccggccggccgcacaaggatcttgagccgatactcggcatgtttgtgaacacgctggcgcttcggacgcgcccggagggcgggaagccgtttgtacagtacttgcaggaagtgcgcgagacagcaatggaagcctttgagcaccaagattacccgttcgaagagcttgttgataagcttgaattgacacgagatatgagcagaaatccgctgtttgacgtaatgtttgttcttcaaaatatggatcaggaatcgttggagctggatgaactttgtctcaaacctgcagcaaacaatgggcatcaaacgtccaaatttgatttaaccctatatgcccaggaacagccccgcggtttgctgacgttccaaatggagtttagtactgacttatataagaaaaaaacgatagaaaagtggcttcaatacttcaacaatatgttactctccatcatcaaagacaacaaagccgctctcggaacaataaatatcctgaatgaggatgaggcccattaccttatccacgagctcaatcgtacggccatagaggccccaagaaatgaaaccatcagcagactctttgaaatgcaggcagaacaaacacctaatgctgtagcaattgtcagcgacacccaagtattcacttacgaggacctgaacagctgggcaaatcaaattgcctcagttctacagataaagggcgtagggcctgatagtgttgtagccttgttgacaggcagaacaccagaactcattgcaggaatgctgggcattctaaaagccgggggagcctatctgcctatcgattctaatctgcctgttgaacgcatagcttatatgctgtctgacagcagggcagcattactccttcaatctgaaaaaacagaaaaacggctattaggcattgaatgtgaacaaatcataatcgaagatattcaaaagcaaggagaggcgaagaacgttgaatcttcagcagggccccattcacttgcatatatcatttatacctctggatcaaccggtaaaccaaagggtgtcatgattgagcagcgaagtgtaattcgtcttgttaaaaacagcaattatattacatttacacctgaagaccgccttctgatgacatcatcaatcggtttcgacgttgggtcatttgaaattttcggaccgctgctaaatggtgccgctttgcatctgtccgatcaacaaacatttctcgattcccatcagcttaagaggtacatagaacatcaaggaatcacaacgatttggctgacatcttctctattcaatcatttgacagagcaaaatgaacaaacattttcacagctgaaacatttgattattggcggagaagctttgtcgccgagccacgtcaatcgaatcagaaatgtctgccctgaagtatctatatggaatggatatggccctaccgaaaatacaactttttcgacatgccttcacattcaaaaaacatatgaactttccattccgatcgggcggccggttggtaattccaccgcttttatcttaaatcaatggggagtgctgcagccggtcggagctgtcggtgaactttgtgtcggcggagatggcgtcgccagaggatatttgggccgtcctgatttaacgaaagagaaatttgtcccacatccatttgcacctggcgatcgactgtatcgcacaggtgatctggcgcgctggctttccgatggcacaattgagtacgttggccgtattgatgatcaagtaaaagtcagaggctatcgggtggagctgggtgaaatcgaaacagcacttcgtcaaatagacggggtcaaagaagccgcagtgttagcacgtacagcccagaccgggagcaaagagctgtttggctatatcagcgtaaaagcaggcacgaatgctgaacaagtgcgttctcttctcgcgcgttcgctgccaaactatatgatcccggcgtatatcattgaaatggagactcttccgctcacatcaaacggcaaattgaaccggaaagcactgcctgaaccagatgtcgcatctaaacaaacatacatcccgccacgcaacgaacttgaagagcagctggcattgatctggcaggaggttctaggcatccagaggatcggaatagaggattcgttttttgaattgggcggagattcaatcaaagcccttcaagtttctgcacgccttgggcgctatggactaagcttgcaggtaagtgatttattccgtcatccaaagataaaggacttatcaccatttatccgtaagtcagagagaatcatagagcaaggacccattcagggtgacgttccttggacgcctgttcagcaatggtttttttcacaagatattgaagaaagacaccatttcaatcagtctgtcatgctattccattctggacgtttgtctgaaaacgcccttagaccagccttgaaaaaactggcggagcatcatgatgcgcttcggatggtttatcgcaacgatgacaggcgatggattcaaatcaaccaaggcattcatgagtcacagctatacagcttaagaatctctgatctttcacagtcagaaagcggctgggagacgaaaatcaaacaagaagttgccgatcttcagcaaagcatcaatttgcaggaaggaccattgttgcacgccgctttgtttaaaacactgaccggagattacttgttccttgcgatccatcaccttgtcgttgatggtgtctcatggcggattttgctggaggatttgtcagccggatatcaacaagctgctgcaggccagacgatccagcttccgcctaaaacggattcctaccaggaatacgcaagacgcatacaggaatatgcccaaagcagtaagctgattcgcgaagaggcgtattggcgaagtgtagaagaacagcaagccgcagaactgccctatgaaataccgcatcatgtgaacatcgacttcagcaaaagggactcattaagcttttcactgactgaagcagacaccgccgtcttgctgcaaaacgtcaatcacgcctatggcacagatacacaagatattctgttaaccgcagcatccttggcgatttgtgaatggacaggaggaagcaagctccgtatcgctatggaaggacacgggagagaacacattctgccagagttagatataagcaggacggtcggctggtttacatccatgtacccggccctcataagctttgaaaatcatagggatgagctcggaacctcagtaaaaaccgttaaagatacactgggccggataccaaacaaaggggtaggttacggtatgctgaaataccttacacaccctgaaaataaaagcattacgttttcaaaaacacctgaaatcagctttaactatttgggccagttcaacgacatcgaaagacaggacaccttccgcccatcaagccttggtagcggaaaggatatcactcatacatggaagcgcgagcaaatcatcgagatgagtgcaatggcagcagacaaaaagctccatttcaatcttagttatccgccagcccgctttcacagaaacacaatggaacagcttattaacaggattgaacactttttgctggacattatgaaacactgcgccggtcaacagaaagcagaaaagacactgagcgatttcagcagtcaatcattaacggcagaggacttggacagcatatccagcttggtggaagaattgtagaaaatcgtgacaggagacatgaacatgacaaaagcgaattcaattcaggatatttatccgctgtcttacatgcaggaagggatgcttttccattccctcctgcaaaaagattcacaggcgtatgttgagcaagcttcttttacaatagaaggaaaagtcaacccgcagttttttcaaaacagcatcaacgctcttgtagaaagacatgatattttcagaacgatttttatcagccaaaatgtttcctccccccagcaggttgttctgagagaacgaaatgtcatcgtactggaagaagacattactcatttaaacgaggcggagcaatcacagtttatcgagcaatggaaagaaaaggaccgggaccgggggtttcatttgcaaaaggatgtgctcatgcgcatcgctctgattcaaacaggagagagccagtactcttgcatttggacctttcatcatatcatgatggacggttggtgcctcagcattgtgctaaaggagtttctgcatatttacgcatcttatgtaaatgcatccccaataacattggagccggtccagccatacggaaagtatatcaaatggctgatggagcaagacaaagagcaggcggtttcttattgggatcattatctttccggccacgaacagcaaaccgtgctcccgaagcagaaaaaaacaaagggaaaaagcaggcaggaacacgttacattttcattctctaaggaagaaagcagcaggctttcagagcttgctgctagagaagaagtgacactcagtacgatttttcataccatttggggcattctgctgcaaaaatataataataacgatgacgccgtattcggttctgtcatttcaggaagacccgcagaaatcgaaggcattgaacatatggtaggtcttttcattaatacgatgccggttcgggtgcagggggcaaaaacgccttttcttcaacttataaaagatatgcaaaaagaccgtcttgccgctgaagcgtacagctaccaccctttatatgagattcaatcccgctcagctgttaagcaagggctgattgatcatattctcgtatttgaaaactatccggtgcagcaagagattcaaatgctgaacaaacaggaacatgcttctgatctttttcagattcataatttcactgtcgcagatgaaaccaactacagcttttatcttatggtggcgccaggggaagaaattcatatcaaaatgaactatgatgcggagcagcacgatcggtcttttgtgctctctgtcaaagagcatcttctgaatgctgtatcacaaatcttaaataatccgaatcttccacctgaagaaatcgatatcacgacagatactgaaaagcggcagctgattggagaaatcacagatcaggccccagtggccgaaaccatccatgccatgtttgaaaagcaagcggaaaagacaccagatgctcatgctgtaattgatcaagcctgctcattaacatacagagaactgaataaagcggctaacagattggcacggcatttacgaatgaaaggcgttgtgagacaggaacccgttgcgattatgatggaacgctcagcggcgtttatcacaggtgttcttggtatcttgaaagcaggcggcgccattgttccggttgatccgcattaccctgctgacagaatccgttatattctgcatgattgcggctgttcgcatgttgtttcacaagcgcatcttccctcatcgttagaagacaattacattatcactcatccagaagatatcgaaagcaaagtagacggcagtaacataaagtcagtcaacaatgctgacgatctgctgtatatgatttatacatcaggcacaacaggtaaaccaaagggtgttcaatttgagcatcgaaacatggctaacttgctgaagttcgaatatactcactccggcattgactttgaagcagatgttctgcaatttgcgacgccttccttcgacgtctgctatcaagaaatattttctgcgcttctgaaaggcggcacactccacatcgtgccagaagccataaaaagagatgtgcctcagctgtttgcatttataaacaagcatcagacgaatattgtgtttctcccaactgcttttatcaaaatgattttcagcgagcgagaacttgcgaactcgtttcctgatggcgtcaaacacctgatcgcagccggggaacaattaatgatttcagaccttttccaagatgtgttgcgtaaacgcggcatacacctgcacaatcattacggaccttcagaaactcatgtggtatctacgtataccattcatcctggagaccctattcctgagcttccgccaatcggtaaaccgataggctgtactgatctatatattttgaatcatcaaaaacagcttcagccatgcggcgtaccaggcgaactctatatttccggcgcaagtgttgccagaggatatgtcaatcacgataaactgacaagcgacaaattttcatccgatccattcaagcctgatgtgatcatgtaccggacaggtgatttggccagacggcttgaagacggcaacatcgaatatatcggacgggcagacaatcaagtgaaaatcagaggttatcgaattgagccgcaagaaatcgaagtcacgctaatgaatcatccggacattagtgaggctgccattctcatctggcaagatcaaaacggtgaacatgaattatgcgcttactattgcagtgtacaaaagctgaacacaatagatttacgcagttatatggctagtgagctcccagaatacatgattccggcgaaatggatatgggttgacagcatacctcttaccccaaacggaaaagtagatcgcgcagcacttccggagccagatgcttcaatcagcggaaacccatatactgcccctcgaaatctgttagaggcaaagctttcgcaactatttgaagatgtgctaaagaatgggcatataggcatccaagacaacttttttgacaatggcggtcactcgttaaaagcaacagtgcttatgtcacggatcgcaaaggaattccatgtgcaagtttcacttaaggacatctttgctcatccgactgttgaaggattagctttaattattcgagaggcagaacaaaatctgtatgcagcaattgaaccagcagaaaaaagggatacatatcctgtatcttcggcccaaaaacgaatctatgtgcttcaacagcttgatgagggtgtcgcctataacatgcctgcggtcttagaactggaaggtgcactggatgtcgccaaactgtctgctgtatgtaaagaactgatcagccggcatgagccgcttcgaacttcctttgtatccggagctgatgacgagccggttcagcgtatccacaccgaagtgccgtttacgttaagtaaagagaccactatcgagggatttgtccgtccctttgatctcagccaggcgccattatttagagcaggccttatagaagtgtcaaacgagaagcatgtattgctggtggatatgcaccatatcatttcagatggcgtatccgttcagctcctaatccgagaatttaccgatctttatgcaaaccggcagcttaagccattgcggatccaatataaagattacgccgtatggcagcagaaatttaaaaagggagactcgtaccaaaagcaggagacttactggcagcagcagtttagcggggaccttcctatactggagcttccaacagataaacgacgtccggcagaacggcaattcataggcggaaaagtaacctttcaattggacaaagagatcacggcccgcataaagcggctcgcccataaaaacagaagcacgctttatatgacgcttctcgctttgtattcagcctttttgtctcggttaagcggtcaggatgatatcgtgattggttcacctatcgccggacggccccatgccgaccttgaagctgttcttgggatgttcgtcaatacattggctctccgcacacgcccggcgggtaataagacatttgaggaatttctgaaagaagtcagacagacggcactagaagcgtatgagcatcaggattacccgtttgaagagcttgtggacaaactcggtgtgcagcgggaaatgagccggaatcctttgtttgacacaacgctagtccttcagaatatggaacagcaaaagctaaaaatgaatgatgtacagcttcagtggaacgacttggagcacccaatatcaaaatttgatatttccctatacgttacagagcatgattccgagcttttctgtcagtttgaatacagtacagctttgtttgagaaagaaaccatccaaaggtgggccagccttttcaccacgcttgtggaacatacagctgccagtcctgaaacagaattggacaatattccaatcttaacaaaagaagaagagcgagatttcattgaatcatgccatctgttggccgtgacggcctattcaatgaatcaaacgctccactatgcactcgaacagcaggcagaaaaaacgcctgatcaggcggccgttatcttcgaagatggagtgatgacctataaagaattgaacgaacaggctaaccgtatcgcctgggagctgatcggacggggggtaaaacccgaaacgactgttgccattataggaaagcgttcacctgaaatgctgcttggcatttatggcattcttaaagctggcggcgcttatctgcccatcgacccggattatccggaagaacgaatcagctttctgctggaggacagcggtacaaacattctcctgcttcagtctgccggccttcatgttccggaatttacaggagagattgtctatctcaatcagacaaatagcggactggcacatcgtttgtccaatccgaatgtggatgttctcccgcaatctttagcctatgtcatctatacatccggctctaccgggatgcctaagggtgttgaaattgaacatcgatcagcggtgaattttttgaattccctacagtcccgctatcagctaaagcattcagatatgattatgcacaaaacatcatattcattcgatgcttcaatatgggagctgttttggtggccttatgccggagcttctgtttatctgcttcctcagggaggcgaaaaagaacctgaagtgatcgcgaaggccatagaagaacaaaagatcacagctatgcattttgtgccttcaatgctccatgcatttttagaacatataaaatatcgctctgtaccgattaagacaaacagactcaagcgagtgttttctgggggagaacagctggggacccatcttgtctcccgattttacgagttgcttccaaatgtttcaataaccaattcctatgggccaacggaagcaaccgtagaagctgcattctttgattgtccgccgcatgaaaaacttgaacggatcccaattggaaaacctgttcatcatgtcagattatatctcctgaatcagaatcagcggatgctgcctgttggatgtatcggcgaactgtacatagccggagcgggtgttgccagaggttatttgaatcggccggcattaacggaggagcgttttcttgaagacccgttttacccgggtgaacgcatgtacaaaaccggggatgtggcgcgctggctccctgacgggaatgttgaattcctcgggcgcacggatgatcaggtgaaaatccgcggctaccggattgagccgggagaaattgaagcggcactaagaagtatagaaggtgtaagagaggcggccgttaccgtacggacagacagcggggagccggaattatgcgcttatgtagaagggctccaaagaaacgaagtccgagcgcagcttgagagactgttgccgggctacatggtcccagcctatatgatagagatggaacagtggccggttacgccaagcggaaagctcgaccgaaacgccctgccagctcctggcggagcggcagatgcggagacctacacagcgccgagaaacgtgactgagatgaagctttctcagctgtgggaggacgtgctgaaaaatggccctgtcgggattcacgacaacttttttgaccgcgggggacattccttaaaagcaacggcgcttgtctcacggatcaccaaagaattcgatgtacaggtgccgctaaaagatgtgtttgcccatccgacggtagaaggactggctaccgttatccgtgaaggaacggacagtccatatgaagcgattaagcccgctgaaaaacaggaaacctatccggtttcctctgcccaaaagcggatttatgtccttcagcagctggaggacggagggacaggctacaatatgccggctgtgttagagctcgaagggaagctcaaccctgaaaggatggacagagctttccaagagctgatcaagcgccacgagtcgcttcgaacctccttcgaacaggacgaaggaggcgatccggtgcagcgcatccatgacgaggtgccgtttacgttacagactacagttctcggcgcacgaaccgaacaggaggccgcagccgcatttatcaaaccgtttgatctcagccaagcgccgctgttccgtgcccaaatcgtaaaggtatcagatgagcggcacctattgctggttgatatgcatcacatcatttcagacggtgtttccgtcaacattctgattcaagaattcggcgagctgtacaataatcggaagcttccggcgctgcgcattcaatataaagattatgccgtatggcaagaaggattcaaaacaggagacgcgtacaaaatgcaggaggcgtactggctgaagcagctcgagggcgagctgcctgtgctggatctccccgctgatcatgcccgcccgccggtgcgaagcttcgcgggtgacaaggtctcatttacgctggaaccagaggttgcatcaggccttcacaagctggcacgagaaaacggaagcacactgtacatggtgctccttgcggcttacaccgcgttcttgtcacgcttaagcggacaggaagatatcatcgtcggctcgccaatcgccggccggccgcacaaggatcttgagccgatactcggcatgtttgtgaacacgctggcgcttcggacgcgcccggagggcgggaagccattcgtacagtatttgcaggaagtgcgtgagacagcattggaagcctttgagcaccagaattacccgttcgaagagcttgtcgataagcttgaattgacacgagatatgagccggaacccagtgtttgatgcgatgttagttgttcaaaataatgattacgagccattgcatcttcatgatttgcaaatgaagccggcacaagtttctcatctcgtttctaaattcgatttgacactacaggcatctgagggcgacggaaacattcatttcctttttgaatattcaaccgcattgttcgagaaaaccaccattgaacgctgggcatcgcatttaacaaatgtacttagcatcatcggcaaaaacccgaaggtgacactcaaccatatcgacatcctgacccaagaagagcggcaccagctgcttaatgagtttaacaccggggccgcgaaggcctacggagttcaaacaatcagtcaattgtttgagcagcaagctgcacgaacaccaaaagcttctgcacttgtcagcggagacaaaacactcacttatcaggagcttgacgagtggtccaatggaatcgcacgtgcattgcgcagccgaggtgttaagccggacacaccagtaggcatcatgatgcatcgttcgttcagtatgatagcatccatacttggtgtgtggaaagccggaggctgttacgttcccattgatcctgaatacccgaaagaacggaaacgctatatcctcagcgacagcggaacgaaactgctgatgacaataaatgaagcggatctgggagtacttgctgactttgaaggagagatcttgacgatagaaagcgtagaggaagacgacaaatcgccgctgccgcaaatgtcgtctgcccatcatttggcttatatcatttatacttcaggaacgacgggccgtccaaaaggggtaatggtcgagcataaagggattgctaacactcttcagtggcggcgaaacgcttatgcattcaacgagacagataccattctgcagctcttttctttctcatttgacggctttataactagtatgtttacaccgcttttgtcaggtgcaaaagccgttttgcttcatgaagaggaagcgaaggatattctggccattaagcatcagctgtctcgtcaacggattacacatatgattattgtgcctgttttatatcgagcgcttttggacgtagtgcagccggaagatgtaaagacgcttagagtcgtcacactggcgggagaagcggctgaccgcgaattgatcgcccgcagcttagctatatgtccgcataccgaactcgccaacgaatatggaccgacagaaaacagcgtggcgactaccgtcatgagacatatggaaaagcaggcatacgtaagcatcggccagccgattgacggaactcaagtgctgattttaaatagcaatcatcagcttcagccaatcggtgttgcgggagagctttgtatagcaggaacagggcttgcaagagggtacgttaatcttccagaactgacagagagagcattcacgcagaatccatttaaacccgaagcacgaatgtaccgaacaggagacgccgccagatggatggccgacggtacactcgaatatctcggaagaatcgatgatcaagtcaaaatcagaggataccgtgtagaaacgaaagaaattgaatcggtcatccggtgtataaagggtgtaaaagacgccgcagtagttgctcatgtaacagcgtcaggacaaaccgaattaagcgcttatgtggtgacaaaaccagggttgagcacaaatgctgtacgctcagaattacaaaacaagctgccggtgtttatgcaccctgcgtttattgaaaaactggactcacttccattgtcaccaaacggcaagctggatcgcggagcacttccaaaacctgtatacaaccacgaaggtgaacgtccattcctcccgccatccagcaaaatggaacaaatactggcagatatatggaaagaagtactgggggcagaaaagatcggaacagctgattcgttctttgaacttggcggagattcaatcaaagcgttacaggtatctgcgcggcttcaccggataggcaagcaaatggcagtgaaagatttgtttagccatccgaccattcaagaattggcagcttatatccgtgattcagatacaagttccagccaagctgcggttgagggagacgtacaatggtcgcctgttcaaaaatggtttctttctcaagatataaaagaaaaacaccattttaatcagtccgtaatgctgcatcgaagcacctctgtacaagaagacgcactgcgaaaaacgttaaaagcaataacgtgtcatcatgatgcgctgcgaatggtgtttacacagaatgaacaaggaaagtgggatcaatataatcggccgctcagtcattcggacgacgcgttgtacggccttcagatgattgatttgtcagctccggacggcactgatggaaatagaccgtatgaacctcttatcaagcgccatgtacttgatattcagcagaaaatggatttgaagaatggtccgctgctgcaagccggtcttttccacacaattgacggtgatttcttatttttatctgctcatcacctcgtcgttgacggcatctcatggcgggttctgcttgaagatttggctttagggtatcgccaagctgctggcggggaggatatcaaactgccgcctaaaacaagctcgtttaaagcgtatgcgaaaaagctctctgactacgctgaaagccagcagctaatgaaacagctcaagtattggcgcgaagccgaagagtatcaaacagaggcattgccttttgatcaaatcgatggaactagagcacacgagggacaacggtccacaatttcgtttaccttaaacgataaagagacagcagcactcttaaaagacgccaacagcgcatataacactgatacgcaggacatgctgctcgcttctgtcattcttgcgctgcgccattggaccaatcaatccgccttcaaactatcattagagggccacgggcgagaggatgtattaaaaggaatagatgtgagccggacgattggatggtttaccgccatttatccgttattgattaaactgaacgcagacttgccagattcggaagaaagcatggttcatgtgctaaaaacaacaaaagatacactgagacgtgtacctgacaaaggattcggctacggtgtcatcaaatatttgactccgcctggcaaaaaagacatcaatttcacaggtgcaccagaaatcagctttaattatcttggtcaatttgaaagcggccgcacagctgaagtacctgaggaggacgccttctcattctctccgctgggtgccggaggtgatatcagcacaacatggaaccgtgaacagtcgctggatatcagcgcaatcgctgcagaaggaaaattgactgtcaatatgacttatgacaatgcccgctttcagcgcaaaaccatcgaacagcttagcgaaacatgccgtcaatttttattacagctgatcgaacactgccagaacaaaagcgaaacagaaaagacgatcagtgattttgatgatcaagaactgaccgaggacgccctgcaagagatcgctgatatgctcagttttcactaatgaatccgtgaagaaaggtgcagacactatgaataccattaaaaaaatcaagaacatttatcctctgagtcatatgcaggaagggatgctgtttcattccttcctccgtaaagaggagggggcgtatgttgagcagtcgctcttcaccattaaaggaagcctcagctatgactggttccagcgcagcattcaagccattatcgaccgccatgatattttcagaaccgtgtttttgccgcacgtcccgcatttgtcgggacctcggcaagtcgtgatgacagaacgtgaattccatttgaacagcgaagacatttctcatctgccgacaaacgaccagaatgagtatattgaacgctttaaagagaaggacaagcaaaaaggctttgatctgcaaaaagacatgctgatgcggatttctctattcaaaacagctaaagatgagcatgtctgtatctggagtcaccatcacattttaatggacggatggtgcctaggtatcgttatgcaggaatttatgcaaatttatcaatcgattcatgcaggaaaaccgctttcattagaccctgtccgtccgtacagcacctatatttcatggctgacaaaccgagacaaagaaaaagcagcggcctactgggatacctatttaaaaaactacagcgctccatcacctctgcctcgtgtgtctgataaagaaacaaaagaaagttatcaccgtgaagatttgatattttcattaaataaaccactgacagacaagctgaaagagactgccaaacaacacggcgtcacgctcgctacccttattcaggcagtctggggtgtgatgctgcagcaatataaccgcacagacgacgttgtgtttggcgcagttgtatcaggaagaccgtcagaaatcccaggcgtggagcaaatgatagggttgtttatcaataccataccgattcgaattaaaacacaccaagacgaaacgtttcacgagctgctcatacgctgccagaaagaaatgctggaagctgagccgtttacctgccagcctttatttgatattcaggcaaacaccgcattaaaacaggaactgattgatcacattatcgtctttgaaaactatccgttacagcagaaaatcgccgattccgctgatcaaaccgattcaccgctgcaaatcgatcaagttcaagtatccgagcaatcaggatataactttaatcttgtcgttgctcctggcgaagagcttgtcatcaagttcagctataatgcattcgtttacgatgctgcctggatcagctgtatcaagaggcaatttacgcaagcgcttagcacagctgcacagcaccctcatatgccaattgctgatttttcttttcttgatgcaacagaaaaagagcagattgtcacacagttcaacaatacggccacggaggccccaaagaatcatacaattatcgatttatttcgcgaacaagcagaaaagacgccagaccataccgcacttgtgtatggcaatatgtctatttcgtataaagagcttgataaacgctctaatgcgctcgccagagagttaattcaaaagggatttcggaaaaacgagacagccggaatattggctgcacattctcccgaattcatgatcagtgtgcttgccgtattaaaagcagggggagcatacctcccgcttgatgcggagcttccgcctgaacgagtcagctttatgcttgaggaaacgcaggcaaaaatgctgattgttcaaaagggattggagcaaaacgctgcgttctcaggaacatgtatcatttcagatgcgcagggattgatggaagagaacgatatccctattaatatcagctccagcccggatgatcttgcgtacatcatgtatacctcaggatcaacaggccggccgaaaggggtcatgatcacgaatcgcaatgtcgtgtcccttgtcagaaacagcaattacacgtctgcgtccggtgatgaccggtttattatgactggatctatcagctttgacgccgtcacctttgaaatgttcggggcacttttaaatggcgcaagccttcatatcattgataaatcgacaatgctgacacctgatcggtttggagcgtatttgcttgaaaatgacattacagtgctatttttaacgacagctctttttaatcagctggcacaggtacgagctgacatgtttcgcggactccatacgttatatgtcggaggagaagcactctctcctgccctgatgaatgccgtcagacacgcctgtccagatctcgcgcttcataatatttacgggccaacggaaaacacgactttttcaaccttttttgaaatgaagagagactatgcggggccgattccgattggaaaaccaatcagtaatagcaccgcttacatcttagatacaaaaggacgtcttttgccaataggcgttcccggcgagctttgtgttggcggtgatggagtcgctaaaggctatttgaacagagtagatctgacaaatgctgtgttttctcctcatcctttcttgcctggagaaagaatataccgtactggtgatttggcgcgctggctgcctgatggaaacttagaatacatcagcagaattgacaggcaaatgaaaatccgcggaaaacgaattgagcctgccgaaatagaagcgcgcctgttagaaatggaaggcgttcaagaagcagcagtgacattgagagaaaaagatggagaggcgcagctgtacactcattacgtcggtgatcacaaaaaaacagatacggattttcgcgccgatttggcgcgtgtgcttccagactatatgatcccgcagcactgggtgcgtgtggagcggatgccgcttaccggaaacggaaaaatagaccgcagcgcgctgcctattccagaaaataagcctgccaaacgacagaacatcatattgccaagaaacttggttgaagaagaattggcgaacatttggaagcaagtcctcggtgttaacacaatcagtattgatgatgacttctttgctattggcggacattcactaagagcactgcaagtcatacatacactaaaacatcagcagaacattgacataccgattgatttcttgttcgaacatccgacaatcgctcagcttgccgaaaaactttattctaaacagctgacagcagcaaatgaacagcatgtgatcaaactgaaccagcacggcgcgcaaaatcttttctgcttcccgccgatatcgggatttggcatttattttaaagaccttgctttattgctgaatgagaaggcagccgtatacgggtttcactttattgaacaagacacccgcattgaacaatatgttaattgcatgacggacatacagcctgagggcccatacgttttattaggctactctgcaggcggaaacctggcttttgaagtggcacaggctatggagcgcaaaggattagaagtcagcgacttcattatcgtggacgcttatctaaaagaacagcctttgcctatcgataccggtaatgacgaatctgcagcatatctgcctgaagcagtcagagaaaaggtgatgaagaaaaaaagaaactatcaggaatattgggcacaattgctgaatgaaggccacatcaaagcaagcattcatttcatcgaagctggaatccaccccgaaaccagcgggcatacaggcttaacgaaatgggaaggcgcctgcggaaactatagtgagtacacgggttttggcgctcataaagacatgctggaaggaacatatgctgaaaagaatgccgacatcatcctcgacattttagaaaagatcacttcaaatcaagtaatactgcacaaacgataaagcggattagcggacagaggccattctctgtccgtctttctttttgtatggccgtctgtgagctttaatgcggtagtttatcacagttaaattgctaacgcagtcaggcaccgtgtatgaaatctaacaatgcgctcatcgtcatcctcggcaccgtcaccctggatgctgtaggcataggcttggttatgccggtactgccgggcctcttgcgggatatcgtccattccgacagcatcgccagtcactatggcgtgctgctagcgctatatgcgttgatgcaatttctatgcgcacccgttctcggagcactgtccgaccgctttggccgccgcccagtcctgctcgcttcgctacttggagccactatcgactacgcgatcatggcgaccacacccgtcctgtggatcctctacgccggacgcatcgtggccggcatcaccggcgccacaggtgcggttgctggcgcctatatcgccgacatcaccgatggggaagatcgggctcgccacttcgggctcatgagcgcttgtttcggcgtgggtatggtggcaggccccgtggccgggggactgttgggcgccatctccttgcatgcaccattccttgcggcggcggtgctcaacggcctcaacctactactgggctgcttcctaatgcaggagtcgcataagggagagcgtcgaccgatgcccttgagagccttcaacccagtcagctccttccggtgggcgcggggcatgactatcgtcgccgcacttatgactgtcttctttatcatgcaactcgtaggacaggtgccggcagcgctctgggtcattttcggcgaggaccgctttcgctggagcgcgacgatgatcggcctgtcgcttgcggtattcggaatcttgcacgccctcgctcaagccttcgtcactggtcccgccaccaaacgtttcggcgagaagcaggccattatcgccggcatggcggccgacgcgctgggctacgtcttgctggcgttcgcgacgcgaggctggatggccttccccattatgattcttctcgcttccggcggcatcgggatgcccgcgttgcaggccatgctgtccaggcaggtagatgacgaccatcagggacagcttcaaggatcgctcgcggctcttaccagcctaacttcgatcattggaccgctgatcgtcacggcgatttatgccgcctcggcgagcacatggaacgggttggcatggattgtaggcgccgccctataccttgtctgcctccccgcgttgcgtcgcggtgcatggagccgggccacctcgacctgaatggaagccggcggcacctcgctaacggattcaccactccaagaattggagccaatcaattcttgcggagaactgtgaatgcgcaaaccaacccttggcagaacatatccatcgcgtccgccatctccagcagccgcacgcggcgcatctcgggcagcgttgggtcctggccacgggtgcgcatgatcgtgctcctgtcgttgaggacccggctaggctggcggggttgccttactggttagcagaatgaatcaccgatacgcgagcgaacgtgaagcgactgctgctgcaaaacgtctgcgacctgagcaacaacatgaatggtcttcggtttccgtgtttcgtaaagtctggaaacgcggaagtcagcgccctgcaccattatgttccggatctgcatcgcaggatgctgctggctaccctgtggaacacctacatctgtattaacgaagcgctggcattgaccctgagtgatttttctctggtcccgccgcatccataccgccagttgtttaccctcacaacgttccagtaaccgggcatgttcatcatcagtaacccgtatcgtgagcatcctctctcgtttcatcggtatcattacccccatgaacagaaatcccccttacacggaggcatcagtgaccaaacaggaaaaaaccgcccttaacatggcccgctttatcagaagccagacattaacgcttctggagaaactcaacgagctggacgcggatgaacaggcagacatctgtgaatcgcttcacgaccacgctgatgagctttaccgcagaattcgcccttcccggtcgatatgaacagcttatttacataattcacgttattggtagttataaatgaaattcctaatatcggttatgaagtgaaattgaatttctacttgatctttctctctatttttgtaaaataaaattaagaatatttaaatattcaatgattcatttttgcagaaatcggaggaagaagaatatatgaaaacatttaacatttctcaacaagatccccccatattgttgtataagtgatgaaatactgaatttaaaacttagtttatatgtggtaaaatgttttaatcaagtttaggaggaattaattatgaagtgtaatgaataatgaatgtaacagggttcaattaaaagagggaagcgtatcattaaccctataaactacgtctgccctcattattggagggtgaaatgtgaatacatcctattcacaatcgaatttacgacacaaccaaattttaatttggctttgcattttatctttttttagcgtattaaatgaaatggttttgaacgtctcattacctgatattgcaaatgattttaataaaccacctgcgagtacaaactgggtgaacacagcctttatgttaaccttttccattggaacagctgtatatggaaagctatctgatcaattaggcatcaaaaggttactcctatttggaattataataaattgtttcgggtcggtaattgggtttgttggccattctttcttttccttacttattatggctcgttttattcaaggggctggtgcagctgcatttccagcactcgtaatggttgtagttgcgcgctatattccaaaggaaaataggggtaaagcatttggtcttattggatcgatagtagccatgggagaaggagtcggtccagcgattggtggaatgatagcccattatattcattggtcctatcttctactcattcctatgataacaattatcactgttccgtttcttatgaaattattaaagaaagaagtaaggataaaaggtcattttgatatcaaaggaattatactaatgtctgtaggcattgtattttttatgttgtttacaacatcatatagcatttcttttcttatcgttagcgtgctgtcattcctgatatttgtaaaacatatcaggaaagtaacagatccttttgttgatcccggattagggaaaaatataccttttatgattggagttctttgtgggggaattatatttggaacagtagcagggtttgtctctatggttccttatatgatgaaagatgttcaccagctaagtactgccgaaatcggaagtgtaattattttccctggaacaatgagtgtcattattttcggctacattggtgggatacttgttgatagaagaggtcctttatacgtgttaaacatcggagttacatttctttctgttagctttttaactgcttcctttcttttagaaacaacatcatggttcatgacaattataatcgtatttgttttaggtgggctttcgttcaccaaaacagttatatcaacaattgtttcaagtagcttgaaacagcaggaagctggtgctggaatgagtttgcttaactttaccagctttttatcagagggaacaggtattgcaattgtaggtggtttattatccatacccttacttgatcaaaggttgttacctatggaagttgatcagtcaacttatctgtatagtaatttgttattacttttttcaggaatcattgtcattagttggctggttaccttgaatgtatataaacattctcaaagggatttctaaatcgttaagggatcaactttgggagagagttcaaaattgatcctttttttataacaggaattgggcatcaaataaaacgaaaggctcagtcgaaagactgggcctttcgttttatctgttgtttgtcggtgaacgctctcctgagtaggacaaatccgccgggagcggatttgaacgttgcgaagcaacggcccggagggtggcgggcaggacgcccgccataaactgccaggcatcaaattaagcagaaggccatcctgacggatggcctttttgcgtttctacaaactcttcctgtcgtcatatctacaattctacacagcccagtccagactattcggcactgaaattatgggtgaagtggtcaagacctcactaggcaccttaaaaatagcgcaccctgaagaagatttatttgaggtagcccttgcctacctagcttccaagaaagatatcctaacagcacaagagcggaaagatgttttgttctacatccagaacaacctctgctaaaattcctgaaaaattttgcaaaaagttgttgactttatctacaaggtgtggcataatgtgtggaattgtgagcggataacaattaagctaattctatggtaaaagcattcctgaacccaatatccttatttttagtggacaaggccttgttctcatatggttgcttgagccagtgccttacaaggctcttccgctttggcaggctgttcaaaattatttattagagcaactcaaggaactaggcggagatccaaaagcaaccgatgcagcacgtgtttttcggattgctgggagcgtcaatagtaagaatggagcggaagtaagagcggaatatcggcacgattacagatatgagttaaggcagattcaatttgattaccttccagaactcaatgaggttattaatcccgctccacaaaagaaaaaacgggggcgtaaaaagaaagtagttcagttattcaatacctacaaactccattacgctcgcctattggatatagtgaaattggtggaactacgaaattatgaggtaactggatacagggaaatcatttgctttttataccgttattggttgtgctgttacacgaacgaccctgtagaggctttaaatcaaacacagacacttaatttacagttcactgagcctttacccttaaaagaggttgaaagggctacacggagcgcagaaaaggcgtgggaagcacgaaataacgaagaggctaaccggattgcaatcgaaaaaggatatcccagtgctggatacaatattagcaataaaaagttgattgaatggctagatatcacaccagaagaacagaagcatttacagacgattatagacgctaatgagaaacggagaagaaagcgggaaagggataggatttatcaagaacaaaaacgtcgtgagcggggagatatgacccgacaggagtatattaagcaacaacaggataaaacagatgataaattatttaaattgcaggagttattagaacagaatcccaaaatctcaaaaattaaattagcaaaaatacttggtgtagataaatcgcacttatacagactgctgaaacaactataactggaaaaaattagtgtctcatggttcgtcgcccttatattatgggcgttagcctgcttgctaattggataggtgttattgtcatttcaacgtcggacgttttggtagatgaacgtcggacgttatttgcttcaatagattgttgatgtattaagggttgcagtgaatcgacaagcaaaaagttatgacgttgtgaaaaaattgaatagaaaattggaaattacgtcggacgttctaacttaaaaaccctgttatatcaatgatttaaaaggaaattaacgtcataaaagacctttctgcaacaaaagtttttctggaagagttgaggttattttataggtattatggacttttgtagactttttgtgtactttttgtggactccacactcgctggtatcgtgttattttttaattgagatatgaatatggaaattaaacgttttaggcgttggtttggtgatgacaaaaaaataagagtacccgctcacaacggatactctttcgagaaatgtacgaaacgctataaataaaaaataactagatacatttacattgtatcacgtttcgtacatttctccaataacaaattgattggaggaatgcaaagtgaataatgaaccagtaaaacgtggtaagaagaacagatgggaattaaacctacctataatgacttatgtagtagctgatgattggattgataaactaggacacgaaacgtttactttatggttgaggttccatacttgggtagatagagaagatgaactccgagattatgatcgcatacctagaagttttgagaacatatataaaaagacactaggaatctcaaaaagtaagttttatagattgataaaacctttatgggaatatggattaatagacatcatagaatacgaagaatctaaccgtaattctactaaacctaaaaatataattgtttatgagtatcctttacacgaaatagaaagaaagtataaaccactagaaaaattaagagattgggataaagactataattccgtttctaaagaattaggtaaaacaggtggtagaccaaggaaaaaagatagtgaagaagaacccgaaaagaaacccgaagaagtaactaaaaagaaacgtaaatataagttaaaaagagttatccacaacggtttcaaaaatgaaacggtggagggtttcaaaaatgaaacggtggagggtttcaaaaatgaaacggtgaccgtttcaaaaataaaacccaataattattcaaatatctttaataacttatcaaatatttctactaatgtttcaaataatttattaattgatgatgatgaggaaatcgaaaatgaaccaactggtcgtacaataaataggtcattacttttttcacaagaagatattaaacaggcctatcaatttattaatagattttcagttatacagttacgtgaaaactttagctttgataaacactttgaagaacggttggtatgttatttatggaaagcagggatttctactttttacacgcacgaaatcagtaaaatgataaaaaaaatagcagactatgaaaaatctaaaaaaggtagattaaacccaatacgtgaccgagccttatatatggtaaatggtcttgtaatgaatagagcttcttcccaaagtgaacatgctacttataaactaaaccaatataaaaaacagaaggaacaggaaaaacaacaacaggagcaacaaagatcaagagtaccgttctataattggttggaggaaagagaagaacaaaccgaaggtcaactacccaccacttaaagcctaacggcttttgaagtggggcttgtaaaaagccctagttgactaccccaagtctttcgaggactacgttggaaaggtcatgacacctacaaatgctcctctagttcgtagccactgtcgttgatggttaaaagtcctgatgggtagggacggtgctgtcaacatcacaagcccttccaacatgggggaagaggaagaacactccgagaaaggagggggctgtcgtacacgccttgttcgtgtacgtgatttttaacacttttatctctaatataatctctccttgagttagcagagactaagaataaaacacattaggattttttatctacataaggaggttcaatacatgcctactatttcgtttaagggaaagtcttttgtacaaaatcatcacttgactgtaaaatatcatgaattgatcccagaaccagaaaaaagtctgaccgataaagttagtcttcatgacaatcttatcattcatggggacaatttaaaggcgttgaaagctctactacctacatatgctggtaagatagattgcatctatattgacccaccatacaatactggaactgaaaaatggatttataatgataatgtcaactccccaatgattagggaatggcttggaaaagtggtagacaaagaagacttatcccgacatgataagtggctttgtatgatgatgccgaggttaaaactgttgaaagagttgttgtcagaagacggagtgatatttgtaagcattgactacaatgaaatacaccatcttacgtgccttatgaacgaaatattcggtgaggagaattttcgtgacgctattatcattcgtagaggagtaaaaaatgttcaagcgcaatttgacacaattgattctctttcaaatggttatgagtctattttggtttacactaaacagccatctcgacgatttaataaggtttatgaagatgtagaagaaaagcctggtagttggaataatcattggagaggtacagaccgtaaaactatgagatatgaattatttggggttactccgacagaaggtcaatggagatgggggaaagaacgtagtctccaggctattgaaaactatcaaatgatgttagatgaacttagacaaaaaggcattactaatccaactcaagaggatattgataaatggtatcttgaatatgtagaaaataatggggaagatattgacttgttacgacaaaatgataatggcacgattgagcactttgttccaccgactagcaaaaagttgttaagtaatgcctggtttgacttaaaacccaacggttctagtcaattaaagaagatatttggaaggaaggttttcgataaccctaaatcaattgatttggtaaaaagactaatacaatttgcgactgaaaacaaagaagcgattgtacttgactcatttgcagggagtggcactactgctcatgcagtattatcgcttaacaaacaagatggagggaatcgtcgtttcatccttattgagatggaagaatatgcacatgagattaccgcagaacgcggatctttatcgatttgcatgcaagctaattcggtggaaacgaggtcatcatttccttccgaaaaaacggttgcatttaaatcttacatatgtaatactttcaaagactacatttgtaagatttgatgtttgagtcggctgaaagatcgtacgtaccaattattgtttcgtgattgttcaagccataacactgtagggatagtggaaagagtgcttcatctggttacgatcaatcaaatattcaaacggagggagacgattttgatgaaaccagtaacgttatacgatgtcgcagagtatgccggtgtctcttatcagaccgtttcccgcgtggtgaaccaggccagccacgtttctgcgaaaacgcgggaaaaagtggaagcggcgatggcggagctgaattacattcccaaccgcgtggcacaacaactggcgggcaaacagtcgttgctgattggcgttgccacctccagtctggccctgcacgcgccgtcgcaaattgtcgcggcgattaaatctcgcgccgatcaactgggtgccagcgtggtggtgtcgatggtagaacgaagcggcgtcgaagcctgtaaaacggcggtgcacaatcttctcgcgcaacgcgtcagtgggctgatcattaactatccgctggatgaccaggatgccattgctgtggaagctgcctgcactaatgttccggcgttatttcttgatgtctctgaccagacacccatcaacagtattattttctcccatgaagacggtacgcgactgggcgtggagcatctggtcgcattgggtcaccagcaaatcgcgctgttagcgggcccattaagttctgtctcggcgcgtctgcgtctggctggctggcataaatatctcactcgcaatcaaattcagccgatagcggaacgggaaggcgactggagtgccatgtccggttttcaacaaaccatgcaaatgctgaatgagggcatcgttcccactgcgatgctggttgccaacgatcagatggcgctgggcgcaatgcgcgccattaccgagtccgggctgcgcgttggtgcggatatctcggtagtgggatacgacgataccgaagacagctcatgttatatcccgccgttaaccaccatcaaacaggattttcgcctgctggggcaaaccagcgtggaccgcttgctgcaactctctcagggccaggcggtgaagggcaatcagctgttgcccgtctcactggtgaaaagaaaaaccaccctggcgcccaatacgcaaaccgcctctccccgcgcgttggccgattcattaatgcagctggcacgacaggtttcccgactggaaagcgggcagtgagcgcaacgcaattaatgtgagttaggatcctgcctcgcgcgtttcggtgatgacggtgaaaacctctgacacatgcagctcccggagacggtcacagcttgtctgtaagcggatgccgggagcagacaagcccgtcagggcgcgtcagcgggtgttggcgggtgtcggggcgcagccatgacccagtcacgtagcgatagcggagtgtatactggcttaactatgcggcatcagagcagattgtactgagagtgcaccatatgcggtgtgaaataccgcacagatgcgtaaggagaaaataccgcatcaggcgctcttccgcttcctcgctcactgactcgctgcgctcggtcgttcggctgcggcgagcggtatcagctcactcaaaggcggtaatacggttatccacagaatcaggggataacgcaggaaagaacatgtgagcaaaaggccagcaaaaggccaggaaccgtaaaaaggccgcgttgctggcgtttttccataggctccgcccccctgacgagcatcacaaaaatcgacgctcaagtcagaggtggcgaaacccgacaggactataaagataccaggcgtttccccctggaagctccctcgtgcgctctcctgttccgaccctgccgcttaccggatacctgtccgcctttctcccttcgggaagcgtggcgctttctcatagctcacgctgtaggtatctcagttcggtgtaggtcgttcgctccaagctgggctgtgtgcacgaaccccccgttcagcccgaccgctgcgccttatccggtaactatcgtcttgagtccaacccggtaagacacgacttatcgccactggcagcagccactggtaacaggattagcagagcgaggtatgtaggcggtgctacagagttcttgaagtggtggcctaactacggctacactagaaggacagtatttggtatctgcgctctgctgaagccagttaccttcggaaaaagagttggtagctcttgatccggcaaacaaaccaccgctggtagcggtggtttttttgtttgcaagcagcagattacgcgcagaaaaaaaggatctcaagaagatcctttgatcttttctacggggtctgacgctcagtggaacgaaaactcacgttaagggattttggtcatgagattatcaaaaaggatcttcacctagatccttttaaattaaaaatgaagttttaaatcaatctaaagtatatatgagtaaacttggtctgacagttaccaatgcttaatcagtgaggcacctatctcagcgatctgtctatttcgttcatccatagttgcctgactccccgtcgtgtagataactacgatacgggagggcttaccatctggccccagtgctgcaatgataccgcgagacccacgctcaccggctccagatttatcagcaataaaccagccagccggaagggccgagcgcagaagtggtcctgcaactttatccgcctccatccagtctattaattgttgccgggaagctagagtaagtagttcgccagttaatagtttgcgcaacgttgttgccattgctgcaggcatcgtggtgtcacgctcgtcgtttggtatggcttcattcagctccggttcccaacgatcaaggcgagttacatgatcccccatgttgtgcaaaaaagcggttagctccttcggtcctccgatcgttgtcagaagtaagttggccgcagtgttatcactcatggttatggcagcactgcataattctcttactgtcatgccatccgtaagatgcttttctgtgactggtgagtactcaaccaagtcattctgagaatagtgtatgcggcgaccgagttgctcttgcccggcgtcaacacgggataataccgcgccacatagcagaactttaaaagtgctcatcattggaaaacgttcttcggggcgaaaactctcaaggatcttaccgctgttgagatccagttcgatgtaacccactcgtgcacccaactgatcttcagcatcttttactttcaccagcgtttctgggtgagcaaaaacaggaaggcaaaatgccgcaaaaaagggaataagggcgacacggaaatgttgaatactcatactcttcctttttcaatattattgaagcatttatcagggttattgtctcatgagcggatacatatttgaatgtatttagaaaaataaacaaataggggttccgcgcacatttccccgaaaagtgccacctgacgtctaagaaaccattattatcatgacattaacctataaaaataggcgtatcacgaggccctttcgtcttcaagaattctcatgtttgacagcttatcatcgataagctcac

SEQ ID NO: 24 - DNA, 40 bp, synthetic construct
  misc_feature 1..40: note = primer srf07-F
  source 1..40: mol_type = other DNA
cagcacggccgcagaggcccctgaaggaatggctgttcac

SEQ ID NO: 25 - DNA, 48 bp, synthetic construct
  misc_feature 1..48: note = primer srf07-R
  source 1..48: mol_type = other DNA
ggttgcggccgtcatggccgtcatatgtctttcttctagcaaagcagc

SEQ ID NO: 26 - DNA, 49 bp, synthetic construct
  misc_feature 1..49: note = primer srf08-F
  source 1..49: mol_type = other DNA
tatgacggccatgacggccgcaacctttgcagcactttttgaaaaacag

SEQ ID NO: 27 - DNA, 43 bp, synthetic construct
  misc_feature 1..43: note = primer srf08-R
  source 1..43: mol_type = other DNA
tgtcggggccgtcggggccttgcccttccatgcctcaagaagc

SEQ ID NO: 28 - DNA, 50720 bp, synthetic construct
  misc_feature 1..50720: note = Chimeric construct 1
  source 1..50720: mol_type = other DNA
atgtggcccgggagacctgttttccaagagaaaacaggtttttttatgtctgtaataacgctttgtcgaaccttccaacaattagaagaatgatgcacaaaagaaaattagtccgattaaaaagtagtgtataagaccttatgtaaaacaatacttttatcactttatatccggaaatttgataaaaaaagaaacgaaaaataaagaaataatactatattcaaaaaaaatgttataaaaatttaatgttttttattgtactttaaaaaatatccgttaatatagtgcatatatggattatatagtcatataatttcttttattgtcatttttctgcttttttctacattttcttatcctcttattatgagaactggagggaatccgttgagcgaacatacttattctttaacccatgcccaaaggagagtgtggtttaccgaactgctggagccagataccagcatttgcaatcttacagcttgtgtgaaatttaaaggcaatattgagcttgatactctggagggagcactgaatcattccatctcccgcaacgacgccattagatttcagctgttagaaggagaagagcttgagcctcgattgcaccttactgaatataaatattatccacttagaataattgatttttcaaatgttgaaatgatagaaatagagcaatggattcaggatcaagcgagcattccatttaaactgttcaactcgcctctttttcaattttacctccttagaattgactctcatgaagtttggctatttgcgaaattccatcatatcataatggatggaatctctttaaatgtgatgggaaatcaaattatagatctttatcaaaaaatgaaaaagaaagatcctttacctgatcagccggaaccttcttacttgagctacatcgaaaaagagagtcaatatctacaatctccacggtttgcaaaggaccgtttattttggacgcaaacctttgagcacccgttggaataccactcgttagccgaccagacgtccttacaaaaacagagcacatctgcatccagagacaccatcattctttcacctgatctagagcaaacgattcgaatcttctgcgaagaacacaagatcaatatcatttccttatttatggcttcattttacatatgcatcagccgaatcacttctaaaaaagatcttgccattggcacctactatggcaacagaggttcaaaggctgaaaaagaaatgctcggcatgttcgttagttcccttccaatcagaataacggttgatcctgacacagattttctttcctttgtccgcacaataggcagggaacagctttctgttatgcgtcatcaacggtttccttataatttgcttgtaaatgaattaagaaatgaacagaaggatttacacaaccttatcggtatatctatgcagtatcagccacttcagtggcacaatgcagatgattttgactatgaaacagcgctttatttcagcggatacaccgcgaacgaactttcagttcaaatacaagaacggatagacaatggaaccattcaattaaatttcgactatcaaaataccttgttttctcttgaggatattaaacgaatacaatctcatctgcttaccatactggaaaacgcccttaaacatccgcacagctttataagagaattagatatgacgaatacaagagaaaagcaaaaattgttgtatgagtttaacaagacggccgtggcggcccctaaagctttcaccctgcatgggctgtttgagcgacaggcagctttcacaccggagcggctggccattcgcttttcaggcggttcgctgacatacgctgagcttgatatgtacgccagccggctggctgcgcaccttgcggcacgcggcgtcacaaacgaaagtatcgtcggtgtcctgtctgaacgctcacctgacatgctgatcgctgtccttgctgtattgaaggccggcggggcgtatttgccgcttgatcctgcgtatccaaaggagcggctgagctacatgctgaaagacagcggggcatcgctcttgctgacacagccgggatgctccgcaccaaacttttctggcgaaacgcttgaagtggacatgacatctcttgcgagcgaaaaagcagaaaaccatgagtttactcctgctgacggcggatctctcgcctatgtcatctatacatcgggctctaccgggcagccgaaaggagtggccgttgagcaccgtcaggctgtttcctttctgaccggcatgcagcaccagtttccgctttcggaagatgacattgtcatggtgaaaacctctttttcctttgatgcgtctgtgtggcagctgttttggtggtcgctttccggtgcttcggcgtatctgcttccgcccggctgggagaaagactccgcattgatcgtacaagccattcatcaggaaaacgtgacaacggctcattttattccggctatgctgaacagctttctcgatcaagcggaaatcgaaaggctgagtgacaggacaagcctaaagcgtgtattcgccggaggtgaaccgcttgcgccgcgtacggcagcccgttttgcttctgtattgccgcaggtatcattaatccatggttacgggccgacagaagcaacggtagacgcggcattttacgtattggatccagaacgggacagggatcgtttgcggattccgattgggaagcccgtacctggtgcgcgtttgtatgttttagatccgcatttagccgtacagccttccggtgtcgccggcgaactgtacattgccggagcgggtgttgccagaggttatttgaatcggccggcattaacggaggagcgttttcttgaagacccgttttacccgggggaacgcatgtacaaaaccggggatgtggcgcgctggctccctgacgggaatgttgaattcctcgggcgcacggatgatcaggtaaaaatccgcggctaccggattgagccgggagaaattgaagcggcactaagaagcatagaaggcgtaagagaggcggctgttaccgtacggacagacagcggggagccggaattatgcgcttatgtagaagggctccaaagaaacgaagtgcgtgcacagcttgagagactgttgccgggctacatggtcccagcctatatgatagagatggaacagtggccggttacgccaagcggaaagctcgaccgaaacgccctgccagctcctggcggagcggcagatgcggagacctacacggcgccgagaaacgtgactgagatgaagctttctcagctgtgggaggacgtgctgaaaaatggccctgtcgggattcacgacaacttttttgaccgcgggggacattccttaaaagcaacggcgcttgtctcacggatcgccaaagaattcgatgtacaggtgccgctaaaagatgtgtttgcccatccgacagtagaaggactggctaccgttatccgtgaaggaacggacagtccatatgaagcgattaagcccgctgaaaaacaggaaacctatccggtttcctctgcccaaaagcggatttatgtccttcagcagctggaggacggagggacaggctacaatatgccggctgtgttagagctcgaagggaagctcaaccctgaaaggatggagagagctttcaaagagctgatcaagcgccacgagtcgcttcggacctccttcgaacaggacgcaggaggcgatccggtgcagcgcatccatgacgaggtgccgtttacgttacagactacagttctcggcgaacgaaccgaacaggaggccgcagccgcatttatcaaaccgtttgatctcagccaagcgccgctgttccgtgcccaaatcgtaaagatatcagatgagcggcacctgttgctggttgatatgcatcacatcatttcagacggtgtttccgtcaacattctgattcgggaattcggcgagctgtacaataatcggaatcttccggcactgcgcattcaatataaagattatgccgtatggcgagaaggattcaaaacaggagacgcgtacaaaacgcaagaggcgtactggctgaagcagctcgagggcgagctgcctgtgctggatcttccggctgatcatgcccgcccgccggtgcgaagcttcgcgggtgacaaggtctcatttacgctggatcaagaggttgcatcaggccttcacaagctggcacgtgaaaacggaagcacactgtacatggtgcttcttgcggcttacaccgcgttcttgtcacgcttaagcggacaggaagatatcatcgtcggctcgccaattgccggccggccgcacaaggatcttgagccgatactcggcatgtttgtgaacacgctggcgcttcggacgcgcccggagggcgggaagccattcgtacagtatttgcaggaagtgcgtgagacagcattggaagcctttgagcaccaggattacccgttcgaagagcttgtcgataagcttgaattgacacgagatatgagccggaacccagtgtttgatgcgatgtttatccttcaaaatgtggaaaaacaagacatagatctgagagaaataaaagtccggcctgccaatttcgcacatcacatttccttatttgatatcacattaatagctacggaaataagtggatctatttgctgcgaaatggaatttagtacagaagtattcctgaaagctacgattgaacgctgggctgatcattttatcgaatttctgcatgaggcactttcaactcctgaaacaagccttgcacaaataaacatacttagtgataaagaaaaacaaaaaatagtctttgaatttaacaaaacggccgttgaggccgctcaaaaagatattccttttcatcgcatatttgaagcgaaagctgaagaaaatccagaacatatagctgttattgataacgaaacagagattagctatcgccttctaaatgaaagagccaatcgtctggcacgaacattgcaaaacagaaaaggaccgaagccaactgtggctgttttagccaagcggtccatcgatgcaattgttggagttctggcagtgatgaaagctggcggagtgtatatcccaatcgatgcacattatccaaaagctcgtattgaatacattcttcgtgatagcggggcagatattcttcttttacagagagagttgaagcatttgatttcgaactcgcctgaatctgagatgtctcacatcttccttgacgatgagggctcttttgaagaaagtaactgcaaccttaacttatctcctgctcctgaagagccggtatatatcatttatacgtcaggaacgacgggtgcgcctaaaggtgttattgtcacctatcagaactttactcatgctgctcttgcttggcgtcaaatttatgaactggatcggaagcctgtcagactgcttcaaatcgcgagcttttcattcgatgtcttctcaggagatttggcgagaacattgaccaacggcgggactctaatcgtttgcccagatgaaacacggctggaacctgctgaaatatataaaatcattaaatctcagagaatcacggtgatggagtcgacaccggctctcattatcccggtgatggagtatgtataccgtaaccagttcaagcttcctgacttagacatactgattcttggttccgacatggtgaaagctcaagatttcaaaacattgacagatcgctttggccaaagcatgcgcatcattaatagctatggtgtcacagaggcaaccattgattcgagtttctatgaaaccagtatgggtggagagtgtacgggagataacgtaccaatcggcagcccgctgccgaatgtacacatgtacgtactcagccagactgatcaaattcagccgatcggtgttgccggcgagctgtgcatcggcggggcaggtgttgcgaaaggctatcatcataaacctgacttaacgcaaatgaaatttacagaaaatccatttgtctctggagaaaggctgtacagaaccggtgatcgagcatgctggcttccaaacggaacgatccggcttcttggccgaatggattatcaagtaaagataaatggatacagaattgaaacagaagaaattgaaagtgttctgcttcaaacggggcttgtcagagaagctgctgttgccgttcagcatgataaaaatggacaggctggtttggcagcatatattgtgccttcagacgtcaatacgaatgctctccgtgctgctttaacaaaggaactgccagcgtatatgattcctgcatatctgattcctttagtaaacatgccgctgaccctaaacggaaagctggacagaaatgccttgccggctccaaataatgtgttatcgcgtccatataccgcaccagttaacgacttacaaaaaacgatggcgtatatatgggaagatgtactgagcatgtcacgagtcggcattcacgattccttttttgagcttggcggagactcaattaaagcattacaagtggcagcacgtctggcagctgaaggctggagcatgacaatacgcgacttattccgttattcaacgattcaggaactatgcggacatatcacaccattggcatctcaagcggaccagggacctgcggaaggtgaagctgaactcaccccgattcagcgaagatttttcggacaggtacatgcttttcactatcattacaaccagtccgtcatgcttttcagtgaaaaaggattcaatgctaacgcgcttcatctagcgctgcgtaaaataaccgagcatcatgatgccattcgcatgattttccaacgtgaccaaaacggccatgtcattcagtttaatcgcggaatcaatcacaaggatcatgaactgtttggcctttatatttcagattggacaaaagcatcgctggaaagggctcatcttgatgaaaaacttgccgctgaggaaaccgtcattcaaagcaaaatgaatgtagaaaaagggcccttactgcaagcaggtttgtttaaaacggcagaaggggatcatttgctgattgcacttcatcatcttgtgatagatggcgtttcttggagaattctgcttgaggatttagctgcagcatatcaacaggctttagaaaagaaagaaatccaattaccgccaaaaacggattcttatttatcctacgccgatggtcttacccaaatagctgaaagtaaacaattgctttcagagaaaacgtattggcaaacgattttagacgctcacactgcttttcttcctaaggacatagaaaatgtgccagacaaactccaaatgaacagcgacgcagcagcgtttgtactatccggggactggactgaaaaattgctgtttgaaacccagcaagcctatggtactgatgccaacgaacttttgcttacggctttaggaatggcgctttctgaatggactgggcatgaccaaatcgtgatcagcactgagggacacggtagagaagggcatgtgccaaacattgatatttcaaggacagttggatggtttacctccatttatcctattctgctagacatgggtattcccgagcctttcgaggatcagctcgcataccgaattaagacgacaaaagatatgctgagaagagtaccgaacaaaggaactggatacggattgttaacacacataggagaactgcggcataaagagcctgaggtcagctttaattatctcggtcaatttagcgaagagaaggaagttgaaacgtttcaattatcatattaccagccccgttacgaaatagcgggtgagagagaacgagagtatgagctggacatcaatgctctcattacggacggacggcttcacgtaaaagcggtatacacccaagtgttcagcaaacactcaattgagtgctttatggatcgttttcacaggcatcttatcgagacgattgagcattgttcgcagaaaaaagcacgcgaaaaaacattgagcgatttcagcaataaagaattaacgttgtctgcattatctagcatcgaagatctcgtgaaagatctttaacttttgaaaaggtgtgtggaattgatggcacaatcggcacaaattcaagatatttatccgttatcgcacatgcaggaaggaatgctgtttcattcactaatggatttcagctcgaaagcatatatcgaacagacctcgtttacgatcacagggaatctatgcgtcgactcgtttcaaaagagcttaaaccttcttgtttctagatatgatattttcagaacgattttcattaaagaagtaccagatcttacaggtccgcagcaggtagttctatcaaaccgtgaattgacagtatatagagaagatatttctcgcctggctgatcaagaacagcagacgctgattgatgcttttatgactaaggatcgggaaaaaggatttgatttgcaaaaagatcctttaatgcgtcttgccctttttgatagaggagacagccaatatacatgtgtctggacacatcaccatatcatcatggatgggtggtgtctcggcattattcttaaagagtttttcagcatgtatgattcgctcaaaaataactcacctgtacagcttggcagcacggtgccgtacagccgttatattgaatggctcggagaacaagatcaagaagagactgctgcctactggagcgaatatttgaaggagtacggcaatactgcttctattccccgaataaagcgccgcacggcagacgggaattataaagccgaccaggtcagcttttcattagcgccggatatggttgagaaactgacagaggctgcccaaaactggggagtgacattaaacacgctgtttatgagtatttggggcgtgctgctccatcgatataatgctgcagatgatgccgtttttggctccgtcatttcgggacgcccgtcagcgattgacgggattgaatcaatggtcggtttgtttatcaatactgttccagtgcgaatccgatctgcggaaggcataacattttcttcgctggtcaaagccgtgcaggaggatattttatcatctgaacagcatgggtattatccgctttatgagattcaaaaccatagtccattgaagcaagggttgatcgatcatatttttgtttttgaaaattaccctgtacagcttcatcaggcattaagcgtggagagtgaaaatgacgaaggcgctctgaagctgagtgacatttcaatgtcggaacaaaccaattacgactttaatatcgttatcgttccgggagaatcattttatatcaaattcagctacaacgcagacgtttacgagcgggaggagatgctgaggattcaggggcatctaaagcaagcactggattgcattttgacaaatcccgatgttgccgtcagtgacatcaatatcgtgccgccggaggagcaacaggttatccaattgtttaacgaaacggcccgtccggccgtgaacaaaacgataccccaattgtttgaggaacaagctcacaaaacacctgaagctgctgcattgaaaatgggaaacgagtgctggacctatcgccagttacaagtaagagccaatcagattgcgcacgccctgatagaaaaaggcgttggatctggggatatcgttgctgtaatgatgggccggtcaatggaaatgcctgcagctctgcttgggatttggaaagcaggcggcgcttatatgccgcttgatccacattttccagcagaacgtctttcttttcttctgaaggacagtcaagcggctcaattgctgatagaagaagaccttatttccttgatccctccgtcctatgaaggaaatacgataacgatagaacatacagaaagttaccaaacagaagcgccaaatatgccgccaggtgatctagcctacttgatctatacgtcgggaacgacggggcgccctaaaggggttttagttgatcatcacggtattgccaatacattgcaatggagacgggaagagtatagcatgaccgaacaggatatatccctccatttgttttcgtacgtgtttgacggctgtgtaacgagcttatttaccccgcttttatctggtgcgtgcgtactgctgacaacagatgacgaagcgaaggatgtgctggcccttaagcgaaaaatagcccgttataaggtcagccacatgatcattgttccttccctgtacagggtgttattggaagtgatgactgctgacgatgcaaaaagtcttcgtattgtgacatttgcgggtgaagcggtcacgcctgatctgcttgagttgaatcaaataatttgtccttctgctgaactggcaaatgaatacgggcccacagaaaacagtgtggcaacaacaatattgcggcatctgaataaaaaagagaggatcacgatcggacacccgatcagaaacacaaaagtatttgttttgcacggaaatcaaatgcagccgatcggcgcggcgggtgaactgtgtatttccggcgcgggtcttgcgagaggatactacaaacagcaagagctgacacagaaagcattctccgatcatccattccttgaaggggagcgtttataccgaacaggtgatgcaggccgctttttgcctgatggaacgattgaatatattggacgttttgatgatcaagtgaaaattaggggttatcgtattgaactgagagagattgaaacagttcttcgacaagcaccgggggtaaaagaagcagcggtactggcccgtgatgtttctgctgaggaaaaggagctcgttgcttatatcgttccggaaaagggaaacagcctcccagatttgtatcagcatcttgccgggacattgccgtcctatatgatcccagcaagtattatcaacatcagccagatgccattaacatccagcggcaagcttgacaggtttgcgcttcctgaaccagaaaacaatacgagtgtcacatatatggcgccccgaaccttaatcgaagctgatctcgcacatatttgggaagatgtgctgaataaacagcacatcggcattcgtgatgatttctttcagttaggcggacagtccttaaaagcggccgcactggtatcaagaatacataaaaagcttaatgtcgagctgccgctcagtgaggtgttttcttatccgacggttgaaagcatggcggtcaaattgatgagcttaaaagaacacgcttttacacagattgaacctgcggatcaaagagatgtctatccgctgtctttctcgcaaaaacgattatatgctcttcatcagctggcagatgacagcacaggctacaacatgccagctgtacttgaattacgcggaaatctgaatcgccagcggttgagaagcgttctcacagaacttgtgaatcggcatgaagcattacggactgtttttgtgcttgacagagacgagcctgtgcagatcatttatccagagatggcttttgatctaaaagagcttgaaatggaatcagaacaaatgcttgagtctgcaatcgagacctttatcaaaccgttttatctatcatccggtccgctttttagagcatgtgtcattacaatgggcaataatcgcggctttttgctgctcgatatgcaccatattattgccgacggtgtctcgatgagcactcttgtccaagaatttactgacttatattgcggaaaagagttgccagctttaaacctgcattataaggattttgctgtttggcagcaagagaagcacccgaaagagctatacaaaaaacaggaggcctactggctcggtcagcttggcgggagtcttcctacactagaattaccgcttgataaaacaaggccgcgtctccctgatttcaggggtggaacaattgaagtcaacattgataaagacatggctgatgaactgcaccgtttaatggctgaaacgggaacaacattgtatatgattcttctggctgtctattctattttgttatctaagctaagcgggcaagaggatattgttgtcggttcgcctgctgccggaagaccgcacgctgatctggagcgcgtcatcggaatgttcgtcaatacattggcgatgcgcagcaagcccgagggccacaaaacgttcagctcctatttgcatgacattcgccacctggctctgaccgcttacgagcatcaggattatccttttgaggagctggcagataagctcgatacaaatcgagaggtaaatcgcaacccgctgttcgatgcgatgcttgtgcttcaaagcagtgaagatttccggttcgaagtgcctggtctgtcgatttcgtctgtcactcctaaacatgatatatctaaattcgatttaacattacatgctgaggagcatctgagtggaatacgctgccgttttgaatacagcactgctctttttgaagaagaaaccattacgcagtgggcatcctattttattgaattggtaaaaggggtaacggcggatactgagatgagaatttcgaacatgcaattgcttcctgctgcagagcgtaggttactccttgaaaaaatggggcaggccgccctggccccgagaaatgaaaacatagtaagcttatttgaaaagcaagtagctcagtatccggagcatatcgcagtggtgtgcggccattctcagcttacgtatcgagacctgaatgaaaaagccgagcgggcagctgctatgctgatcaaacaaggggtcagaactggcgatatcgtcggtctgatgctcgatcggtcacctgatatgatcattggcgttttatcgattttaaaagctggcggggcctatttgccgattgatcctgaatatcccaaggagcgtattagctttatgctcaatgacagcggagcaaaactgctgctgacagagcgcggtctaaacaaacctgcagactacaccgggcatattttgtatatcgatgaatgtgaaaacaactcaattccggctgatgtaaacattgaagaaatagtaacggatcagcccgcatacgtgatatacacatctggaacgactggtcagccaaagggagtcattgtcgagcaccgcaatgtgatcagtctcttgaagcatcaaaacctgccttttgaatttaaccatgaagacgtctggacgttatttcattcttattgctttgatttctctgtatgggagatgttcggtgcgttattgaacggaagtacattagtcgtggtctctaaagaaacagcccgtgacccccaagcattccgattattgttaaaaaaagagcgcgtcactgtactcaatcagaccccgactgctttttacggcttgatgcttgaagaccaaaatcatacagatcatttaaacatccgctatgtgatttttggcggcgaagccttacagcccggattgcttcaaagctggaatgaaaaatatcctcatactgatttgattaatatgtacggtattacagaaacaacggtccatgtaacattcaaaaaattgtccgcagcagacattgcaaaaaataaaagcaatatcggccggcctctttctactctgcaggctcatgtgatggatgcccatatgaacctgcagccgaccggagttccaggggagctgtatataggcggcgaaggtgtggcacggggatatctcaacagagatgagctgaccgctgaccgttttgtatccaatccttatcttccgggagacagattataccgaacaggagatcttgctaagcgcctgtcaaatggcgagctggaatacttaggccgcattgatgagcaggtgaaagtcagagggcaccgtattgagttaggcgaaatccaagcggcacttcttcagtatccaatgattaaagaggcggctgtcattaccagagcagacgagcaagggcaaacagctatatatgcatatatggtgataaaagatcaacaggctgcgaatatatcagacatccgaacttacctaaaaaacgccttgcctgactttatgctgcctgcccgtatgatacaaattgacagcatcccggtgactgttaatggaaagctcgatcagaaagccctgccagagcctgaaaaacaagcttatacagctgatgatatcagtcctagaaatgagattgaaacggtgatggctgaaatttgggaagagcttcttaatgtagatgagctgggtgtaagcgccaatttctttaagcttggcggagactctattaaagcgctgcaggtttgtgccagactgaagcagcgcggatttgaaacgacagtacgtgagatgtttgaacatcagactcttggtgaactgtccgcccgggttcgaaaagacgtacgcgccattgaccaaggcccggtcgaaggcgagattacttggacacctatccagcagtggtttttctcgcaatctctggaaagccatcattttaaccaatccgttatgatctaccgggctgaacgatttgatgaggctgcgcttagaaaagtactaaaaagccttgtgactcatcatgatgcactgagaatcgtatgccggcatgaagatggcaggcaagtgcagataaacagagggatagatctttcagatgaggagctatatgcacttgaactgtttgatgtaaaggatagcctaacagaagcccggaacacgattgaggaagcagccagccggatgcaagaacatattcgtttggaaaccggccccttacttcacgctggattgtttagaaccgagaatggtgaccatttatttctaacgattcatcacttagttgttgatgcggtttcttggcgcattttgtttgaggatttttcaacagcttacaaacaggcagtctcaggagaatctattaaactgccgcaaaaaacagattcatatttaacgtattcacaaagaatagctgactactctataagccgccaggtgcagcgcgaagcagcgtactgggatgagtgcgagaaccgtcacatccagcctattccaaaagacaatgacgcagcatctaacacattcaaagatacagaagtgattgattttgagctatctcgccatcacacagaattactattaacggctgcacataaagcttacagcacggagatgaatgatatccttctgacagctttaggtcttgctttgcagaaatggacgggaaataaccaatttaaaatcagcatggagggccatggaagggaatcatatcttgaggacatcgatattagcagaactgttggctggttcacctccatttatcctgtgtggcttgatatgagagattccgatcataaggacaaagaagagcggctgggccaccttattaaacagacaaaagatatgctgcaccgtataccgcataaaggcgcgggctacggcgtgctgaaatatatcagcaaaagatggggctctcagaaaaacagcccagaaatcagctttaattatttaggccagtttgatcaggatattcaatcaaatgcctttgaggtgtctgacatcaagccaggaaatgagatcagcccgaactgggagcgtccttatgcactggatatcagcggcgccgtttcttcggggtgcctgaacatgcacatcatctataacaggtttcaatttgaggaaaaaacaatccaaacattttccaggcattttaaacagactctggaaaacatcattgagcattgtaccggcaaagaaaaccaagagtggagcgcatctgatttcactgatgaagacttaacgcttgatgaattgagtgagatcatgggagccgtcaacaaactataggagaggagattcactgatgccgcagcaacctgaaatacaggatatataccctttgtcatttatgcaggaagggatgctttttcactcactgtatgatgaacagtcgagagcttattttgaacaggcttcttttacgatccatggacagcttgacttggagcgtttccaaaaaagtatggatgctgtttttgacaggtacgatatctttcgaacagcattcatctataaaaatgtagccaaacctcgtcaagtcgtgctcaagcaacgtcattgccctattcatattgaagatatttcccatctcaatgaaagggataaagaacattgtaccgaggcattcaaagagcaggacaaatccaaaggctttgatctccaaacggatgtactgatgagaatatctattttaaaatgggcgcctgatcattatgtctgtatctggagccaccatcatattttaatggatggctggtgtttaggcatcgtcattaaagactttctccatatttatcaagcgctgggtaaaggccagcttcctgatttgcctcccgtacagccgtacgggacgtatattaaatggctgatgcagcaagatcgtgaagaagcagctgagtactggaaaaagaggcttcagcatttcgaaaaatctacacccctgccgaaaagaacagatcaaattccgaatgggacactacagcagatcacgtttgccattcccgaaaaagaaaccgccgaattacagaaaatcgcagcagcttctggtgcgacactaaacactgttttccaagctttatgggggattatgcttcaaaaggtcaatcgcagcagcgatgctgtgttcggttcagttatatcaggcagaccttctgagctaaaagatgtggaaaacatggtcgggctttttatcaataccattcctattcgagcccaaagtgattctctgtctttttctgacctagtcaggagaatgcaaaaggacatgaatgaggcagaagcctatagttactttcccttgtatgatattcaggcgcagagtgctctaaagcaagagttgatcgatcatattatcgtctttgaaaatacacctacccagcaagagatcgaagagctgaatcaagcggggtcatttgatttctccgtcaaagattttgagatggaagaggtgaccaattatagttgcagtgtcaaagtgatcccaggccgtaccttgtacgttcggattcattttcagaccagcgcttatcaaccaagcatgatgtccgaaataaaagattatttgctgcacatggtctctgacgtcatctctgatccatctcttcctgtgtcaaagatgacgttgctagatgaggacaaaacacggaaaatcgtttctcaaaataacaggacggccagtgtggcccctgaagccccaaccctgcatgggctgtttgaacgacaggcggcagtcacaccggagcggctggccattcgcttttcaggcggttcgctgacatacgctgagcttgatatgtacgccagccggctggctgcgcaccttgcggcacgcggcgtcacaaacgaaagtatcgtcggtgtcctgtctgaacgctcacctgacatgctgatcgctgtccttgctgtattgaaggccggaggggcgtatttgccgcttgatcctgcgtatccaaaggagcggctgagctacatgctgaaagacagcggggcatcgctcttgctgacacagccgggatgctccgcaccaaacttttctggcgaaacgcttgaagtggacatgacatctcttgagtgtgaagaagtaaaacgtcatgtgtctgcttctgttagcgacggatctctcgcctatgtcatctatacatcgggctctaccgggcagccgaaaggagtggccgttgagcaccgccaggctgtttcctttctgaccggcatgcagcaccagtttcggctttcggaagatgacattgtcatggtgaaaacctctttttcctttgatgcgtctgtgtggcagctgttttggtgggctctttccggtgcttcggcgtatctgcttccgcccggctgggaaaaagactccgcattgatcgtacaagccattcatcaggaaaacgtgacaacggctcattttattccggctatgctgaacagctttctcgatcaagcggaaatcgaaaggctgagtgacaggacaagcctaaagcgtgtattcgccggaggtgaaccgcttgcgccgcgtacggcagcccgttttgcttctgtattgccgcaggtatcattaatccatggctacgggccgacagaagccacggtagacgcggcattttacgtgttagatccagaacgggacagagaccgtttgcggattccgattgggaagcccgtacctggtgcgcgtttgtatgttttagatccgcatttagccgtacagccttccggtgtcgccggcgaactatacattgccggagcgggtgttgccagaggttatttgaatcggccggcattaacggaggagcgttttcttgaagacccgttttacctgggggaacgcatgtacaaaaccggggatgtggcgcgctggctccctgacgggaatgttgaattcctcgggcgcacggatgatcaggtgaaaatccgcggctaccggattgagccgggagagattgaagcggcactaagaagcatagaaggcgtaagggaggcggccgttaccgtacggacagacagcggcgagccggaattatgcgcttatgtagaagggctccaaagaaacgaagtgcgtgcacagcttcagagactgttgccgggctacatggtcccagcctatatgatagaaatggaacagtggccggttacaccaagcggaaagctcgaccgaaacgccctgccagctcctggcggagcggcagatgcggagacctacacggcgccgagaaacgtgactgagatgaagctttctcagctgtgggaggacgtgctgaaaaatggccctgtcgggattcacgacaacttttttgaccgcgggggacattccttaaaagcaacggcgcttgtctcacggatcgccaaagaattcgatgtacaggtgccgctaaaagatgtgtttgcccatccgacggtagaaggactggctaccgttatccgtgaaggaacggacagtccatatgaagcgattaagcccgctgaaaaacaggaaacctatccggtttcctctgcccaaaagcggatttatgtccttcagcagctggaggacggagggacaggctacaatatgccggctgtgttagagctcgaagggaagctcaaccttgaaaggatggacagagctttcaaagagctgatcaagcgccacgagtcgcttcggaccgccttcgaacaggacgcaggaggcgacccggtgcagcgcatccatgacgaggtgccgtttacgttacagactacagttctcggcgcacgaaccgaagaggaggccgcagccgcatttatcaaaccgtttgatctcagccaagcgccgctgttccgtgcccaaatcgtaaaggtatcagatgagcggcacctgttgctggttgatatgcatcacatcatttcagacggtgtttccgtcaacattctgattcgggaattcggcgaactgtacaataatcggaagcttccggcactgcgcattcaatataaagattatgccgtatggcaagaaggattcaaaacaggagacgcgtacaaaacgcagggggcgtactggctgaagcagctcgagggcgagctgcctgtgctggatcttccggctgatcatgcccgcccgccgatgcgaagcttcgcgggtgacaaggtctcatttacgctggatcaagaggttacatcaggcctttacaagctggcacgagaaaacggaagcacactgtacatggtgctccttgcagcttacaccgcgttcttgtcacgcttaagcggacaggaagatatcatcgtcggctcgccaattgccggccggccgcacaaggatcttgagccgatactcggcatgtttgtgaacacgctggcgcttcggacgcgcccggagggcgggaagccgtttgtacagtacttgcaggaagtgcgcgagacagcaatggaagcctttgagcaccaagattacccgttcgaagagcttgttgataagcttgaattgacacgagatatgagcagaaatccgctgtttgacgtaatgtttgttcttcaaaatatggatcaggaatcgttggagctggatgaactttgtctcaaacctgcagcaaacaatgggcatcaaacgtccaaatttgatttaaccctatatgcccaggaacagccccgcggtttgctgacgttccaaatggagtttagtactgacttatataagaaaaaaacgatagaaaagtggcttcaatacttcaacaatatgttactctccatcatcaaagacaacaaagccgctctcggaacaataaatatcctgaatgaggatgaggcccattaccttatccacgagctcaatcgtacggccatagaggccccaagaaatgaaaccatcagcagactctttgaaatgcaggcagaacaaacacctaatgctgtagcaattgtcagcgacacccaagtattcacttacgaggacctgaacagctgggcaaatcaaattgcctcagttctacagataaagggcgtagggcctgatagtgttgtagccttgttgacaggcagaacaccagaactcattgcaggaatgctgggcattctaaaagccgggggagcctatctgcctatcgattctaatctgcctgttgaacgcatagcttatatgctgtctgacagcagggcagcattactccttcaatctgaaaaaacagaaaaacggctattaggcattgaatgtgaacaaatcataatcgaagatattcaaaagcaaggagaggcgaagaacgttgaatcttcagcagggccccattcacttgcatatatcatttatacctctggatcaaccggtaaaccaaagggtgtcatgattgagcagcgaagtgtaattcgtcttgttaaaaacagcaattatattacatttacacctgaagaccgccttctgatgacatcatcaatcggtttcgacgttgggtcatttgaaattttcggaccgctgctaaatggtgccgctttgcatctgtccgatcaacaaacatttctcgattcccatcagcttaagaggtacatagaacatcaaggaatcacaacgatttggctgacatcttctctattcaatcatttgacagagcaaaatgaacaaacattttcacagctgaaacatttgattattggcggagaagctttgtcgccgagccacgtcaatcgaatcagaaatgtctgccctgaagtatctatatggaatggatatggccctaccgaaaatacaactttttcgacatgccttcacattcaaaaaacatatgaactttccattccgatcgggcggccggttggtaattccaccgcttttatcttaaatcaatggggagtgctgcagccggtcggagctgtcggtgaactttgtgtcggcggagatggcgtcgccagaggatatttgggccgtcctgatttaacgaaagagaaatttgtcccacatccatttgcacctggcgatcgactgtatcgcacaggtgatctggcgcgctggctttccgatggcacaattgagtacgttggccgtattgatgatcaagtaaaagtcagaggctatcgggtggagctgggtgaaatcgaaacagcacttcgtcaaatagacggggtcaaagaagccgcagtgttagcacgtacagcccagaccgggagcaaagagctgtttggctatatcagcgtaaaagcaggcacgaatgctgaacaagtgcgttctcttctcgcgcgttcgctgccaaactatatgatcccggcgtatatcattgaaatggagactcttccgctcacatcaaacggcaaattgaaccggaaagcactgcctgaaccagatgtcgcatctaaacaaacatacatcccgccacgcaacgaacttgaagagcagctggcattgatctggcaggaggttctaggcatccagaggatcggaatagaggattcgttttttgaattgggcggagattcaatcaaagcccttcaagtttctgcacgccttgggcgctatggactaagcttgcaggtaagtgatttattccgtcatccaaagataaaggacttatcaccatttatccgtaagtcagagagaatcatagagcaaggacccattcagggtgacgttccttggacgcctgttcagcaatggtttttttcacaagatattgaagaaagacaccatttcaatcagtctgtcatgctattccattctggacgtttgtctgaaaacgcccttagaccagccttgaaaaaactggcggagcatcatgatgcgcttcggatggtttatcgcaacgatgacaggcgatggattcaaatcaaccaaggcattcatgagtcacagctatacagcttaagaatctctgatctttcacagtcagaaagcggctgggagacgaaaatcaaacaagaagttgccgatcttcagcaaagcatcaatttgcaggaaggaccattgttgcacgccgctttgtttaaaacactgaccggagattacttgttccttgcgatccatcaccttgtcgttgatggtgtctcatggcggattttgctggaggatttgtcagccggatatcaacaagctgctgcaggccagacgatccagcttccgcctaaaacggattcctaccaggaatacgcaagacgcatacaggaatatgcccaaagcagtaagctgattcgcgaagaggcgtattggcgaagtgtagaagaacagcaagccgcagaactgccctatgaaataccgcatcatgtgaacatcgacttcagcaaaagggactcattaagcttttcactgactgaagcagacaccgccgtcttgctgcaaaacgtcaatcacgcctatggcacagatacacaagatattctgttaaccgcagcatccttggcgatttgtgaatggacaggaggaagcaagctccgtatcgctatggaaggacacgggagagaacacattctgccagagttagatataagcaggacggtcggctggtttacatccatgtacccggccctcataagctttgaaaatcatagggatgagctcggaacctcagtaaaaaccgttaaagatacactgggccggataccaaacaaaggggtaggttacggtatgctgaaataccttacacaccctgaaaataaaagcattacgttttcaaaaacacctgaaatcagctttaactatttgggccagttcaacgacatcgaaagacaggacaccttccgcccatcaagccttggtagcggaaaggatatcactcatacatggaagcgcgagcaaatcatcgagatgagtgcaatggcagcagacaaaaagctccatttcaatcttagttatccgccagcccgctttcacagaaacacaatggaacagcttattaacaggattgaacactttttgctggacattatgaaacactgcgccggtcaacagaaagcagaaaagacactgagcgatttcagcagtcaatcattaacggcagaggacttggacagcatatccagcttggtggaagaattgtagaaaatcgtgacaggagacatgaacatgacaaaagcgaattcaattcaggatatttatccgctgtcttacatgcaggaagggatgcttttccattccctcctgcaaaaagattcacaggcgtatgttgagcaagcttcttttacaatagaaggaaaagtcaacccgcagttttttcaaaacagcatcaacgctcttgtagaaagacatgatattttcagaacgatttttatcagccaaaatgtttcctccccccagcaggttgttctgagagaacgaaatgtcatcgtactggaagaagacattactcatttaaacgaggcggagcaatcacagtttatcgagcaatggaaagaaaaggaccgggaccgggggtttcatttgcaaaaggatgtgctcatgcgcatcgctctgattcaaacaggagagagccagtactcttgcatttggacctttcatcatatcatgatggacggttggtgcctcagcattgtgctaaaggagtttctgcatatttacgcatcttatgtaaatgcatccccaataacattggagccggtccagccatacggaaagtatatcaaatggctgatggagcaagacaaagagcaggcggtttcttattgggatcattatctttccggccacgaacagcaaaccgtgctcccgaagcagaaaaaaacaaagggaaaaagcaggcaggaacacgttacattttcattctctaaggaagaaagcagcaggctttcagagcttgctgctagagaagaagtgacactcagtacgatttttcataccatttggggcattctgctgcaaaaatataataataacgatgacgccgtattcggttctgtcatttcaggaagacccgcagaaatcgaaggcattgaacatatggtaggtcttttcattaatacgatgccggttcgggtgcagggggcaaaaacgccttttcttcaacttataaaagatatgcaaaaagaccgtcttgccgctgaagcgtacagctaccaccctttatatgagattcaatcccgctcagctgttaagcaagggctgattgatcatattctcgtatttgaaaactatccggtgcagcaagagattcaaatgctgaacaaacaggaacatgcttctgatctttttcagattcataatttcactgtcgcagatgaaaccaactacagcttttatcttatggtggcgccaggggaagaaattcatatcaaaatgaactatgatgcggagcagcacgatcggtcttttgtgctctctgtcaaagagcatcttctgaatgctgtatcacaaatcttaaataatccgaatcttccacctgaagaaatcgatatcacgacagatactgaaaagcggcagctgattggagaaatcacagatcaggccccagaggcccctgaaggaatggctgttcaccaagtgtttgaagagcaagcgaaacggacgccggcgagcaccgccgtcgtatatgaaggaaccaagctgacgtaccgcgagctgaatgcagcggctaaccgtctggcgagaaagcttgtcgaacatgggcttcaaaaaggggaaacagcagcgattatgaacgaccgctcagtagaaaccgttgtcggcatgctggctgttttaaaagcaggcgccgcatatgtgccgcttgatccagcgcttcctggggatcgtcttcgtttcatggcagaggacagctccgttcgaatggttttgatcggaaattcttatacagggcaggcacatcagctgcaagtgccggttcttacactggacataggctttgaagagagtgaagcggctgacaatctcaacctgccatccgccccgtctgatttggcgtacatcatgtacacatccggttcaacgggcaaaccgaaaggcgtcatgatcgaacataaaagcattctgcgcctcgtcaaaaatgccgggtacgttcctgttactgaagaagaccgcatggcgcaaacgggagctgtcagctttgatgccggaacgtttgaggtattcggcgcactgctgaatggcgcagcactttatccggtcaaaaaagagacactgcttgatgcgaaacaatttgctgcattcctgcgtgagcaaagcatcacaactatgtggctgacatcacctttattcaaccagcttgctgcaaaggatgcgggtatgttcggcacactgcgccatttaatcatcggcggagatgcccttgtcccgcatattgtcagcaaagtaaaacaggcatcgccgtcgctttcattgtggaacggatacggcccgacagaaaacacgacgttttcaaccagttttctgatcgaccgcgagtatggcggctctatcccaatcgggaagccgatcggaaattccactgcctatattatggatgagcagcaatgcctgcagccaatcggcgcgcctggtgagctttgcgtaggcggaatcggtgtagcgcgtgggtatgtcaatctccctgagctgacggagaagcaatttctggaagacccgttcagaccgggtgagagaatttaccgcactggtgacttggcaagatggctgccggacggcaatatcgaatttttaggcagaatcgacaaccaagtgaaggtgcgcggcttccgaattgagcttggcgaaattgaaacaaaactgaacatggctgagcatgtgacagaagccgcggtgatcatacgcaagaacaaagcagacgaaaatgaaatttgcgcgtacttcacggcggatcgtgaagtggctgtgagtgagctgagaaaaacactgtctcagtctttgcctgactatatggtccctgcccacctgattcaaatggacagcctgccgctcacgccaaacgggaaaatcaacaaaaaggaactgcctgcaccgcaatcagaagccgtgcagccggaatacgcagcaccaaaaacagagagtgaaaagaaattagcggagatctgggaaggaatactcggcgtcaaagcaggcgttaccgataacttctttatgatcggcggccattctttgaaagcgatgatgatgacggcgaaaattcaagagcattttcataaggaagttccgataaaagtgctttttgaaaagccgactattcaagaactggcactgtatttggaagagaacgaaagcaaagaagagcagacgttcgaaccgatcaggcaagcatcttatcagcagcattatcctgtatccccggcccagcggagaatgtatatcctcaatcagcttggacaagcaaacacaagctacaacgtccccgctgtacttctgctggagggagaagtagataaagaccggcttgaaaacgcgattcagcaattaatcaaccggcacgaaatcctccgtacatcgtttgacatgatcgacggagaggttgtgcaaaccgttcataaaaacatatcgttccagctggaggctgccaagggacgggaagaagacgcggaagagataatcaaagcatttgttcagccgtttgaattaaaccgcgcgccgctcgtccgttcgaagctgtccagcttggaagaaaaacgccacctgctgctcattgatatgcatcatattattactgacggaagttcaacaggcattctaatcggtgatcttgccaaaatatatcaaggcgcagatctggaactgccacaaattcactataaagattacgcagtttggcacaaagaacaaactaattatcaaaaagatgaggaatactggctcgatgtctttaaaggcgaactgccaatactggatcttcccgcggatttcgagcggccagctgaacggagctttgcgggagagcgcgtgatgtttgggcttgataagcaaatcacggctcaaatcaaatcgctcatggcagaaacagatacgacaatgtacatgtttttgctggcggcgttcaatgtactcctttccaagtacgcgtcacaggatgatatcattgtcggctcgccgacagctggcagaacacatcctgatctgcaaggtgtgccgggtatgtttgtcaacacggtggcactcagaacggcaccagcgggagataaaaccttcgcgcaattccttgaagaggtcaaaacagccagccttcaagcattcgagcaccagagctatccgcttgaggagctgattgaaaagcttccgcttacaagggatacaagcagaagtccgctgttcagcgtgatgttcaacatgcagaatatggagattccttcattaagattaggagatttgaagatttcctcgtattccatgcttcatcatgttgcgaaatttgatctttccttggaagcggtcgagcgtgaagaggatatcggcctaagctttgactatgcgactgccttgtttaaggacgagacgatccgccgctggagccgccactttgtcaatatcatcaaagcggccgcggctaatccgaacgttcggctgtctgatgtagatctgctttcatctgcagaaacggctgctttgctagaagaaagacatatgacggccatgacggcctattcaatgaatcaaacgctccactatgcactcgaacagcaggcagaaaaaacgcctgatcaggcggccgttatcttcgaagatggagtgatgacctataaagaattgaacgaacaggctaaccgtatcgcctgggagctgatcggacggggggtaaaacccgaaacgactgttgccattataggaaagcgttcacctgaaatgctgcttggcatttatggcattcttaaagctggcggcgcttatctgcccatcgacccggattatccggaagaacgaatcagctttctgctggaggacagcggtacaaacattctcctgcttcagtctgccggccttcatgttccggaatttacaggagagattgtctatctcaatcagacaaatagcggactggcacatcgtttgtccaatccgaatgtggatgttctcccgcaatctttagcctatgtcatctatacatccggctctaccgggatgcctaagggtgttgaaattgaacatcgatcagcggtgaattttttgaattccctacagtcccgctatcagctaaagcattcagatatgattatgcacaaaacatcatattcattcgatgcttcaatatgggagctgttttggtggccttatgccggagcttctgtttatctgcttcctcagggaggcgaaaaagaacctgaagtgatcgcgaaggccatagaagaacaaaagatcacagctatgcattttgtgccttcaatgctccatgcatttttagaacatataaaatatcgctctgtaccgattaagacaaacagactcaagcgagtgttttctgggggagaacagctggggacccatcttgtctcccgattttacgagttgcttccaaatgtttcaataaccaattcctatgggccaacggaagcaaccgtagaagctgcattctttgattgtccgccgcatgaaaaacttgaacggatcccaattggaaaacctgttcatcatgtcagattatatctcctgaatcagaatcagcggatgctgcctgttggatgtatcggcgaactgtacatagccggagcgggtgttgccagaggttatttgaatcggccggcattaacggaggagcgttttcttgaagacccgttttacccgggtgaacgcatgtacaaaaccggggatgtggcgcgctggctccctgacgggaatgttgaattcctcgggcgcacggatgatcaggtgaaaatccgcggctaccggattgagccgggagaaattgaagcggcactaagaagtatagaaggtgtaagagaggcggccgttaccgtacggacagacagcggggagccggaattatgcgcttatgtagaagggctccaaagaaacgaagtccgagcgcagcttgagagactgttgccgggctacatggtcccagcctatatgatagagatggaacagtggccggttacgccaagcggaaagctcgaccgaaacgccctgccagctcctggcggagcggcagatgcggagacctacacagcgccgagaaacgtgactgagatgaagctttctcagctgtgggaggacgtgctgaaaaatggccctgtcgggattcacgacaacttttttgaccgcgggggacattccttaaaagcaacggcgcttgtctcacggatcaccaaagaattcgatgtacaggtgccgctaaaagatgtgtttgcccatccgacggtagaaggactggctaccgttatccgtgaaggaacggacagtccatatgaagcgattaagcccgctgaaaaacaggaaacctatccggtttcctctgcccaaaagcggatttatgtccttcagcagctggaggacggagggacaggctacaatatgccggctgtgttagagctcgaagggaagctcaaccctgaaaggatggacagagctttccaagagctgatcaagcgccacgagtcgcttcgaacctccttcgaacaggacgaaggaggcgatccggtgcagcgcatccatgacgaggtgccgtttacgttacagactacagttctcggcgcacgaaccgaacaggaggccgcagccgcatttatcaaaccgtttgatctcagccaagcgccgctgttccgtgcccaaatcgtaaaggtatcagatgagcggcacctattgctggttgatatgcatcacatcatttcagacggtgtttccgtcaacattctgattcaagaattcggcgagctgtacaataatcggaagcttccggcgctgcgcattcaatataaagattatgccgtatggcaagaaggattcaaaacaggagacgcgtacaaaatgcaggaggcgtactggctgaagcagctcgagggcgagctgcctgtgctggatctccccgctgatcatgcccgcccgccggtgcgaagcttcgcgggtgacaaggtctcatttacgctggaaccagaggttgcatcaggccttcacaagctggcacgagaaaacggaagcacactgtacatggtgctccttgcggcttacaccgcgttcttgtcacgcttaagcggacaggaagatatcatcgtcggctcgccaatcgccggccggccgcacaaggatcttgagccgatactcggcatgtttgtgaacacgctggcgcttcggacgcgcccggagggcgggaagccattcgtacagtatttgcaggaagtgcgtgagacagcattggaagcctttgagcaccagaattacccgttcgaagagcttgtcgataagcttgaattgacacgagatatgagccggaacccagtgtttgatgcgatgttagttgttcaaaataatgattacgagccattgcatcttcatgatttgcaaatgaagccggcacaagtttctcatctcgtttctaaattcgatttgacactacaggcatctgagggcgacggaaacattcatttcctttttgaatattcaaccgcattgttcgagaaaaccaccattgaacgctgggcatcgcatttaacaaatgtacttagcatcatcggcaaaaacccgaaggtgacactcaaccatatcgacatcctgacccaagaagagcggcaccagctgcttaatgagtttaacaccggggccgcgaaggcctacggagttcaaacaatcagtcaattgtttgagcagcaagctgcacgaacaccaaaagcttctgcacttgtcagcggagacaaaacactcacttatcaggagcttgacgagtggtccaatggaatcgcacgtgcattgcgcagccgaggtgttaagccggacacaccagtaggcatcatgatgcatcgttcgttcagtatgatagcatccatacttggtgtgtggaaagccggaggctgttacgttcccattgatcctgaatacccgaaagaacggaaacgctatatcctcagcgacagcggaacgaaactgctgatgacaataaatgaagcggatctgggagtacttgctgactttgaaggagagatcttgacgatagaaagcgtagaggaagacgacaaatcgccgctgccgcaaatgtcgtctgcccatcatttggcttatatcatttatacttcaggaacgacgggccgtccaaaaggggtaatggtcgagcataaagggattgctaacactcttcagtggcggcgaaacgcttatgcattcaacgagacagataccattctgcagctcttttctttctcatttgacggctttataactagtatgtttacaccgcttttgtcaggtgcaaaagccgttttgcttcatgaagaggaagcgaaggatattctggccattaagcatcagctgtctcgtcaacggattacacatatgattattgtgcctgttttatatcgagcgcttttggacgtagtgcagccggaagatgtaaagacgcttagagtcgtcacactggcgggagaagcggctgaccgcgaattgatcgcccgcagcttagctatatgtccgcataccgaactcgccaacgaatatggaccgacagaaaacagcgtggcgactaccgtcatgagacatatggaaaagcaggcatacgtaagcatcggccagccgattgacggaactcaagtgctgattttaaatagcaatcatcagcttcagccaatcggtgttgcgggagagctttgtatagcaggaacagggcttgcaagagggtacgttaatcttccagaactgacagagagagcattcacgcagaatccatttaaacccgaagcacgaatgtaccgaacaggagacgccgccagatggatggccgacggtacactcgaatatctcggaagaatcgatgatcaagtcaaaatcagaggataccgtgtagaaacgaaagaaattgaatcggtcatccggtgtataaagggtgtaaaagacgccgcagtagttgctcatgtaacagcgtcaggacaaaccgaattaagcgcttatgtggtgacaaaaccagggttgagcacaaatgctgtacgctcagaattacaaaacaagctgccggtgtttatgcaccctgcgtttattgaaaaactggactcacttccattgtcaccaaacggcaagctggatcgcggagcacttccaaaacctgtatacaaccacgaaggtgaacgtccattcctcccgccatccagcaaaatggaacaaatactggcagatatatggaaagaagtactgggggcagaaaagatcggaacagctgattcgttctttgaacttggcggagattcaatcaaagcgttacaggtatctgcgcggcttcaccggataggcaagcaaatggcagtgaaagatttgtttagccatccgaccattcaagaattggcagcttatatccgtgattcagatacaagttccagccaagctgcggttgagggagacgtacaatggtcgcctgttcaaaaatggtttctttctcaagatataaaagaaaaacaccattttaatcagtccgtaatgctgcatcgaagcacctctgtacaagaagacgcactgcgaaaaacgttaaaagcaataacgtgtcatcatgatgcgctgcgaatggtgtttacacagaatgaacaaggaaagtgggatcaatataatcggccgctcagtcattcggacgacgcgttgtacggccttcagatgattgatttgtcagctccggacggcactgatggaaatagaccgtatgaacctcttatcaagcgccatgtacttgatattcagcagaaaatggatttgaagaatggtccgctgctgcaagccggtcttttccacacaattgacggtgatttcttatttttatctgctcatcacctcgtcgttgacggcatctcatggcgggttctgcttgaagatttggctttagggtatcgccaagctgctggcggggaggatatcaaactgccgcctaaaacaagctcgtttaaagcgtatgcgaaaaagctctctgactacgctgaaagccagcagctaatgaaacagctcaagtattggcgcgaagccgaagagtatcaaacagaggcattgccttttgatcaaatcgatggaactagagcacacgagggacaacggtccacaatttcgtttaccttaaacgataaagagacagcagcactcttaaaagacgccaacagcgcatataacactgatacgcaggacatgctgctcgcttctgtcattcttgcgctgcgccattggaccaatcaatccgccttcaaactatcattagagggccacgggcgagaggatgtattaaaaggaatagatgtgagccggacgattggatggtttaccgccatttatccgttattgattaaactgaacgcagacttgccagattcggaagaaagcatggttcatgtgctaaaaacaacaaaagatacactgagacgtgtacctgacaaaggattcggctacggtgtcatcaaatatttgactccgcctggcaaaaaagacatcaatttcacaggtgcaccagaaatcagctttaattatcttggtcaatttgaaagcggccgcacagctgaagtacctgaggaggacgccttctcattctctccgctgggtgccggaggtgatatcagcacaacatggaaccgtgaacagtcgctggatatcagcgcaatcgctgcagaaggaaaattgactgtcaatatgacttatgacaatgcccgctttcagcgcaaaaccatcgaacagcttagcgaaacatgccgtcaatttttattacagctgatcgaacactgccagaacaaaagcgaaacagaaaagacgatcagtgattttgatgatcaagaactgaccgaggacgccctgcaagagatcgctgatatgctcagttttcactaatgaatccgtgaagaaaggtgcagacactatgaataccattaaaaaaatcaagaacatttatcctctgagtcatatgcaggaagggatgctgtttcattccttcctccgtaaagaggagggggcgtatgttgagcagtcgctcttcaccattaaaggaagcctcagctatgactggttccagcgcagcattcaagccattatcgaccgccatgatattttcagaaccgtgtttttgccgcacgtcccgcatttgtcgggacctcggcaagtcgtgatgacagaacgtgaattccatttgaacagcgaagacatttctcatctgccgacaaacgaccagaatgagtatattgaacgctttaaagagaaggacaagcaaaaaggctttgatctgcaaaaagacatgctgatgcggatttctctattcaaaacagctaaagatgagcatgtctgtatctggagtcaccatcacattttaatggacggatggtgcctaggtatcgttatgcaggaatttatgcaaatttatcaatcgattcatgcaggaaaaccgctttcattagaccctgtccgtccgtacagcacctatatttcatggctgacaaaccgagacaaagaaaaagcagcggcctactgggatacctatttaaaaaactacagcgctccatcacctctgcctcgtgtgtctgataaagaaacaaaagaaagttatcaccgtgaagatttgatattttcattaaataaaccactgacagacaagctgaaagagactgccaaacaacacggcgtcacgctcgctacccttattcaggcagtctggggtgtgatgctgcagcaatataaccgcacagacgacgttgtgtttggcgcagttgtatcaggaagaccgtcagaaatcccaggcgtggagcaaatgatagggttgtttatcaataccataccgattcgaattaaaacacaccaagacgaaacgtttcacgagctgctcatacgctgccagaaagaaatgctggaagctgagccgtttacctgccagcctttatttgatattcaggcaaacaccgcattaaaacaggaactgattgatcacattatcgtctttgaaaactatccgttacagcagaaaatcgccgattccgctgatcaaaccgattcaccgctgcaaatcgatcaagttcaagtatccgagcaatcaggatataactttaatcttgtcgttgctcctggcgaagagcttgtcatcaagttcagctataatgcattcgtttacgatgctgcctggatcagctgtatcaagaggcaatttacgcaagcgcttagcacagctgcacagcaccctcatatgccaattgctgatttttcttttcttgatgcaacagaaaaagagcagattgtcacacagttcaacaatacggccacggaggccccaaagaatcatacaattatcgatttatttcgcgaacaagcagaaaagacgccagaccataccgcacttgtgtatggcaatatgtctatttcgtataaagagcttgataaacgctctaatgcgctcgccagagagttaattcaaaagggatttcggaaaaacgagacagccggaatattggctgcacattctcccgaattcatgatcagtgtgcttgccgtattaaaagcagggggagcatacctcccgcttgatgcggagcttccgcctgaacgagtcagctttatgcttgaggaaacgcaggcaaaaatgctgattgttcaaaagggattggagcaaaacgctgcgttctcaggaacatgtatcatttcagatgcgcagggattgatggaagagaacgatatccctattaatatcagctccagcccggatgatcttgcgtacatcatgtatacctcaggatcaacaggccggccgaaaggggtcatgatcacgaatcgcaatgtcgtgtcccttgtcagaaacagcaattacacgtctgcgtccggtgatgaccggtttattatgactggatctatcagctttgacgccgtcacctttgaaatgttcggggcacttttaaatggcgcaagccttcatatcattgataaatcgacaatgctgacacctgatcggtttggagcgtatttgcttgaaaatgacattacagtgctatttttaacgacagctctttttaatcagctggcacaggtacgagctgacatgtttcgcggactccatacgttatatgtcggaggagaagcactctctcctgccctgatgaatgccgtcagacacgcctgtccagatctcgcgcttcataatatttacgggccaacggaaaacacgactttttcaaccttttttgaaatgaagagagactatgcggggccgattccgattggaaaaccaatcagtaatagcaccgcttacatcttagatacaaaaggacgtcttttgccaataggcgttcccggcgagctttgtgttggcggtgatggagtcgctaaaggctatttgaacagagtagatctgacaaatgctgtgttttctcctcatcctttcttgcctggagaaagaatataccgtactggtgatttggcgcgctggctgcctgatggaaacttagaatacatcagcagaattgacaggcaaatgaaaatccgcggaaaacgaattgagcctgccgaaatagaagcgcgcctgttagaaatggaaggcgttcaagaagcagcagtgacattgagagaaaaagatggagaggcgcagctgtacactcattacgtcggtgatcacaaaaaaacagatacggattttcgcgccgatttggcgcgtgtgcttccagactatatgatcccgcagcactgggtgcgtgtggagcggatgccgcttaccggaaacggaaaaatagaccgcagcgcgctgcctattccagaaaataagcctgccaaacgacagaacatcatattgccaagaaacttggttgaagaagaattggcgaacatttggaagcaagtcctcggtgttaacacaatcagtattgatgatgacttctttgctattggcggacattcactaagagcactgcaagtcatacatacactaaaacatcagcagaacattgacataccgattgatttcttgttcgaacatccgacaatcgctcagcttgccgaaaaactttattctaaacagctgacagcagcaaatgaacagcatgtgatcaaactgaaccagcacggcgcgcaaaatcttttctgcttcccgccgatatcgggatttggcatttattttaaagaccttgctttattgctgaatgagaaggcagccgtatacgggtttcactttattgaacaagacacccgcattgaacaatatgttaattgcatgacggacatacagcctgagggcccatacgttttattaggctactctgcaggcggaaacctggcttttgaagtggcacaggctatggagcgcaaaggattagaagtcagcgacttcattatcgtggacgcttatctaaaagaacagcctttgcctatcgataccggtaatgacgaatctgcagcatatctgcctgaagcagtcagagaaaaggtgatgaagaaaaaaagaaactatcaggaatattgggcacaattgctgaatgaaggccacatcaaagcaagcattcatttcatcgaagctggaatccaccccgaaaccagcgggcatacaggcttaacgaaatgggaaggcgcctgcggaaactatagtgagtacacgggttttggcgctcataaagacatgctggaaggaacatatgctgaaaagaatgccgacatcatcctcgacattttagaaaagatcacttcaaatcaagtaatactgcacaaacgataaagcggattagcggacagaggccattctctgtccgtctttctttttgtatggccgtctgtgagctttaatgcggtagtttatcacagttaaattgctaacgcagtcaggcaccgtgtatgaaatctaacaatgcgctcatcgtcatcctcggcaccgtcaccctggatgctgtaggcataggcttggttatgccggtactgccgggcctcttgcgggatatcgtccattccgacagcatcgccagtcactatggcgtgctgctagcgctatatgcgttgatgcaatttctatgcgcacccgttctcggagcactgtccgaccgctttggccgccgcccagtcctgctcgcttcgctacttggagccactatcgactacgcgatcatggcgaccacacccgtcctgtggatcctctacgccggacgcatcgtggccggcatcaccggcgccacaggtgcggttgctggcgcctatatcgccgacatcaccgatggggaagatcgggctcgccacttcgggctcatgagcgcttgtttcggcgtgggtatggtggcaggccccgtggccgggggactgttgggcgccatctccttgcatgcaccattccttgcggcggcggtgctcaacggcctcaacctactactgggctgcttcctaatgcaggagtcgcataagggagagcgtcgaccgatgcccttgagagccttcaacccagtcagctccttccggtgggcgcggggcatgactatcgtcgccgcacttatgactgtcttctttatcatgcaactcgtaggacaggtgccggcagcgctctgggtcattttcggcgaggaccgctttcgctggagcgcgacgatgatcggcctgtcgcttgcggtattcggaatcttgcacgccctcgctcaagccttcgtcactggtcccgccaccaaacgtttcggcgagaagcaggccattatcgccggcatggcggccgacgcgctgggctacgtcttgctggcgttcgcgacgcgaggctggatggccttccccattatgattcttctcgcttccggcggcatcgggatgcccgcgttgcaggccatgctgtccaggcaggtagatgacgaccatcagggacagcttcaaggatcgctcgcggctcttaccagcctaacttcgatcattggaccgctgatcgtcacggcgatttatgccgcctcggcgagcacatggaacgggttggcatggattgtaggcgccgccctataccttgtctgcctccccgcgttgcgtcgcggtgcatggagccgggccacctcgacctgaatggaagccggcggcacctcgctaacggattcaccactccaagaattggagccaatcaattcttgcggagaactgtgaatgcgcaaaccaacccttggcagaacatatccatcgcgtccgccatctccagcagccgcacgcggcgcatctcgggcagcgttgggtcctggccacgggtgcgcatgatcgtgctcctgtcgttgaggacccggctaggctggcggggttgccttactggttagcagaatgaatcaccgatacgcgagcgaacgtgaagcgactgctgctgcaaaacgtctgcgacctgagcaacaacatgaatggtcttcggtttccgtgtttcgtaaagtctggaaacgcggaagtcagcgccctgcaccattatgttccggatctgcatcgcaggatgctgctggctaccctgtggaacacctacatctgtattaacgaagcgctggcattgaccctgagtgatttttctctggtcccgccgcatccataccgccagttgtttaccctcacaacgttccagtaaccgggcatgttcatcatcagtaacccgtatcgtgagcatcctctctcgtttcatcggtatcattacccccatgaacagaaatcccccttacacggaggcatcagtgaccaaacaggaaaaaaccgcccttaacatggcccgctttatcagaagccagacattaacgcttctggagaaactcaacgagctggacgcggatgaacaggcagacatctgtgaatcgcttcacgaccacgctgatgagctttaccgcagaattcgcccttcccggtcgatatgaacagcttatttacataattcacgttattggtagttataaatgaaattcctaatatcggttatgaagtgaaattgaatttctacttgatctttctctctatttttgtaaaataaaattaagaatatttaaatattcaatgattcatttttgcagaaatcggaggaagaagaatatatgaaaacatttaacatttctcaacaagatccccccatattgttgtataagtgatgaaatactgaatttaaaacttagtttatatgtggtaaaatgttttaatcaagtttaggaggaattaattatgaagtgtaatgaataatgaatgtaacagggttcaattaaaagagggaagcgtatcattaaccctataaactacgtctgccctcattattggagggtgaaatgtgaatacatcctattcacaatcgaatttacgacacaaccaaattttaatttggctttgcattttatctttttttagcgtattaaatgaaatggttttgaacgtctcattacctgatattgcaaatgattttaataaaccacctgcgagtacaaactgggtgaacacagcctttatgttaaccttttccattggaacagctgtatatggaaagctatctgatcaattaggcatcaaaaggttactcctatttggaattataataaattgtttcgggtcggtaattgggtttgttggccattctttcttttccttacttattatggctcgttttattcaaggggctggtgcagctgcatttccagcactcgtaatggttgtagttgcgcgctatattccaaaggaaaataggggtaaagcatttggtcttattggatcgatagtagccatgggagaaggagtcggtccagcgattggtggaatgatagcccattatattcattggtcctatcttctactcattcctatgataacaattatcactgttccgtttcttatgaaattattaaagaaagaagtaaggataaaaggtcattttgatatcaaaggaattatactaatgtctgtaggcattgtattttttatgttgtttacaacatcatatagcatttcttttcttatcgttagcgtgctgtcattcctgatatttgtaaaacatatcaggaaagtaacagatccttttgttgatcccggattagggaaaaatataccttttatgattggagttctttgtgggggaattatatttggaacagtagcagggtttgtctctatggttccttatatgatgaaagatgttcaccagctaagtactgccgaaatcggaagtgtaattattttccctggaacaatgagtgtcattattttcggctacattggtgggatacttgttgatagaagaggtcctttatacgtgttaaacatcggagttacatttctttctgttagctttttaactgcttcctttcttttagaaacaacatcatggttcatgacaattataatcgtatttgttttaggtgggctttcgttcaccaaaacagttatatcaacaattgtttcaagtagcttgaaacagcaggaagctggtgctggaatgagtttgcttaactttaccagctttttatcagagggaacaggtattgcaattgtaggtggtttattatccatacccttacttgatcaaaggttgttacctatggaagttgatcagtcaacttatctgtatagtaatttgttattacttttttcaggaatcattgtcattagttggctggttaccttgaatgtatataaacattctcaaagggatttctaaatcgttaagggatcaactttgggagagagttcaaaattgatcctttttttataacaggaattgggcatcaaataaaacgaaaggctcagtcgaaagactgggcctttcgttttatctgttgtttgtcggtgaacgctctcctgagtaggacaaatccgccgggagcggatttgaacgttgcgaagcaacggcccggagggtggcgggcaggacgcccgccataaactgccaggcatcaaattaagcagaaggccatcctgacggatggcctttttgcgtttctacaaactcttcctgtcgtcatatctacaattctacacagcccagtccagactattcggcactgaaattatgggtgaagtggtcaagacctcactaggcaccttaaaaatagcgcaccctgaagaagatttatttgaggtagcccttgcctacctagcttccaagaaagatatcctaacagcacaagagcggaaagatgttttgttctacatccagaacaacctctgctaaaattcctgaaaaattttgcaaaaagttgttgactttatctacaaggtgtggcataatgtgtggaattgtgagcggataacaattaagctaattctatggtaaaagcattcctgaacccaatatccttatttttagtggacaaggccttgttctcatatggttgcttgagccagtgccttacaaggctcttccgctttggcaggctgttcaaaattatttattagagcaactcaaggaactaggcggagatccaaaagcaaccgatgcagcacgtgtttttcggattgctgggagcgtcaatagtaagaatggagcggaagtaagagcggaatatcggcacgattacagatatgagttaaggcagattcaatttgattaccttccagaactcaatgaggttattaatcccgctccacaaaagaaaaaacgggggcgtaaaaagaaagtagttcagttattcaatacctacaaactccattacgctcgcctattggatatagtgaaattggtggaactacgaaattatgaggtaactggatacagggaaatcatttgctttttataccgttattggttgtgctgttacacgaacgaccctgtagaggctttaaatcaaacacagacacttaatttacagttcactgagcctttacccttaaaagaggttgaaagggctacacggagcgcagaaaaggcgtgggaagcacgaaataacgaagaggctaaccggattgcaatcgaaaaaggatatcccagtgctggatacaatattagcaataaaaagttgattgaatggctagatatcacaccagaagaacagaagcatttacagacgattatagacgctaatgagaaacggagaagaaagcgggaaagggataggatttatcaagaacaaaaacgtcgtgagcggggagatatgacccgacaggagtatattaagcaacaacaggataaaacagatgataaattatttaaattgcaggagttattagaacagaatcccaaaatctcaaaaattaaattagcaaaaatacttggtgtagataaatcgcacttatacagactgctgaaacaactataactggaaaaaattagtgtctcatggttcgtcgcccttatattatgggcgttagcctgcttgctaattggataggtgttattgtcatttcaacgtcggacgttttggtagatgaacgtcggacgttatttgcttcaatagattgttgatgtattaagggttgcagtgaatcgacaagcaaaaagttatgacgttgtgaaaaaattgaatagaaaattggaaattacgtcggacgttctaacttaaaaaccctgttatatcaatgatttaaaaggaaattaacgtcataaaagacctttctgcaacaaaagtttttctggaagagttgaggttattttataggtattatggacttttgtagactttttgtgtactttttgtggactccacactcgctggtatcgtgttattttttaattgagatatgaatatggaaattaaacgttttaggcgttggtttggtgatgacaaaaaaataagagtacccgctcacaacggatactctttcgagaaatgtacgaaacgctataaataaaaaataactagatacatttacattgtatcacgtttcgtacatttctccaataacaaattgattggaggaatgcaaagtgaataatgaaccagtaaaacgtggtaagaagaacagatgggaattaaacctacctataatgacttatgtagtagctgatgattggattgataaactaggacacgaaacgtttactttatggttgaggttccatacttgggtagatagagaagatgaactccgagattatgatcgcatacctagaagttttgagaacatatataaaaagacactaggaatctcaaaaagtaagttttatagattgataaaacctttatgggaatatggattaatagacatcatagaatacgaagaatctaaccgtaattctactaaacctaaaaatataattgtttatgagtatcctttacacgaaatagaaagaaagtataaaccactagaaaaattaagagattgggataaagactataattccgtttctaaagaattaggtaaaacaggtggtagaccaaggaaaaaagatagtgaagaagaacccgaaaagaaacccgaagaagtaactaaaaagaaacgtaaatataagttaaaaagagttatccacaacggtttcaaaaatgaaacggtggagggtttcaaaaatgaaacggtggagggtttcaaaaatgaaacggtgaccgtttcaaaaataaaacccaataattattcaaatatctttaataacttatcaaatatttctactaatgtttcaaataatttattaattgatgatgatgaggaaatcgaaaatgaaccaactggtcgtacaataaataggtcattacttttttcacaagaagatattaaacaggcctatcaatttattaatagattttcagttatacagttacgtgaaaactttagctttgataaacactttgaagaacggttggtatgttatttatggaaagcagggatttctactttttacacgcacgaaatcagtaaaatgataaaaaaaatagcagactatgaaaaatctaaaaaaggtagattaaacccaatacgtgaccgagccttatatatggtaaatggtcttgtaatgaatagagcttcttcccaaagtgaacatgctacttataaactaaaccaatataaaaaacagaaggaacaggaaaaacaacaacaggagcaacaaagatcaagagtaccgttctataattggttggaggaaagagaagaacaaaccgaaggtcaactacccaccacttaaagcctaacggcttttgaagtggggcttgtaaaaagccctagttgactaccccaagtctttcgaggactacgttggaaaggtcatgacacctacaaatgctcctctagttcgtagccactgtcgttgatggttaaaagtcctgatgggtagggacggtgctgtcaacatcacaagcccttccaacatgggggaagaggaagaacactccgagaaaggagggggctgtcgtacacgccttgttcgtgtacgtgatttttaacacttttatctctaatataatctctccttgagttagcagagactaagaataaaacacattaggattttttatctacataaggaggttcaatacatgcctactatttcgtttaagggaaagtcttttgtacaaaatcatcacttgactgtaaaatatcatgaattgatcccagaaccagaaaaaagtctgaccgataaagttagtcttcatgacaatcttatcattcatggggacaatttaaaggcgttgaaagctctactacctacatatgctggtaagatagattgcatctatattgacccaccatacaatactggaactgaaaaatggatttataatgataatgtcaactccccaatgattagggaatggcttggaaaagtggtagacaaagaagacttatcccgacatgataagtggctttgtatgatgatgccgaggttaaaactgttgaaagagttgttgtcagaagacggagtgatatttgtaagcattgactacaatgaaatacaccatcttacgtgccttatgaacgaaatattcggtgaggagaattttcgtgacgctattatcattcgtagaggagtaaaaaatgttcaagcgcaatttgacacaattgattctctttcaaatggttatgagtctattttggtttacactaaacagccatctcgacgatttaataaggtttatgaagatgtagaagaaaagcctggtagttggaataatcattggagaggtacagaccgtaaaactatgagatatgaattatttggggttactccgacagaaggtcaatggagatgggggaaagaacgtagtctccaggctattgaaaactatcaaatgatgttagatgaacttagacaaaaaggcattactaatccaactcaagaggatattgataaatggtatcttgaatatgtagaaaataatggggaagatattgacttgttacgacaaaatgataatggcacgattgagcactttgttccaccgactagcaaaaagttgttaagtaatgcctggtttgacttaaaacccaacggttctagtcaattaaagaagatatttggaaggaaggttttcgataaccctaaatcaattgatttggtaaaaagactaatacaatttgcgactgaaaacaaagaagcgattgtacttgactcatttgcagggagtggcactactgctcatgcagtattatcgcttaacaaacaagatggagggaatcgtcgtttcatccttattgagatggaagaatatgcacatgagattaccgcagaacgcggatctttatcgatttgcatgcaagctaattcggtggaaacgaggtcatcatttccttccgaaaaaacggttgcatttaaatcttacatatgtaatactttcaaagactacatttgtaagatttgatgtttgagtcggctgaaagatcgtacgtaccaattattgtttcgtgattgttcaagccataacactgtagggatagtggaaagagtgcttcatctggttacgatcaatcaaatattcaaacggagggagacgattttgatgaaaccagtaacgttatacgatgtcgcagagtatgccggtgtctcttatcagaccgtttcccgcgtggtgaaccaggccagccacgtttctgcgaaaacgcgggaaaaagtggaagcggcgatggcggagctgaattacattcccaaccgcgtggcacaacaactggcgggcaaacagtcgttgctgattggcgttgccacctccagtctggccctgcacgcgccgtcgcaaattgtcgcggcgattaaatctcgcgccgatcaactgggtgccagcgtggtggtgtcgatggtagaacgaagcggcgtcgaagcctgtaaaacggcggtgcacaatcttctcgcgcaacgcgtcagtgggctgatcattaactatccgctggatgaccaggatgccattgctgtggaagctgcctgcactaatgttccggcgttatttcttgatgtctctgaccagacacccatcaacagtattattttctcccatgaagacggtacgcgactgggcgtggagcatctggtcgcattgggtcaccagcaaatcgcgctgttagcgggcccattaagttctgtctcggcgcgtctgcgtctggctggctggcataaatatctcactcgcaatcaaattcagccgatagcggaacgggaaggcgactggagtgccatgtccggttttcaacaaaccatgcaaatgctgaatgagggcatcgttcccactgcgatgctggttgccaacgatcagatggcgctgggcgcaatgcgcgccattaccgagtccgggctgcgcgttggtgcggatatctcggtagtgggatacgacgataccgaagacagctcatgttatatcccgccgttaaccaccatcaaacaggattttcgcctgctggggcaaaccagcgtggaccgcttgctgcaactctctcagggccaggcggtgaagggcaatcagctgttgcccgtctcactggtgaaaagaaaaaccaccctggcgcccaatacgcaaaccgcctctccccgcgcgttggccgattcattaatgcagctggcacgacaggtttcccgactggaaagcgggcagtgagcgcaacgcaattaatgtgagttaggatcctgcctcgcgcgtttcggtgatgacggtgaaaacctctgacacatgcagctcccggagacggtcacagcttgtctgtaagcggatgccgggagcagacaagcccgtcagggcgcgtcagcgggtgttggcgggtgtcggggcgcagccatgacccagtcacgtagcgatagcggagtgtatactggcttaactatgcggcatcagagcagattgtactgagagtgcaccatatgcggtgtgaaataccgcacagatgcgtaaggagaaaataccgcatcaggcgctcttccgcttcctcgctcactgactcgctgcgctcggtcgttcggctgcggcgagcggtatcagctcactcaaaggcggtaatacggttatccacagaatcaggggataacgcaggaaagaacatgtgagcaaaaggccagcaaaaggccaggaaccgtaaaaaggccgcgttgctggcgtttttccataggctccgcccccctgacgagcatcacaaaaatcgacgctcaagtcagaggtggcgaaacccgacaggactataaagataccaggcgtttccccctggaagctccctcgtgcgctctcctgttccgaccctgccgcttaccggatacctgtccgcctttctcccttcgggaagcgtggcgctttctcatagctcacgctgtaggtatctcagttcggtgtaggtcgttcgctccaagctgggctgtgtgcacgaaccccccgttcagcccgaccgctgcgccttatccggtaactatcgtcttgagtccaacccggtaagacacgacttatcgccactggcagcagccactggtaacaggattagcagagcgaggtatgtaggcggtgctacagagttcttgaagtggtggcctaactacggctacactagaaggacagtatttggtatctgcgctctgctgaagccagttaccttcggaaaaagagttggtagctcttgatccggcaaacaaaccaccgctggtagcggtggtttttttgtttgcaagcagcagattacgcgcagaaaaaaaggatctcaagaagatcctttgatcttttctacggggtctgacgctcagtggaacgaaaactcacgttaagggattttggtcatgagattatcaaaaaggatcttcacctagatccttttaaattaaaaatgaagttttaaatcaatctaaagtatatatgagtaaacttggtctgacagttaccaatgcttaatcagtgaggcacctatctcagcgatctgtctatttcgttcatccatagttgcctgactccccgtcgtgtagataactacgatacgggagggcttaccatctggccccagtgctgcaatgataccgcgagacccacgctcaccggctccagatttatcagcaataaaccagccagccggaagggccgagcgcagaagtggtcctgcaactttatccgcctccatccagtctattaattgttgccgggaagctagagtaagtagttcgccagttaatagtttgcgcaacgttgttgccattgctgcaggcatcgtggtgtcacgctcgtcgtttggtatggcttcattcagctccggttcccaacgatcaaggcgagttacatgatcccccatgttgtgcaaaaaagcggttagctccttcggtcctccgatcgttgtcagaagtaagttggccgcagtgttatcactcatggttatggcagcactgcataattctcttactgtcatgccatccgtaagatgcttttctgtgactggtgagtactcaaccaagtcattctgagaatagtgtatgcggcgaccgagttgctcttgcccggcgtcaacacgggataataccgcgccacatagcagaactttaaaagtgctcatcattggaaaacgttcttcggggcgaaaactctcaaggatcttaccgctgttgagatccagttcgatgtaacccactcgtgcacccaactgatcttcagcatcttttactttcaccagcgtttctgggtgagcaaaaacaggaaggcaaaatgccgcaaaaaagggaataagggcgacacggaaatgttgaatactcatactcttcctttttcaatattattgaagcatttatcagggttattgtctcatgagcggatacatatttgaatgtatttagaaaaataaacaaataggggttccgcgcacatttccccgaaaagtgccacctgacgtctaagaaaccattattatcatgacattaacctataaaaataggcgtatcacgaggccctttcgtcttcaagaattctcatgtttgacagcttatcatcgataagctcac

SEQ ID NO: 29 - DNA, 50705 bp, synthetic construct
  misc_feature 1..50705: note = Chimeric construct 2
  source 1..50705: mol_type = other DNA
atgtggcccgggagacctgttttccaagagaaaacaggtttttttatgtctgtaataacgctttgtcgaaccttccaacaattagaagaatgatgcacaaaagaaaattagtccgattaaaaagtagtgtataagaccttatgtaaaacaatacttttatcactttatatccggaaatttgataaaaaaagaaacgaaaaataaagaaataatactatattcaaaaaaaatgttataaaaatttaatgttttttattgtactttaaaaaatatccgttaatatagtgcatatatggattatatagtcatataatttcttttattgtcatttttctgcttttttctacattttcttatcctcttattatgagaactggagggaatccgttgagcgaacatacttattctttaacccatgcccaaaggagagtgtggtttaccgaactgctggagccagataccagcatttgcaatcttacagcttgtgtgaaatttaaaggcaatattgagcttgatactctggagggagcactgaatcattccatctcccgcaacgacgccattagatttcagctgttagaaggagaagagcttgagcctcgattgcaccttactgaatataaatattatccacttagaataattgatttttcaaatgttgaaatgatagaaatagagcaatggattcaggatcaagcgagcattccatttaaactgttcaactcgcctctttttcaattttacctccttagaattgactctcatgaagtttggctatttgcgaaattccatcatatcataatggatggaatctctttaaatgtgatgggaaatcaaattatagatctttatcaaaaaatgaaaaagaaagatcctttacctgatcagccggaaccttcttacttgagctacatcgaaaaagagagtcaatatctacaatctccacggtttgcaaaggaccgtttattttggacgcaaacctttgagcacccgttggaataccactcgttagccgaccagacgtccttacaaaaacagagcacatctgcatccagagacaccatcattctttcacctgatctagagcaaacgattcgaatcttctgcgaagaacacaagatcaatatcatttccttatttatggcttcattttacatatgcatcagccgaatcacttctaaaaaagatcttgccattggcacctactatggcaacagaggttcaaaggctgaaaaagaaatgctcggcatgttcgttagttcccttccaatcagaataacggttgatcctgacacagattttctttcctttgtccgcacaataggcagggaacagctttctgttatgcgtcatcaacggtttccttataatttgcttgtaaatgaattaagaaatgaacagaaggatttacacaaccttatcggtatatctatgcagtatcagccacttcagtggcacaatgcagatgattttgactatgaaacagcgctttatttcagcggatacaccgcgaacgaactttcagttcaaatacaagaacggatagacaatggaaccattcaattaaatttcgactatcaaaataccttgttttctcttgaggatattaaacgaatacaatctcatctgcttaccatactggaaaacgcccttaaacatccgcacagctttataagagaattagatatgacgaatacaagagaaaagcaaaaattgttgtatgagtttaacaagacggccgtggcggcccctaaagctttcaccctgcatgggctgtttgagcgacaggcagctttcacaccggagcggctggccattcgcttttcaggcggttcgctgacatacgctgagcttgatatgtacgccagccggctggctgcgcaccttgcggcacgcggcgtcacaaacgaaagtatcgtcggtgtcctgtctgaacgctcacctgacatgctgatcgctgtccttgctgtattgaaggccggcggggcgtatttgccgcttgatcctgcgtatccaaaggagcggctgagctacatgctgaaagacagcggggcatcgctcttgctgacacagccgggatgctccgcaccaaacttttctggcgaaacgcttgaagtggacatgacatctcttgcgagcgaaaaagcagaaaaccatgagtttactcctgctgacggcggatctctcgcctatgtcatctatacatcgggctctaccgggcagccgaaaggagtggccgttgagcaccgtcaggctgtttcctttctgaccggcatgcagcaccagtttccgctttcggaagatgacattgtcatggtgaaaacctctttttcctttgatgcgtctgtgtggcagctgttttggtggtcgctttccggtgcttcggcgtatctgcttccgcccggctgggagaaagactccgcattgatcgtacaagccattcatcaggaaaacgtgacaacggctcattttattccggctatgctgaacagctttctcgatcaagcggaaatcgaaaggctgagtgacaggacaagcctaaagcgtgtattcgccggaggtgaaccgcttgcgccgcgtacggcagcccgttttgcttctgtattgccgcaggtatcattaatccatggttacgggccgacagaagcaacggtagacgcggcattttacgtattggatccagaacgggacagggatcgtttgcggattccgattgggaagcccgtacctggtgcgcgtttgtatgttttagatccgcatttagccgtacagccttccggtgtcgccggcgaactgtacattgccggagcgggtgttgccagaggttatttgaatcggccggcattaacggaggagcgttttcttgaagacccgttttacccgggggaacgcatgtacaaaaccggggatgtggcgcgctggctccctgacgggaatgttgaattcctcgggcgcacggatgatcaggtaaaaatccgcggctaccggattgagccgggagaaattgaagcggcactaagaagcatagaaggcgtaagagaggcggctgttaccgtacggacagacagcggggagccggaattatgcgcttatgtagaagggctccaaagaaacgaagtgcgtgcacagcttgagagactgttgccgggctacatggtcccagcctatatgatagagatggaacagtggccggttacgccaagcggaaagctcgaccgaaacgccctgccagctcctggcggagcggcagatgcggagacctacacggcgccgagaaacgtgactgagatgaagctttctcagctgtgggaggacgtgctgaaaaatggccctgtcgggattcacgacaacttttttgaccgcgggggacattccttaaaagcaacggcgcttgtctcacggatcgccaaagaattcgatgtacaggtgccgctaaaagatgtgtttgcccatccgacagtagaaggactggctaccgttatccgtgaaggaacggacagtccatatgaagcgattaagcccgctgaaaaacaggaaacctatccggtttcctctgcccaaaagcggatttatgtccttcagcagctggaggacggagggacaggctacaatatgccggctgtgttagagctcgaagggaagctcaaccctgaaaggatggagagagctttcaaagagctgatcaagcgccacgagtcgcttcggacctccttcgaacaggacgcaggaggcgatccggtgcagcgcatccatgacgaggtgccgtttacgttacagactacagttctcggcgaacgaaccgaacaggaggccgcagccgcatttatcaaaccgtttgatctcagccaagcgccgctgttccgtgcccaaatcgtaaagatatcagatgagcggcacctgttgctggttgatatgcatcacatcatttcagacggtgtttccgtcaacattctgattcgggaattcggcgagctgtacaataatcggaatcttccggcactgcgcattcaatataaagattatgccgtatggcgagaaggattcaaaacaggagacgcgtacaaaacgcaagaggcgtactggctgaagcagctcgagggcgagctgcctgtgctggatcttccggctgatcatgcccgcccgccggtgcgaagcttcgcgggtgacaaggtctcatttacgctggatcaagaggttgcatcaggccttcacaagctggcacgtgaaaacggaagcacactgtacatggtgcttcttgcggcttacaccgcgttcttgtcacgcttaagcggacaggaagatatcatcgtcggctcgccaattgccggccggccgcacaaggatcttgagccgatactcggcatgtttgtgaacacgctggcgcttcggacgcgcccggagggcgggaagccattcgtacagtatttgcaggaagtgcgtgagacagcattggaagcctttgagcaccaggattacccgttcgaagagcttgtcgataagcttgaattgacacgagatatgagccggaacccagtgtttgatgcgatgtttatccttcaaaatgtggaaaaacaagacatagatctgagagaaataaaagtccggcctgccaatttcgcacatcacatttccttatttgatatcacattaatagctacggaaataagtggatctatttgctgcgaaatggaatttagtacagaagtattcctgaaagctacgattgaacgctgggctgatcattttatcgaatttctgcatgaggcactttcaactcctgaaacaagccttgcacaaataaacatacttagtgataaagaaaaacaaaaaatagtctttgaatttaacaaaacggccgttgaggccgctcaaaaagatattccttttcatcgcatatttgaagcgaaagctgaagaaaatccagaacatatagctgttattgataacgaaacagagattagctatcgccttctaaatgaaagagccaatcgtctggcacgaacattgcaaaacagaaaaggaccgaagccaactgtggctgttttagccaagcggtccatcgatgcaattgttggagttctggcagtgatgaaagctggcggagtgtatatcccaatcgatgcacattatccaaaagctcgtattgaatacattcttcgtgatagcggggcagatattcttcttttacagagagagttgaagcatttgatttcgaactcgcctgaatctgagatgtctcacatcttccttgacgatgagggctcttttgaagaaagtaactgcaaccttaacttatctcctgctcctgaagagccggtatatatcatttatacgtcaggaacgacgggtgcgcctaaaggtgttattgtcacctatcagaactttactcatgctgctcttgcttggcgtcaaatttatgaactggatcggaagcctgtcagactgcttcaaatcgcgagcttttcattcgatgtcttctcaggagatttggcgagaacattgaccaacggcgggactctaatcgtttgcccagatgaaacacggctggaacctgctgaaatatataaaatcattaaatctcagagaatcacggtgatggagtcgacaccggctctcattatcccggtgatggagtatgtataccgtaaccagttcaagcttcctgacttagacatactgattcttggttccgacatggtgaaagctcaagatttcaaaacattgacagatcgctttggccaaagcatgcgcatcattaatagctatggtgtcacagaggcaaccattgattcgagtttctatgaaaccagtatgggtggagagtgtacgggagataacgtaccaatcggcagcccgctgccgaatgtacacatgtacgtactcagccagactgatcaaattcagccgatcggtgttgccggcgagctgtgcatcggcggggcaggtgttgcgaaaggctatcatcataaacctgacttaacgcaaatgaaatttacagaaaatccatttgtctctggagaaaggctgtacagaaccggtgatcgagcatgctggcttccaaacggaacgatccggcttcttggccgaatggattatcaagtaaagataaatggatacagaattgaaacagaagaaattgaaagtgttctgcttcaaacggggcttgtcagagaagctgctgttgccgttcagcatgataaaaatggacaggctggtttggcagcatatattgtgccttcagacgtcaatacgaatgctctccgtgctgctttaacaaaggaactgccagcgtatatgattcctgcatatctgattcctttagtaaacatgccgctgaccctaaacggaaagctggacagaaatgccttgccggctccaaataatgtgttatcgcgtccatataccgcaccagttaacgacttacaaaaaacgatggcgtatatatgggaagatgtactgagcatgtcacgagtcggcattcacgattccttttttgagcttggcggagactcaattaaagcattacaagtggcagcacgtctggcagctgaaggctggagcatgacaatacgcgacttattccgttattcaacgattcaggaactatgcggacatatcacaccattggcatctcaagcggaccagggacctgcggaaggtgaagctgaactcaccccgattcagcgaagatttttcggacaggtacatgcttttcactatcattacaaccagtccgtcatgcttttcagtgaaaaaggattcaatgctaacgcgcttcatctagcgctgcgtaaaataaccgagcatcatgatgccattcgcatgattttccaacgtgaccaaaacggccatgtcattcagtttaatcgcggaatcaatcacaaggatcatgaactgtttggcctttatatttcagattggacaaaagcatcgctggaaagggctcatcttgatgaaaaacttgccgctgaggaaaccgtcattcaaagcaaaatgaatgtagaaaaagggcccttactgcaagcaggtttgtttaaaacggcagaaggggatcatttgctgattgcacttcatcatcttgtgatagatggcgtttcttggagaattctgcttgaggatttagctgcagcatatcaacaggctttagaaaagaaagaaatccaattaccgccaaaaacggattcttatttatcctacgccgatggtcttacccaaatagctgaaagtaaacaattgctttcagagaaaacgtattggcaaacgattttagacgctcacactgcttttcttcctaaggacatagaaaatgtgccagacaaactccaaatgaacagcgacgcagcagcgtttgtactatccggggactggactgaaaaattgctgtttgaaacccagcaagcctatggtactgatgccaacgaacttttgcttacggctttaggaatggcgctttctgaatggactgggcatgaccaaatcgtgatcagcactgagggacacggtagagaagggcatgtgccaaacattgatatttcaaggacagttggatggtttacctccatttatcctattctgctagacatgggtattcccgagcctttcgaggatcagctcgcataccgaattaagacgacaaaagatatgctgagaagagtaccgaacaaaggaactggatacggattgttaacacacataggagaactgcggcataaagagcctgaggtcagctttaattatctcggtcaatttagcgaagagaaggaagttgaaacgtttcaattatcatattaccagccccgttacgaaatagcgggtgagagagaacgagagtatgagctggacatcaatgctctcattacggacggacggcttcacgtaaaagcggtatacacccaagtgttcagcaaacactcaattgagtgctttatggatcgttttcacaggcatcttatcgagacgattgagcattgttcgcagaaaaaagcacgcgaaaaaacattgagcgatttcagcaataaagaattaacgttgtctgcattatctagcatcgaagatctcgtgaaagatctttaacttttgaaaaggtgtgtggaattgatggcacaatcggcacaaattcaagatatttatccgttatcgcacatgcaggaaggaatgctgtttcattcactaatggatttcagctcgaaagcatatatcgaacagacctcgtttacgatcacagggaatctatgcgtcgactcgtttcaaaagagcttaaaccttcttgtttctagatatgatattttcagaacgattttcattaaagaagtaccagatcttacaggtccgcagcaggtagttctatcaaaccgtgaattgacagtatatagagaagatatttctcgcctggctgatcaagaacagcagacgctgattgatgcttttatgactaaggatcgggaaaaaggatttgatttgcaaaaagatcctttaatgcgtcttgccctttttgatagaggagacagccaatatacatgtgtctggacacatcaccatatcatcatggatgggtggtgtctcggcattattcttaaagagtttttcagcatgtatgattcgctcaaaaataactcacctgtacagcttggcagcacggtgccgtacagccgttatattgaatggctcggagaacaagatcaagaagagactgctgcctactggagcgaatatttgaaggagtacggcaatactgcttctattccccgaataaagcgccgcacggcagacgggaattataaagccgaccaggtcagcttttcattagcgccggatatggttgagaaactgacagaggctgcccaaaactggggagtgacattaaacacgctgtttatgagtatttggggcgtgctgctccatcgatataatgctgcagatgatgccgtttttggctccgtcatttcgggacgcccgtcagcgattgacgggattgaatcaatggtcggtttgtttatcaatactgttccagtgcgaatccgatctgcggaaggcataacattttcttcgctggtcaaagccgtgcaggaggatattttatcatctgaacagcatgggtattatccgctttatgagattcaaaaccatagtccattgaagcaagggttgatcgatcatatttttgtttttgaaaattaccctgtacagcttcatcaggcattaagcgtggagagtgaaaatgacgaaggcgctctgaagctgagtgacatttcaatgtcggaacaaaccaattacgactttaatatcgttatcgttccgggagaatcattttatatcaaattcagctacaacgcagacgtttacgagcgggaggagatgctgaggattcaggggcatctaaagcaagcactggattgcattttgacaaatcccgatgttgccgtcagtgacatcaatatcgtgccgccggaggagcaacaggttatccaattgtttaacgaaacggcccgtccggccgtgaacaaaacgataccccaattgtttgaggaacaagctcacaaaacacctgaagctgctgcattgaaaatgggaaacgagtgctggacctatcgccagttacaagtaagagccaatcagattgcgcacgccctgatagaaaaaggcgttggatctggggatatcgttgctgtaatgatgggccggtcaatggaaatgcctgcagctctgcttgggatttggaaagcaggcggcgcttatatgccgcttgatccacattttccagcagaacgtctttcttttcttctgaaggacagtcaagcggctcaattgctgatagaagaagaccttatttccttgatccctccgtcctatgaaggaaatacgataacgatagaacatacagaaagttaccaaacagaagcgccaaatatgccgccaggtgatctagcctacttgatctatacgtcgggaacgacggggcgccctaaaggggttttagttgatcatcacggtattgccaatacattgcaatggagacgggaagagtatagcatgaccgaacaggatatatccctccatttgttttcgtacgtgtttgacggctgtgtaacgagcttatttaccccgcttttatctggtgcgtgcgtactgctgacaacagatgacgaagcgaaggatgtgctggcccttaagcgaaaaatagcccgttataaggtcagccacatgatcattgttccttccctgtacagggtgttattggaagtgatgactgctgacgatgcaaaaagtcttcgtattgtgacatttgcgggtgaagcggtcacgcctgatctgcttgagttgaatcaaataatttgtccttctgctgaactggcaaatgaatacgggcccacagaaaacagtgtggcaacaacaatattgcggcatctgaataaaaaagagaggatcacgatcggacacccgatcagaaacacaaaagtatttgttttgcacggaaatcaaatgcagccgatcggcgcggcgggtgaactgtgtatttccggcgcgggtcttgcgagaggatactacaaacagcaagagctgacacagaaagcattctccgatcatccattccttgaaggggagcgtttataccgaacaggtgatgcaggccgctttttgcctgatggaacgattgaatatattggacgttttgatgatcaagtgaaaattaggggttatcgtattgaactgagagagattgaaacagttcttcgacaagcaccgggggtaaaagaagcagcggtactggcccgtgatgtttctgctgaggaaaaggagctcgttgcttatatcgttccggaaaagggaaacagcctcccagatttgtatcagcatcttgccgggacattgccgtcctatatgatcccagcaagtattatcaacatcagccagatgccattaacatccagcggcaagcttgacaggtttgcgcttcctgaaccagaaaacaatacgagtgtcacatatatggcgccccgaaccttaatcgaagctgatctcgcacatatttgggaagatgtgctgaataaacagcacatcggcattcgtgatgatttctttcagttaggcggacagtccttaaaagcggccgcactggtatcaagaatacataaaaagcttaatgtcgagctgccgctcagtgaggtgttttcttatccgacggttgaaagcatggcggtcaaattgatgagcttaaaagaacacgcttttacacagattgaacctgcggatcaaagagatgtctatccgctgtctttctcgcaaaaacgattatatgctcttcatcagctggcagatgacagcacaggctacaacatgccagctgtacttgaattacgcggaaatctgaatcgccagcggttgagaagcgttctcacagaacttgtgaatcggcatgaagcattacggactgtttttgtgcttgacagagacgagcctgtgcagatcatttatccagagatggcttttgatctaaaagagcttgaaatggaatcagaacaaatgcttgagtctgcaatcgagacctttatcaaaccgttttatctatcatccggtccgctttttagagcatgtgtcattacaatgggcaataatcgcggctttttgctgctcgatatgcaccatattattgccgacggtgtctcgatgagcactcttgtccaagaatttactgacttatattgcggaaaagagttgccagctttaaacctgcattataaggattttgctgtttggcagcaagagaagcacccgaaagagctatacaaaaaacaggaggcctactggctcggtcagcttggcgggagtcttcctacactagaattaccgcttgataaaacaaggccgcgtctccctgatttcaggggtggaacaattgaagtcaacattgataaagacatggctgatgaactgcaccgtttaatggctgaaacgggaacaacattgtatatgattcttctggctgtctattctattttgttatctaagctaagcgggcaagaggatattgttgtcggttcgcctgctgccggaagaccgcacgctgatctggagcgcgtcatcggaatgttcgtcaatacattggcgatgcgcagcaagcccgagggccacaaaacgttcagctcctatttgcatgacattcgccacctggctctgaccgcttacgagcatcaggattatccttttgaggagctggcagataagctcgatacaaatcgagaggtaaatcgcaacccgctgttcgatgcgatgcttgtgcttcaaagcagtgaagatttccggttcgaagtgcctggtctgtcgatttcgtctgtcactcctaaacatgatatatctaaattcgatttaacattacatgctgaggagcatctgagtggaatacgctgccgttttgaatacagcactgctctttttgaagaagaaaccattacgcagtgggcatcctattttattgaattggtaaaaggggtaacggcggatactgagatgagaatttcgaacatgcaattgcttcctgctgcagagcgtaggttactccttgaaaaaatggggcaggccgccctggccccgagaaatgaaaacatagtaagcttatttgaaaagcaagtagctcagtatccggagcatatcgcagtggtgtgcggccattctcagcttacgtatcgagacctgaatgaaaaagccgagcgggcagctgctatgctgatcaaacaaggggtcagaactggcgatatcgtcggtctgatgctcgatcggtcacctgatatgatcattggcgttttatcgattttaaaagctggcggggcctatttgccgattgatcctgaatatcccaaggagcgtattagctttatgctcaatgacagcggagcaaaactgctgctgacagagcgcggtctaaacaaacctgcagactacaccgggcatattttgtatatcgatgaatgtgaaaacaactcaattccggctgatgtaaacattgaagaaatagtaacggatcagcccgcatacgtgatatacacatctggaacgactggtcagccaaagggagtcattgtcgagcaccgcaatgtgatcagtctcttgaagcatcaaaacctgccttttgaatttaaccatgaagacgtctggacgttatttcattcttattgctttgatttctctgtatgggagatgttcggtgcgttattgaacggaagtacattagtcgtggtctctaaagaaacagcccgtgacccccaagcattccgattattgttaaaaaaagagcgcgtcactgtactcaatcagaccccgactgctttttacggcttgatgcttgaagaccaaaatcatacagatcatttaaacatccgctatgtgatttttggcggcgaagccttacagcccggattgcttcaaagctggaatgaaaaatatcctcatactgatttgattaatatgtacggtattacagaaacaacggtccatgtaacattcaaaaaattgtccgcagcagacattgcaaaaaataaaagcaatatcggccggcctctttctactctgcaggctcatgtgatggatgcccatatgaacctgcagccgaccggagttccaggggagctgtatataggcggcgaaggtgtggcacggggatatctcaacagagatgagctgaccgctgaccgttttgtatccaatccttatcttccgggagacagattataccgaacaggagatcttgctaagcgcctgtcaaatggcgagctggaatacttaggccgcattgatgagcaggtgaaagtcagagggcaccgtattgagttaggcgaaatccaagcggcacttcttcagtatccaatgattaaagaggcggctgtcattaccagagcagacgagcaagggcaaacagctatatatgcatatatggtgataaaagatcaacaggctgcgaatatatcagacatccgaacttacctaaaaaacgccttgcctgactttatgctgcctgcccgtatgatacaaattgacagcatcccggtgactgttaatggaaagctcgatcagaaagccctgccagagcctgaaaaacaagcttatacagctgatgatatcagtcctagaaatgagattgaaacggtgatggctgaaatttgggaagagcttcttaatgtagatgagctgggtgtaagcgccaatttctttaagcttggcggagactctattaaagcgctgcaggtttgtgccagactgaagcagcgcggatttgaaacgacagtacgtgagatgtttgaacatcagactcttggtgaactgtccgcccgggttcgaaaagacgtacgcgccattgaccaaggcccggtcgaaggcgagattacttggacacctatccagcagtggtttttctcgcaatctctggaaagccatcattttaaccaatccgttatgatctaccgggctgaacgatttgatgaggctgcgcttagaaaagtactaaaaagccttgtgactcatcatgatgcactgagaatcgtatgccggcatgaagatggcaggcaagtgcagataaacagagggatagatctttcagatgaggagctatatgcacttgaactgtttgatgtaaaggatagcctaacagaagcccggaacacgattgaggaagcagccagccggatgcaagaacatattcgtttggaaaccggccccttacttcacgctggattgtttagaaccgagaatggtgaccatttatttctaacgattcatcacttagttgttgatgcggtttcttggcgcattttgtttgaggatttttcaacagcttacaaacaggcagtctcaggagaatctattaaactgccgcaaaaaacagattcatatttaacgtattcacaaagaatagctgactactctataagccgccaggtgcagcgcgaagcagcgtactgggatgagtgcgagaaccgtcacatccagcctattccaaaagacaatgacgcagcatctaacacattcaaagatacagaagtgattgattttgagctatctcgccatcacacagaattactattaacggctgcacataaagcttacagcacggagatgaatgatatccttctgacagctttaggtcttgctttgcagaaatggacgggaaataaccaatttaaaatcagcatggagggccatggaagggaatcatatcttgaggacatcgatattagcagaactgttggctggttcacctccatttatcctgtgtggcttgatatgagagattccgatcataaggacaaagaagagcggctgggccaccttattaaacagacaaaagatatgctgcaccgtataccgcataaaggcgcgggctacggcgtgctgaaatatatcagcaaaagatggggctctcagaaaaacagcccagaaatcagctttaattatttaggccagtttgatcaggatattcaatcaaatgcctttgaggtgtctgacatcaagccaggaaatgagatcagcccgaactgggagcgtccttatgcactggatatcagcggcgccgtttcttcggggtgcctgaacatgcacatcatctataacaggtttcaatttgaggaaaaaacaatccaaacattttccaggcattttaaacagactctggaaaacatcattgagcattgtaccggcaaagaaaaccaagagtggagcgcatctgatttcactgatgaagacttaacgcttgatgaattgagtgagatcatgggagccgtcaacaaactataggagaggagattcactgatgccgcagcaacctgaaatacaggatatataccctttgtcatttatgcaggaagggatgctttttcactcactgtatgatgaacagtcgagagcttattttgaacaggcttcttttacgatccatggacagcttgacttggagcgtttccaaaaaagtatggatgctgtttttgacaggtacgatatctttcgaacagcattcatctataaaaatgtagccaaacctcgtcaagtcgtgctcaagcaacgtcattgccctattcatattgaagatatttcccatctcaatgaaagggataaagaacattgtaccgaggcattcaaagagcaggacaaatccaaaggctttgatctccaaacggatgtactgatgagaatatctattttaaaatgggcgcctgatcattatgtctgtatctggagccaccatcatattttaatggatggctggtgtttaggcatcgtcattaaagactttctccatatttatcaagcgctgggtaaaggccagcttcctgatttgcctcccgtacagccgtacgggacgtatattaaatggctgatgcagcaagatcgtgaagaagcagctgagtactggaaaaagaggcttcagcatttcgaaaaatctacacccctgccgaaaagaacagatcaaattccgaatgggacactacagcagatcacgtttgccattcccgaaaaagaaaccgccgaattacagaaaatcgcagcagcttctggtgcgacactaaacactgttttccaagctttatgggggattatgcttcaaaaggtcaatcgcagcagcgatgctgtgttcggttcagttatatcaggcagaccttctgagctaaaagatgtggaaaacatggtcgggctttttatcaataccattcctattcgagcccaaagtgattctctgtctttttctgacctagtcaggagaatgcaaaaggacatgaatgaggcagaagcctatagttactttcccttgtatgatattcaggcgcagagtgctctaaagcaagagttgatcgatcatattatcgtctttgaaaatacacctacccagcaagagatcgaagagctgaatcaagcggggtcatttgatttctccgtcaaagattttgagatggaagaggtgaccaattatagttgcagtgtcaaagtgatcccaggccgtaccttgtacgttcggattcattttcagaccagcgcttatcaaccaagcatgatgtccgaaataaaagattatttgctgcacatggtctctgacgtcatctctgatccatctcttcctgtgtcaaagatgacgttgctagatgaggacaaaacacggaaaatcgtttctcaaaataacaggacggccagtgtggcccctgaagccccaaccctgcatgggctgtttgaacgacaggcggcagtcacaccggagcggctggccattcgcttttcaggcggttcgctgacatacgctgagcttgatatgtacgccagccggctggctgcgcaccttgcggcacgcggcgtcacaaacgaaagtatcgtcggtgtcctgtctgaacgctcacctgacatgctgatcgctgtccttgctgtattgaaggccggaggggcgtatttgccgcttgatcctgcgtatccaaaggagcggctgagctacatgctgaaagacagcggggcatcgctcttgctgacacagccgggatgctccgcaccaaacttttctggcgaaacgcttgaagtggacatgacatctcttgagtgtgaagaagtaaaacgtcatgtgtctgcttctgttagcgacggatctctcgcctatgtcatctatacatcgggctctaccgggcagccgaaaggagtggccgttgagcaccgccaggctgtttcctttctgaccggcatgcagcaccagtttcggctttcggaagatgacattgtcatggtgaaaacctctttttcctttgatgcgtctgtgtggcagctgttttggtgggctctttccggtgcttcggcgtatctgcttccgcccggctgggaaaaagactccgcattgatcgtacaagccattcatcaggaaaacgtgacaacggctcattttattccggctatgctgaacagctttctcgatcaagcggaaatcgaaaggctgagtgacaggacaagcctaaagcgtgtattcgccggaggtgaaccgcttgcgccgcgtacggcagcccgttttgcttctgtattgccgcaggtatcattaatccatggctacgggccgacagaagccacggtagacgcggcattttacgtgttagatccagaacgggacagagaccgtttgcggattccgattgggaagcccgtacctggtgcgcgtttgtatgttttagatccgcatttagccgtacagccttccggtgtcgccggcgaactatacattgccggagcgggtgttgccagaggttatttgaatcggccggcattaacggaggagcgttttcttgaagacccgttttacctgggggaacgcatgtacaaaaccggggatgtggcgcgctggctccctgacgggaatgttgaattcctcgggcgcacggatgatcaggtgaaaatccgcggctaccggattgagccgggagagattgaagcggcactaagaagcatagaaggcgtaagggaggcggccgttaccgtacggacagacagcggcgagccggaattatgcgcttatgtagaagggctccaaagaaacgaagtgcgtgcacagcttcagagactgttgccgggctacatggtcccagcctatatgatagaaatggaacagtggccggttacaccaagcggaaagctcgaccgaaacgccctgccagctcctggcggagcggcagatgcggagacctacacggcgccgagaaacgtgactgagatgaagctttctcagctgtgggaggacgtgctgaaaaatggccctgtcgggattcacgacaacttttttgaccgcgggggacattccttaaaagcaacggcgcttgtctcacggatcgccaaagaattcgatgtacaggtgccgctaaaagatgtgtttgcccatccgacggtagaaggactggctaccgttatccgtgaaggaacggacagtccatatgaagcgattaagcccgctgaaaaacaggaaacctatccggtttcctctgcccaaaagcggatttatgtccttcagcagctggaggacggagggacaggctacaatatgccggctgtgttagagctcgaagggaagctcaaccttgaaaggatggacagagctttcaaagagctgatcaagcgccacgagtcgcttcggaccgccttcgaacaggacgcaggaggcgacccggtgcagcgcatccatgacgaggtgccgtttacgttacagactacagttctcggcgcacgaaccgaagaggaggccgcagccgcatttatcaaaccgtttgatctcagccaagcgccgctgttccgtgcccaaatcgtaaaggtatcagatgagcggcacctgttgctggttgatatgcatcacatcatttcagacggtgtttccgtcaacattctgattcgggaattcggcgaactgtacaataatcggaagcttccggcactgcgcattcaatataaagattatgccgtatggcaagaaggattcaaaacaggagacgcgtacaaaacgcagggggcgtactggctgaagcagctcgagggcgagctgcctgtgctggatcttccggctgatcatgcccgcccgccgatgcgaagcttcgcgggtgacaaggtctcatttacgctggatcaagaggttacatcaggcctttacaagctggcacgagaaaacggaagcacactgtacatggtgctccttgcagcttacaccgcgttcttgtcacgcttaagcggacaggaagatatcatcgtcggctcgccaattgccggccggccgcacaaggatcttgagccgatactcggcatgtttgtgaacacgctggcgcttcggacgcgcccggagggcgggaagccgtttgtacagtacttgcaggaagtgcgcgagacagcaatggaagcctttgagcaccaagattacccgttcgaagagcttgttgataagcttgaattgacacgagatatgagcagaaatccgctgtttgacgtaatgtttgttcttcaaaatatggatcaggaatcgttggagctggatgaactttgtctcaaacctgcagcaaacaatgggcatcaaacgtccaaatttgatttaaccctatatgcccaggaacagccccgcggtttgctgacgttccaaatggagtttagtactgacttatataagaaaaaaacgatagaaaagtggcttcaatacttcaacaatatgttactctccatcatcaaagacaacaaagccgctctcggaacaataaatatcctgaatgaggatgaggcccattaccttatccacgagctcaatcgtacggccatagaggccccaagaaatgaaaccatcagcagactctttgaaatgcaggcagaacaaacacctaatgctgtagcaattgtcagcgacacccaagtattcacttacgaggacctgaacagctgggcaaatcaaattgcctcagttctacagataaagggcgtagggcctgatagtgttgtagccttgttgacaggcagaacaccagaactcattgcaggaatgctgggcattctaaaagccgggggagcctatctgcctatcgattctaatctgcctgttgaacgcatagcttatatgctgtctgacagcagggcagcattactccttcaatctgaaaaaacagaaaaacggctattaggcattgaatgtgaacaaatcataatcgaagatattcaaaagcaaggagaggcgaagaacgttgaatcttcagcagggccccattcacttgcatatatcatttatacctctggatcaaccggtaaaccaaagggtgtcatgattgagcagcgaagtgtaattcgtcttgttaaaaacagcaattatattacatttacacctgaagaccgccttctgatgacatcatcaatcggtttcgacgttgggtcatttgaaattttcggaccgctgctaaatggtgccgctttgcatctgtccgatcaacaaacatttctcgattcccatcagcttaagaggtacatagaacatcaaggaatcacaacgatttggctgacatcttctctattcaatcatttgacagagcaaaatgaacaaacattttcacagctgaaacatttgattattggcggagaagctttgtcgccgagccacgtcaatcgaatcagaaatgtctgccctgaagtatctatatggaatggatatggccctaccgaaaatacaactttttcgacatgccttcacattcaaaaaacatatgaactttccattccgatcgggcggccggttggtaattccaccgcttttatcttaaatcaatggggagtgctgcagccggtcggagctgtcggtgaactttgtgtcggcggagatggcgtcgccagaggatatttgggccgtcctgatttaacgaaagagaaatttgtcccacatccatttgcacctggcgatcgactgtatcgcacaggtgatctggcgcgctggctttccgatggcacaattgagtacgttggccgtattgatgatcaagtaaaagtcagaggctatcgggtggagctgggtgaaatcgaaacagcacttcgtcaaatagacggggtcaaagaagccgcagtgttagcacgtacagcccagaccgggagcaaagagctgtttggctatatcagcgtaaaagcaggcacgaatgctgaacaagtgcgttctcttctcgcgcgttcgctgccaaactatatgatcccggcgtatatcattgaaatggagactcttccgctcacatcaaacggcaaattgaaccggaaagcactgcctgaaccagatgtcgcatctaaacaaacatacatcccgccacgcaacgaacttgaagagcagctggcattgatctggcaggaggttctaggcatccagaggatcggaatagaggattcgttttttgaattgggcggagattcaatcaaagcccttcaagtttctgcacgccttgggcgctatggactaagcttgcaggtaagtgatttattccgtcatccaaagataaaggacttatcaccatttatccgtaagtcagagagaatcatagagcaaggacccattcagggtgacgttccttggacgcctgttcagcaatggtttttttcacaagatattgaagaaagacaccatttcaatcagtctgtcatgctattccattctggacgtttgtctgaaaacgcccttagaccagccttgaaaaaactggcggagcatcatgatgcgcttcggatggtttatcgcaacgatgacaggcgatggattcaaatcaaccaaggcattcatgagtcacagctatacagcttaagaatctctgatctttcacagtcagaaagcggctgggagacgaaaatcaaacaagaagttgccgatcttcagcaaagcatcaatttgcaggaaggaccattgttgcacgccgctttgtttaaaacactgaccggagattacttgttccttgcgatccatcaccttgtcgttgatggtgtctcatggcggattttgctggaggatttgtcagccggatatcaacaagctgctgcaggccagacgatccagcttccgcctaaaacggattcctaccaggaatacgcaagacgcatacaggaatatgcccaaagcagtaagctgattcgcgaagaggcgtattggcgaagtgtagaagaacagcaagccgcagaactgccctatgaaataccgcatcatgtgaacatcgacttcagcaaaagggactcattaagcttttcactgactgaagcagacaccgccgtcttgctgcaaaacgtcaatcacgcctatggcacagatacacaagatattctgttaaccgcagcatccttggcgatttgtgaatggacaggaggaagcaagctccgtatcgctatggaaggacacgggagagaacacattctgccagagttagatataagcaggacggtcggctggtttacatccatgtacccggccctcataagctttgaaaatcatagggatgagctcggaacctcagtaaaaaccgttaaagatacactgggccggataccaaacaaaggggtaggttacggtatgctgaaataccttacacaccctgaaaataaaagcattacgttttcaaaaacacctgaaatcagctttaactatttgggccagttcaacgacatcgaaagacaggacaccttccgcccatcaagccttggtagcggaaaggatatcactcatacatggaagcgcgagcaaatcatcgagatgagtgcaatggcagcagacaaaaagctccatttcaatcttagttatccgccagcccgctttcacagaaacacaatggaacagcttattaacaggattgaacactttttgctggacattatgaaacactgcgccggtcaacagaaagcagaaaagacactgagcgatttcagcagtcaatcattaacggcagaggacttggacagcatatccagcttggtggaagaattgtagaaaatcgtgacaggagacatgaacatgacaaaagcgaattcaattcaggatatttatccgctgtcttacatgcaggaagggatgcttttccattccctcctgcaaaaagattcacaggcgtatgttgagcaagcttcttttacaatagaaggaaaagtcaacccgcagttttttcaaaacagcatcaacgctcttgtagaaagacatgatattttcagaacgatttttatcagccaaaatgtttcctccccccagcaggttgttctgagagaacgaaatgtcatcgtactggaagaagacattactcatttaaacgaggcggagcaatcacagtttatcgagcaatggaaagaaaaggaccgggaccgggggtttcatttgcaaaaggatgtgctcatgcgcatcgctctgattcaaacaggagagagccagtactcttgcatttggacctttcatcatatcatgatggacggttggtgcctcagcattgtgctaaaggagtttctgcatatttacgcatcttatgtaaatgcatccccaataacattggagccggtccagccatacggaaagtatatcaaatggctgatggagcaagacaaagagcaggcggtttcttattgggatcattatctttccggccacgaacagcaaaccgtgctcccgaagcagaaaaaaacaaagggaaaaagcaggcaggaacacgttacattttcattctctaaggaagaaagcagcaggctttcagagcttgctgctagagaagaagtgacactcagtacgatttttcataccatttggggcattctgctgcaaaaatataataataacgatgacgccgtattcggttctgtcatttcaggaagacccgcagaaatcgaaggcattgaacatatggtaggtcttttcattaatacgatgccggttcgggtgcagggggcaaaaacgccttttcttcaacttataaaagatatgcaaaaagaccgtcttgccgctgaagcgtacagctaccaccctttatatgagattcaatcccgctcagctgttaagcaagggctgattgatcatattctcgtatttgaaaactatccggtgcagcaagagattcaaatgctgaacaaacaggaacatgcttctgatctttttcagattcataatttcactgtcgcagatgaaaccaactacagcttttatcttatggtggcgccaggggaagaaattcatatcaaaatgaactatgatgcggagcagcacgatcggtcttttgtgctctctgtcaaagagcatcttctgaatgctgtatcacaaatcttaaataatccgaatcttccacctgaagaaatcgatatcacgacagatactgaaaagcggcagctgattggagaaatcacagatcaggccccagtggccgaaaccatccatgccatgtttgaaaagcaagcggaaaagacaccagatgctcatgctgtaattgatcaagcctgctcattaacatacagagaactgaataaagcggctaacagattggcacggcatttacgaatgaaaggcgttgtgagacaggaacccgttgcgattatgatggaacgctcagcggcgtttatcacaggtgttcttggtatcttgaaagcaggcggcgccattgttccggttgatccgcattaccctgctgacagaatccgttatattctgcatgattgcggctgttcgcatgttgtttcacaagcgcatcttccctcatcgttagaagacaattacattatcactcatccagaagatatcgaaagcaaagtagacggcagtaacataaagtcagtcaacaatgctgacgatctgctgtatatgatttatacatcaggcacaacaggtaaaccaaagggtgttcaatttgagcatcgaaacatggctaacttgctgaagttcgaatatactcactccggcattgactttgaagcagatgttctgcaatttgcgacgccttccttcgacgtctgctatcaagaaatattttctgcgcttctgaaaggcggcacactccacatcgtgccagaagccataaaaagagatgtgcctcagctgtttgcatttataaacaagcatcagacgaatattgtgtttctcccaactgcttttatcaaaatgattttcagcgagcgagaacttgcgaactcgtttcctgatggcgtcaaacacctgatcgcagccggggaacaattaatgatttcagaccttttccaagatgtgttgcgtaaacgcggcatacacctgcacaatcattacggaccttcagaaactcatgtggtatctacgtataccattcatcctggagaccctattcctgagcttccgccaatcggtaaaccgataggctgtactgatctatatattttgaatcatcaaaaacagcttcagccatgcggcgtaccaggcgaactctatatttccggcgcaagtgttgccagaggatatgtcaatcacgataaactgacaagcgacaaattttcatccgatccattcaagcctgatgtgatcatgtaccggacaggtgatttggccagacggcttgaagacggcaacatcgaatatatcggacgggcagacaatcaagtgaaaatcagaggttatcgaattgagccgcaagaaatcgaagtcacgctaatgaatcatccggacattagtgaggctgccattctcatctggcaagatcaaaacggtgaacatgaattatgcgcttactattgcagtgtacaaaagctgaacacaatagatttacgcagttatatggctagtgagctcccagaatacatgattccggcgaaatggatatgggttgacagcatacctcttaccccaaacggaaaagtagatcgcgcagcacttccggagccagatgcttcaatcagcggaaacccatatactgcccctcgaaatctgttagaggcaaagctttcgcaactatttgaagatgtgctaaagaatgggcatataggcatccaagacaacttttttgacaatggcggtcactcgttaaaagcaacagtgcttatgtcacggatcgcaaaggaattccatgtgcaagtttcacttaaggacatctttgctcatccgactgttgaaggattagctttaattattcgagaggcagaacaaaatctgtatgcagcaattgaaccagcagaaaaaagggatacatatcctgtatcttcggcccaaaaacgaatctatgtgcttcaacagcttgatgagggtgtcgcctataacatgcctgcggtcttagaactggaaggtgcactggatgtcgccaaactgtctgctgtatgtaaagaactgatcagccggcatgagccgcttcgaacttcctttgtatccggagctgatgacgagccggttcagcgtatccacaccgaagtgccgtttacgttaagtaaagagaccactatcgagggatttgtccgtccctttgatctcagccaggcgccattatttagagcaggccttatagaagtgtcaaacgagaagcatgtattgctggtggatatgcaccatatcatttcagatggcgtatccgttcagctcctaatccgagaatttaccgatctttatgcaaaccggcagcttaagccattgcggatccaatataaagattacgccgtatggcagcagaaatttaaaaagggagactcgtaccaaaagcaggagacttactggcagcagcagtttagcggggaccttcctatactggagcttccaacagataaacgacgtccggcagaacggcaattcataggcggaaaagtaacctttcaattggacaaagagatcacggcccgcataaagcggctcgcccataaaaacagaagcacgctttatatgacgcttctcgctttgtattcagcctttttgtctcggttaagcggtcaggatgatatcgtgattggttcacctatcgccggacggccccatgccgaccttgaagctgttcttgggatgttcgtcaatacattggctctccgcacacgcccggcgggtaataagacatttgaggaatttctgaaagaagtcagacagacggcactagaagcgtatgagcatcaggattacccgtttgaagagcttgtggacaaactcggtgtgcagcgggaaatgagccggaatcctttgtttgacacaacgctagtccttcagaatatggaacagcaaaagctaaaaatgaatgatgtacagcttcagtggaacgacttggagcacccaatatcaaaatttgatatttccctatacgttacagagcatgattccgagcttttctgtcagtttgaatacagtacagctttgtttgagaaagaaaccatccaaaggtgggccagccttttcaccacgcttgtggaacatacagctgccagtcctgaaacagaattggacaatattccaatcttaacaaaagaagaagagcgagatttcattgaatcatgccatctgttggccgtgacggccgcaacctttgcagcactttttgaaaaacaggcccagcaaacacctgaccattctgcggtgaaggctggcggaaatctgttgacctatcgcgagcttgatgaacaggcgaaccagctggcgcatcatcttcgtgcccaaggggcaggaaatgaagacatcgtcgcgattgttatggaccggtcagctgaagtcatggtatccattctcggtgtcatgaaggcgggggcagctttccttccgattgatcctgatacacctgaagaacgaatccgttattcattagaggacagcggagcaaaatttgcggtcgtgaatgaaagaaacatgacggctattgggcaatatgaagggataattgtcagccttgatgacggtaaatggagaaatgaaagcaaggagcgcccatcatccatttccgggtctcgcaatcttgcatacgtcatttatacgtccggtacgaccggaaagccaaagggcgtgcagattgagcatcgtaatctgacaaactatgtctcttggtttagtgaagaggcgggcctgacggaaaatgataagactgtattgctttcatcttacgcatttgaccttggctatacgagcatgttccctgtacttctgggcgggggcgagctccatatcgtccagaaggaaacctatacggcgccggatgaaatagcgcactatatcaaggagcatgggatcacttatatcaagctgacaccgtctctgttccatacaatagtgaacaccgccagttttgcaaaagatgcgaactttgaatccttgcgcttgatcgtcttgggaggagaaaaaatcatcccgactgatgttatcgccttccgtaagatgtatggacataccgaatttatcaatcactacggcccgacagaagcaacgatcggcgccatcgccgggcgggttgatctgtatgagccggatgcatttgcgaaacgcccgacaatcggacgcccgattgcgaatgccggtgcgcttgtcttaaatgaagcattgaagcttgtgccgcctggagcgagcggacagctctatatcacgggacaggggctcgcgagagggtatctcaacaggcctcagctgacagccgagagatttgtagaaaatccatattcgccgggaagcctcatgtacaaaaccggagatgtcgtacgaagactttctgacggtacgcttgcatttatcggccgggctgatgatcaggtgaaaatccgaggctaccgcattgagccgaaagaaattgaaacggtcatgctcagcctcagcggaattcaagaagcggttgtactagcggtttccgagggcggtcttcaagagctttgcgcgtattatacgtcggatcaagatattgaaaaagcagagctccggtaccagctttccctaacactgccgtctcatatgattcctgctttctttgtgcaggttgacgcgattccgctgacggcaaacggaaaaaccgacagaaacgctctgccgaagcctaacgcggcacaatccggaggcaaggccttggccgcaccggagacagcgcttgaagaaagtttatgccgcatttggcagaaaacgcttggcatagaagccatcggcattgatgacaattttttcgatttaggcggccattcattaaaagggatgatgctgattgccaacattcaggcggaattggagaaaagcgtaccgcttaaagcactgttcgagcagccgacagttcgccagctggcggcttatatggaggcgtctgctgtttcaggcggccatcaagtactcaaaccggctgacaagcaggatatgtatccattgtcatccgcacagaaacgaatgtacgtgctcaatcagcttgaccgccagacgataagctacaacatgccatctgttcttctaatggaaggagagcttgatatttcgcgcctgcgcgactcactcaatcagcttgtgaaccgtcacgaatcattgcggacgtcatttatggaagctaatggtgagcctgttcagcgcatcattgagaaggcggaggttgatcttcatgtgtttgaagccaaagaagacgaagcggaccaaaagattaaggaatttatccggccattcgacttaaacgacgcaccgctcattcgcgcagctttgcttcgaatagaagcgaaaaaacatttgctgcttttagatatgcatcatatcatcgcagacggcgtctcaagaggcatctttgtaaaagaattggcgctgctttacaaaggagagcagcttccggagccgacgcttcattataaagatttcgccgtttggcaaaatgaagctgagcaaaaagaacggatgaaggagcatgaggcgtactggatgtcagttctttcaggcgagctgccagagcttgatctcccgctcgattatgcccgtccgcctgtgcaaagctttaaaggagatacgatccgtttccgtacgggaagtgagacggcaaaggcggtagaaaaactgcttgccgaaaccggaacgaccttgcacatggtgctccatgctgttttccacgtctttttaagcaaaatttccggacagcgggatatcgtcatcggctccgttactgccggccggacgaatgctgatgttcaggacatgccgggaatgttcgtcaatacacttgccctgagaatggaagcgaaagaacagcaaacatttgcggagcttttggagctagcaaagcagacgaacctgtcagcccttgagcatcaggagtatccgtttgaagatctggttaatcagcttgatctccctcgggatatgagccgaaacccattgtttaatgtgatggtgacgacagaaaaccctgataaagaacagcttacattgcaaaatctgagcatttcaccttatgaggctcatcagggaacttctaagtttgatctgacactgggcggatttactgatgaaaatggcattggcttgcagctcgaatatgcgacagatctgttcgcaaaagaaacagctgaaaaatggagcgaatacgttctgcggctactaaaggctgttgcggataacccgaaccagccgctttccagtctgttactggtcaccgagacagaaaagcaagcgcttcttgaggcatggaagggcaaggccccgaaggcctacggagttcaaacaatcagtcaattgtttgagcagcaagctgcacgaacaccaaaagcttctgcacttgtcagcggagacaaaacactcacttatcaggagcttgacgagtggtccaatggaatcgcacgtgcattgcgcagccgaggtgttaagccggacacaccagtaggcatcatgatgcatcgttcgttcagtatgatagcatccatacttggtgtgtggaaagccggaggctgttacgttcccattgatcctgaatacccgaaagaacggaaacgctatatcctcagcgacagcggaacgaaactgctgatgacaataaatgaagcggatctgggagtacttgctgactttgaaggagagatcttgacgatagaaagcgtagaggaagacgacaaatcgccgctgccgcaaatgtcgtctgcccatcatttggcttatatcatttatacttcaggaacgacgggccgtccaaaaggggtaatggtcgagcataaagggattgctaacactcttcagtggcggcgaaacgcttatgcattcaacgagacagataccattctgcagctcttttctttctcatttgacggctttataactagtatgtttacaccgcttttgtcaggtgcaaaagccgttttgcttcatgaagaggaagcgaaggatattctggccattaagcatcagctgtctcgtcaacggattacacatatgattattgtgcctgttttatatcgagcgcttttggacgtagtgcagccggaagatgtaaagacgcttagagtcgtcacactggcgggagaagcggctgaccgcgaattgatcgcccgcagcttagctatatgtccgcataccgaactcgccaacgaatatggaccgacagaaaacagcgtggcgactaccgtcatgagacatatggaaaagcaggcatacgtaagcatcggccagccgattgacggaactcaagtgctgattttaaatagcaatcatcagcttcagccaatcggtgttgcgggagagctttgtatagcaggaacagggcttgcaagagggtacgttaatcttccagaactgacagagagagcattcacgcagaatccatttaaacccgaagcacgaatgtaccgaacaggagacgccgccagatggatggccgacggtacactcgaatatctcggaagaatcgatgatcaagtcaaaatcagaggataccgtgtagaaacgaaagaaattgaatcggtcatccggtgtataaagggtgtaaaagacgccgcagtagttgctcatgtaacagcgtcaggacaaaccgaattaagcgcttatgtggtgacaaaaccagggttgagcacaaatgctgtacgctcagaattacaaaacaagctgccggtgtttatgcaccctgcgtttattgaaaaactggactcacttccattgtcaccaaacggcaagctggatcgcggagcacttccaaaacctgtatacaaccacgaaggtgaacgtccattcctcccgccatccagcaaaatggaacaaatactggcagatatatggaaagaagtactgggggcagaaaagatcggaacagctgattcgttctttgaacttggcggagattcaatcaaagcgttacaggtatctgcgcggcttcaccggataggcaagcaaatggcagtgaaagatttgtttagccatccgaccattcaagaattggcagcttatatccgtgattcagatacaagttccagccaagctgcggttgagggagacgtacaatggtcgcctgttcaaaaatggtttctttctcaagatataaaagaaaaacaccattttaatcagtccgtaatgctgcatcgaagcacctctgtacaagaagacgcactgcgaaaaacgttaaaagcaataacgtgtcatcatgatgcgctgcgaatggtgtttacacagaatgaacaaggaaagtgggatcaatataatcggccgctcagtcattcggacgacgcgttgtacggccttcagatgattgatttgtcagctccggacggcactgatggaaatagaccgtatgaacctcttatcaagcgccatgtacttgatattcagcagaaaatggatttgaagaatggtccgctgctgcaagccggtcttttccacacaattgacggtgatttcttatttttatctgctcatcacctcgtcgttgacggcatctcatggcgggttctgcttgaagatttggctttagggtatcgccaagctgctggcggggaggatatcaaactgccgcctaaaacaagctcgtttaaagcgtatgcgaaaaagctctctgactacgctgaaagccagcagctaatgaaacagctcaagtattggcgcgaagccgaagagtatcaaacagaggcattgccttttgatcaaatcgatggaactagagcacacgagggacaacggtccacaatttcgtttaccttaaacgataaagagacagcagcactcttaaaagacgccaacagcgcatataacactgatacgcaggacatgctgctcgcttctgtcattcttgcgctgcgccattggaccaatcaatccgccttcaaactatcattagagggccacgggcgagaggatgtattaaaaggaatagatgtgagccggacgattggatggtttaccgccatttatccgttattgattaaactgaacgcagacttgccagattcggaagaaagcatggttcatgtgctaaaaacaacaaaagatacactgagacgtgtacctgacaaaggattcggctacggtgtcatcaaatatttgactccgcctggcaaaaaagacatcaatttcacaggtgcaccagaaatcagctttaattatcttggtcaatttgaaagcggccgcacagctgaagtacctgaggaggacgccttctcattctctccgctgggtgccggaggtgatatcagcacaacatggaaccgtgaacagtcgctggatatcagcgcaatcgctgcagaaggaaaattgactgtcaatatgacttatgacaatgcccgctttcagcgcaaaaccatcgaacagcttagcgaaacatgccgtcaatttttattacagctgatcgaacactgccagaacaaaagcgaaacagaaaagacgatcagtgattttgatgatcaagaactgaccgaggacgccctgcaagagatcgctgatatgctcagttttcactaatgaatccgtgaagaaaggtgcagacactatgaataccattaaaaaaatcaagaacatttatcctctgagtcatatgcaggaagggatgctgtttcattccttcctccgtaaagaggagggggcgtatgttgagcagtcgctcttcaccattaaaggaagcctcagctatgactggttccagcgcagcattcaagccattatcgaccgccatgatattttcagaaccgtgtttttgccgcacgtcccgcatttgtcgggacctcggcaagtcgtgatgacagaacgtgaattccatttgaacagcgaagacatttctcatctgccgacaaacgaccagaatgagtatattgaacgctttaaagagaaggacaagcaaaaaggctttgatctgcaaaaagacatgctgatgcggatttctctattcaaaacagctaaagatgagcatgtctgtatctggagtcaccatcacattttaatggacggatggtgcctaggtatcgttatgcaggaatttatgcaaatttatcaatcgattcatgcaggaaaaccgctttcattagaccctgtccgtccgtacagcacctatatttcatggctgacaaaccgagacaaagaaaaagcagcggcctactgggatacctatttaaaaaactacagcgctccatcacctctgcctcgtgtgtctgataaagaaacaaaagaaagttatcaccgtgaagatttgatattttcattaaataaaccactgacagacaagctgaaagagactgccaaacaacacggcgtcacgctcgctacccttattcaggcagtctggggtgtgatgctgcagcaatataaccgcacagacgacgttgtgtttggcgcagttgtatcaggaagaccgtcagaaatcccaggcgtggagcaaatgatagggttgtttatcaataccataccgattcgaattaaaacacaccaagacgaaacgtttcacgagctgctcatacgctgccagaaagaaatgctggaagctgagccgtttacctgccagcctttatttgatattcaggcaaacaccgcattaaaacaggaactgattgatcacattatcgtctttgaaaactatccgttacagcagaaaatcgccgattccgctgatcaaaccgattcaccgctgcaaatcgatcaagttcaagtatccgagcaatcaggatataactttaatcttgtcgttgctcctggcgaagagcttgtcatcaagttcagctataatgcattcgtttacgatgctgcctggatcagctgtatcaagaggcaatttacgcaagcgcttagcacagctgcacagcaccctcatatgccaattgctgatttttcttttcttgatgcaacagaaaaagagcagattgtcacacagttcaacaatacggccacggaggccccaaagaatcatacaattatcgatttatttcgcgaacaagcagaaaagacgccagaccataccgcacttgtgtatggcaatatgtctatttcgtataaagagcttgataaacgctctaatgcgctcgccagagagttaattcaaaagggatttcggaaaaacgagacagccggaatattggctgcacattctcccgaattcatgatcagtgtgcttgccgtattaaaagcagggggagcatacctcccgcttgatgcggagcttccgcctgaacgagtcagctttatgcttgaggaaacgcaggcaaaaatgctgattgttcaaaagggattggagcaaaacgctgcgttctcaggaacatgtatcatttcagatgcgcagggattgatggaagagaacgatatccctattaatatcagctccagcccggatgatcttgcgtacatcatgtatacctcaggatcaacaggccggccgaaaggggtcatgatcacgaatcgcaatgtcgtgtcccttgtcagaaacagcaattacacgtctgcgtccggtgatgaccggtttattatgactggatctatcagctttgacgccgtcacctttgaaatgttcggggcacttttaaatggcgcaagccttcatatcattgataaatcgacaatgctgacacctgatcggtttggagcgtatttgcttgaaaatgacattacagtgctatttttaacgacagctctttttaatcagctggcacaggtacgagctgacatgtttcgcggactccatacgttatatgtcggaggagaagcactctctcctgccctgatgaatgccgtcagacacgcctgtccagatctcgcgcttcataatatttacgggccaacggaaaacacgactttttcaaccttttttgaaatgaagagagactatgcggggccgattccgattggaaaaccaatcagtaatagcaccgcttacatcttagatacaaaaggacgtcttttgccaataggcgttcccggcgagctttgtgttggcggtgatggagtcgctaaaggctatttgaacagagtagatctgacaaatgctgtgttttctcctcatcctttcttgcctggagaaagaatataccgtactggtgatttggcgcgctggctgcctgatggaaacttagaatacatcagcagaattgacaggcaaatgaaaatccgcggaaaacgaattgagcctgccgaaatagaagcgcgcctgttagaaatggaaggcgttcaagaagcagcagtgacattgagagaaaaagatggagaggcgcagctgtacactcattacgtcggtgatcacaaaaaaacagatacggattttcgcgccgatttggcgcgtgtgcttccagactatatgatcccgcagcactgggtgcgtgtggagcggatgccgcttaccggaaacggaaaaatagaccgcagcgcgctgcctattccagaaaataagcctgccaaacgacagaacatcatattgccaagaaacttggttgaagaagaattggcgaacatttggaagcaagtcctcggtgttaacacaatcagtattgatgatgacttctttgctattggcggacattcactaagagcactgcaagtcatacatacactaaaacatcagcagaacattgacataccgattgatttcttgttcgaacatccgacaatcgctcagcttgccgaaaaactttattctaaacagctgacagcagcaaatgaacagcatgtgatcaaactgaaccagcacggcgcgcaaaatcttttctgcttcccgccgatatcgggatttggcatttattttaaagaccttgctttattgctgaatgagaaggcagccgtatacgggtttcactttattgaacaagacacccgcattgaacaatatgttaattgcatgacggacatacagcctgagggcccatacgttttattaggctactctgcaggcggaaacctggcttttgaagtggcacaggctatggagcgcaaaggattagaagtcagcgacttcattatcgtggacgcttatctaaaagaacagcctttgcctatcgataccggtaatgacgaatctgcagcatatctgcctgaagcagtcagagaaaaggtgatgaagaaaaaaagaaactatcaggaatattgggcacaattgctgaatgaaggccacatcaaagcaagcattcatttcatcgaagctggaatccaccccgaaaccagcgggcatacaggcttaacgaaatgggaaggcgcctgcggaaactatagtgagtacacgggttttggcgctcataaagacatgctggaaggaacatatgctgaaaagaatgccgacatcatcctcgacattttagaaaagatcacttcaaatcaagtaatactgcacaaacgataaagcggattagcggacagaggccattctctgtccgtctttctttttgtatggccgtctgtgagctttaatgcggtagtttatcacagttaaattgctaacgcagtcaggcaccgtgtatgaaatctaacaatgcgctcatcgtcatcctcggcaccgtcaccctggatgctgtaggcataggcttggttatgccggtactgccgggcctcttgcgggatatcgtccattccgacagcatcgccagtcactatggcgtgctgctagcgctatatgcgttgatgcaatttctatgcgcacccgttctcggagcactgtccgaccgctttggccgccgcccagtcctgctcgcttcgctacttggagccactatcgactacgcgatcatggcgaccacacccgtcctgtggatcctctacgccggacgcatcgtggccggcatcaccggcgccacaggtgcggttgctggcgcctatatcgccgacatcaccgatggggaagatcgggctcgccacttcgggctcatgagcgcttgtttcggcgtgggtatggtggcaggccccgtggccgggggactgttgggcgccatctccttgcatgcaccattccttgcggcggcggtgctcaacggcctcaacctactactgggctgcttcctaatgcaggagtcgcataagggagagcgtcgaccgatgcccttgagagccttcaacccagtcagctccttccggtgggcgcggggcatgactatcgtcgccgcacttatgactgtcttctttatcatgcaactcgtaggacaggtgccggcagcgctctgggtcattttcggcgaggaccgctttcgctggagcgcgacgatgatcggcctgtcgcttgcggtattcggaatcttgcacgccctcgctcaagccttcgtcactggtcccgccaccaaacgtttcggcgagaagcaggccattatcgccggcatggcggccgacgcgctgggctacgtcttgctggcgttcgcgacgcgaggctggatggccttccccattatgattcttctcgcttccggcggcatcgggatgcccgcgttgcaggccatgctgtccaggcaggtagatgacgaccatcagggacagcttcaaggatcgctcgcggctcttaccagcctaacttcgatcattggaccgctgatcgtcacggcgatttatgccgcctcggcgagcacatggaacgggttggcatggattgtaggcgccgccctataccttgtctgcctccccgcgttgcgtcgcggtgcatggagccgggccacctcgacctgaatggaagccggcggcacctcgctaacggattcaccactccaagaattggagccaatcaattcttgcggagaactgtgaatgcgcaaaccaacccttggcagaacatatccatcgcgtccgccatctccagcagccgcacgcggcgcatctcgggcagcgttgggtcctggccacgggtgcgcatgatcgtgctcctgtcgttgaggacccggctaggctggcggggttgccttactggttagcagaatgaatcaccgatacgcgagcgaacgtgaagcgactgctgctgcaaaacgtctgcgacctgagcaacaacatgaatggtcttcggtttccgtgtttcgtaaagtctggaaacgcggaagtcagcgccctgcaccattatgttccggatctgcatcgcaggatgctgctggctaccctgtggaacacctacatctgtattaacgaagcgctggcattgaccctgagtgatttttctctggtcccgccgcatccataccgccagttgtttaccctcacaacgttccagtaaccgggcatgttcatcatcagtaacccgtatcgtgagcatcctctctcgtttcatcggtatcattacccccatgaacagaaatcccccttacacggaggcatcagtgaccaaacaggaaaaaaccgcccttaacatggcccgctttatcagaagccagacattaacgcttctggagaaactcaacgagctggacgcggatgaacaggcagacatctgtgaatcgcttcacgaccacgctgatgagctttaccgcagaattcgcccttcccggtcgatatgaacagcttatttacataattcacgttattggtagttataaatgaaattcctaatatcggttatgaagtgaaattgaatttctacttgatctttctctctatttttgtaaaataaaattaagaatatttaaatattcaatgattcatttttgcagaaatcggaggaagaagaatatatgaaaacatttaacatttctcaacaagatccccccatattgttgtataagtgatgaaatactgaatttaaaacttagtttatatgtggtaaaatgttttaatcaagtttaggaggaattaattatgaagtgtaatgaataatgaatgtaacagggttcaattaaaagagggaagcgtatcattaaccctataaactacgtctgccctcattattggagggtgaaatgtgaatacatcctattcacaatcgaatttacgacacaaccaaattttaatttggctttgcattttatctttttttagcgtattaaatgaaatggttttgaacgtctcattacctgatattgcaaatgattttaataaaccacctgcgagtacaaactgggtgaacacagcctttatgttaaccttttccattggaacagctgtatatggaaagctatctgatcaattaggcatcaaaaggttactcctatttggaattataataaattgtttcgggtcggtaattgggtttgttggccattctttcttttccttacttattatggctcgttttattcaaggggctggtgcagctgcatttccagcactcgtaatggttgtagttgcgcgctatattccaaaggaaaataggggtaaagcatttggtcttattggatcgatagtagccatgggagaaggagtcggtccagcgattggtggaatgatagcccattatattcattggtcctatcttctactcattcctatgataacaattatcactgttccgtttcttatgaaattattaaagaaagaagtaaggataaaaggtcattttgatatcaaaggaattatactaatgtctgtaggcattgtattttttatgttgtttacaacatcatatagcatttcttttcttatcgttagcgtgctgtcattcctgatatttgtaaaacatatcaggaaagtaacagatccttttgttgatcccggattagggaaaaatataccttttatgattggagttctttgtgggggaattatatttggaacagtagcagggtttgtctctatggttccttatatgatgaaagatgttcaccagctaagtactgccgaaatcggaagtgtaattattttccctggaacaatgagtgtcattattttcggctacattggtgggatacttgttgatagaagaggtcctttatacgtgttaaacatcggagttacatttctttctgttagctttttaactgcttcctttcttttagaaacaacatcatggttcatgacaattataatcgtatttgttttaggtgggctttcgttcaccaaaacagttatatcaacaattgtttcaagtagcttgaaacagcaggaagctggtgctggaatgagtttgcttaactttaccagctttttatcagagggaacaggtattgcaattgtaggtggtttattatccatacccttacttgatcaaaggttgttacctatggaagttgatcagtcaacttatctgtatagtaatttgttattacttttttcaggaatcattgtcattagttggctggttaccttgaatgtatataaacattctcaaagggatttctaaatcgttaagggatcaactttgggagagagttcaaaattgatcctttttttataacaggaattgggcatcaaataaaacgaaaggctcagtcgaaagactgggcctttcgttttatctgttgtttgtcggtgaacgctctcctgagtaggacaaatccgccgggagcggatttgaacgttgcgaagcaacggcccggagggtggcgggcaggacgcccgccataaactgccaggcatcaaattaagcagaaggccatcctgacggatggcctttttgcgtttctacaaactcttcctgtcgtcatatctacaattctacacagcccagtccagactattcggcactgaaattatgggtgaagtggtcaagacctcactaggcaccttaaaaatagcgcaccctgaagaagatttatttgaggtagcccttgcctacctagcttccaagaaagatatcctaacagcacaagagcggaaagatgttttgttctacatccagaacaacctctgctaaaattcctgaaaaattttgcaaaaagttgttgactttatctacaaggtgtggcataatgtgtggaattgtgagcggataacaattaagctaattctatggtaaaagcattcctgaacccaatatccttatttttagtggacaaggccttgttctcatatggttgcttgagccagtgccttacaaggctcttccgctttggcaggctgttcaaaattatttattagagcaactcaaggaactaggcggagatccaaaagcaaccgatgcagcacgtgtttttcggattgctgggagcgtcaatagtaagaatggagcggaagtaagagcggaatatcggcacgattacagatatgagttaaggcagattcaatttgattaccttccagaactcaatgaggttattaatcccgctccacaaaagaaaaaacgggggcgtaaaaagaaagtagttcagttattcaatacctacaaactccattacgctcgcctattggatatagtgaaattggtggaactacgaaattatgaggtaactggatacagggaaatcatttgctttttataccgttattggttgtgctgttacacgaacgaccctgtagaggctttaaatcaaacacagacacttaatttacagttcactgagcctttacccttaaaagaggttgaaagggctacacggagcgcagaaaaggcgtgggaagcacgaaataacgaagaggctaaccggattgcaatcgaaaaaggatatcccagtgctggatacaatattagcaataaaaagttgattgaatggctagatatcacaccagaagaacagaagcatttacagacgattatagacgctaatgagaaacggagaagaaagcgggaaagggataggatttatcaagaacaaaaacgtcgtgagcggggagatatgacccgacaggagtatattaagcaacaacaggataaaacagatgataaattatttaaattgcaggagttattagaacagaatcccaaaatctcaaaaattaaattagcaaaaatacttggtgtagataaatcgcacttatacagactgctgaaacaactataactggaaaaaattagtgtctcatggttcgtcgcccttatattatgggcgttagcctgcttgctaattggataggtgttattgtcatttcaacgtcggacgttttggtagatgaacgtcggacgttatttgcttcaatagattgttgatgtattaagggttgcagtgaatcgacaagcaaaaagttatgacgttgtgaaaaaattgaatagaaaattggaaattacgtcggacgttctaacttaaaaaccctgttatatcaatgatttaaaaggaaattaacgtcataaaagacctttctgcaacaaaagtttttctggaagagttgaggttattttataggtattatggacttttgtagactttttgtgtactttttgtggactccacactcgctggtatcgtgttattttttaattgagatatgaatatggaaattaaacgttttaggcgttggtttggtgatgacaaaaaaataagagtacccgctcacaacggatactctttcgagaaatgtacgaaacgctataaataaaaaataactagatacatttacattgtatcacgtttcgtacatttctccaataacaaattgattggaggaatgcaaagtgaataatgaaccagtaaaacgtggtaagaagaacagatgggaattaaacctacctataatgacttatgtagtagctgatgattggattgataaactaggacacgaaacgtttactttatggttgaggttccatacttgggtagatagagaagatgaactccgagattatgatcgcatacctagaagttttgagaacatatataaaaagacactaggaatctcaaaaagtaagttttatagattgataaaacctttatgggaatatggattaatagacatcatagaatacgaagaatctaaccgtaattctactaaacctaaaaatataattgtttatgagtatcctttacacgaaatagaaagaaagtataaaccactagaaaaattaagagattgggataaagactataattccgtttctaaagaattaggtaaaacaggtggtagaccaaggaaaaaagatagtgaagaagaacccgaaaagaaacccgaagaagtaactaaaaagaaacgtaaatataagttaaaaagagttatccacaacggtttcaaaaatgaaacggtggagggtttcaaaaatgaaacggtggagggtttcaaaaatgaaacggtgaccgtttcaaaaataaaacccaataattattcaaatatctttaataacttatcaaatatttctactaatgtttcaaataatttattaattgatgatgatgaggaaatcgaaaatgaaccaactggtcgtacaataaataggtcattacttttttcacaagaagatattaaacaggcctatcaatttattaatagattttcagttatacagttacgtgaaaactttagctttgataaacactttgaagaacggttggtatgttatttatggaaagcagggatttctactttttacacgcacgaaatcagtaaaatgataaaaaaaatagcagactatgaaaaatctaaaaaaggtagattaaacccaatacgtgaccgagccttatatatggtaaatggtcttgtaatgaatagagcttcttcccaaagtgaacatgctacttataaactaaaccaatataaaaaacagaaggaacaggaaaaacaacaacaggagcaacaaagatcaagagtaccgttctataattggttggaggaaagagaagaacaaaccgaaggtcaactacccaccacttaaagcctaacggcttttgaagtggggcttgtaaaaagccctagttgactaccccaagtctttcgaggactacgttggaaaggtcatgacacctacaaatgctcctctagttcgtagccactgtcgttgatggttaaaagtcctgatgggtagggacggtgctgtcaacatcacaagcccttccaacatgggggaagaggaagaacactccgagaaaggagggggctgtcgtacacgccttgttcgtgtacgtgatttttaacacttttatctctaatataatctctccttgagttagcagagactaagaataaaacacattaggattttttatctacataaggaggttcaatacatgcctactatttcgtttaagggaaagtcttttgtacaaaatcatcacttgactgtaaaatatcatgaattgatcccagaaccagaaaaaagtctgaccgataaagttagtcttcatgacaatcttatcattcatggggacaatttaaaggcgttgaaagctctactacctacatatgctggtaagatagattgcatctatattgacccaccatacaatactggaactgaaaaatggatttataatgataatgtcaactccccaatgattagggaatggcttggaaaagtggtagacaaagaagacttatcccgacatgataagtggctttgtatgatgatgccgaggttaaaactgttgaaagagttgttgtcagaagacggagtgatatttgtaagcattgactacaatgaaatacaccatcttacgtgccttatgaacgaaatattcggtgaggagaattttcgtgacgctattatcattcgtagaggagtaaaaaatgttcaagcgcaatttgacacaattgattctctttcaaatggttatgagtctattttggtttacactaaacagccatctcgacgatttaataaggtttatgaagatgtagaagaaaagcctggtagttggaataatcattggagaggtacagaccgtaaaactatgagatatgaattatttggggttactccgacagaaggtcaatggagatgggggaaagaacgtagtctccaggctattgaaaactatcaaatgatgttagatgaacttagacaaaaaggcattactaatccaactcaagaggatattgataaatggtatcttgaatatgtagaaaataatggggaagatattgacttgttacgacaaaatgataatggcacgattgagcactttgttccaccgactagcaaaaagttgttaagtaatgcctggtttgacttaaaacccaacggttctagtcaattaaagaagatatttggaaggaaggttttcgataaccctaaatcaattgatttggtaaaaagactaatacaatttgcgactgaaaacaaagaagcgattgtacttgactcatttgcagggagtggcactactgctcatgcagtattatcgcttaacaaacaagatggagggaatcgtcgtttcatccttattgagatggaagaatatgcacatgagattaccgcagaacgcggatctttatcgatttgcatgcaagctaattcggtggaaacgaggtcatcatttccttccgaaaaaacggttgcatttaaatcttacatatgtaatactttcaaagactacatttgtaagatttgatgtttgagtcggctgaaagatcgtacgtaccaattattgtttcgtgattgttcaagccataacactgtagggatagtggaaagagtgcttcatctggttacgatcaatcaaatattcaaacggagggagacgattttgatgaaaccagtaacgttatacgatgtcgcagagtatgccggtgtctcttatcagaccgtttcccgcgtggtgaaccaggccagccacgtttctgcgaaaacgcgggaaaaagtggaagcggcgatggcggagctgaattacattcccaaccgcgtggcacaacaactggcgggcaaacagtcgttgctgattggcgttgccacctccagtctggccctgcacgcgccgtcgcaaattgtcgcggcgattaaatctcgcgccgatcaactgggtgccagcgtggtggtgtcgatggtagaacgaagcggcgtcgaagcctgtaaaacggcggtgcacaatcttctcgcgcaacgcgtcagtgggctgatcattaactatccgctggatgaccaggatgccattgctgtggaagctgcctgcactaatgttccggcgttatttcttgatgtctctgaccagacacccatcaacagtattattttctcccatgaagacggtacgcgactgggcgtggagcatctggtcgcattgggtcaccagcaaatcgcgctgttagcgggcccattaagttctgtctcggcgcgtctgcgtctggctggctggcataaatatctcactcgcaatcaaattcagccgatagcggaacgggaaggcgactggagtgccatgtccggttttcaacaaaccatgcaaatgctgaatgagggcatcgttcccactgcgatgctggttgccaacgatcagatggcgctgggcgcaatgcgcgccattaccgagtccgggctgcgcgttggtgcggatatctcggtagtgggatacgacgataccgaagacagctcatgttatatcccgccgttaaccaccatcaaacaggattttcgcctgctggggcaaaccagcgtggaccgcttgctgcaactctctcagggccaggcggtgaagggcaatcagctgttgcccgtctcactggtgaaaagaaaaaccaccctggcgcccaatacgcaaaccgcctctccccgcgcgttggccgattcattaatgcagctggcacgacaggtttcccgactggaaagcgggcagtgagcgcaacgcaattaatgtgagttaggatcctgcctcgcgcgtttcggtgatgacggtgaaaacctctgacacatgcagctcccggagacggtcacagcttgtctgtaagcggatgccgggagcagacaagcccgtcagggcgcgtcagcgggtgttggcgggtgtcggggcgcagccatgacccagtcacgtagcgatagcggagtgtatactggcttaactatgcggcatcagagcagattgtactgagagtgcaccatatgcggtgtgaaataccgcacagatgcgtaaggagaaaataccgcatcaggcgctcttccgcttcctcgctcactgactcgctgcgctcggtcgttcggctgcggcgagcggtatcagctcactcaaaggcggtaatacggttatccacagaatcaggggataacgcaggaaagaacatgtgagcaaaaggccagcaaaaggccaggaaccgtaaaaaggccgcgttgctggcgtttttccataggctccgcccccctgacgagcatcacaaaaatcgacgctcaagtcagaggtggcgaaacccgacaggactataaagataccaggcgtttccccctggaagctccctcgtgcgctctcctgttccgaccctgccgcttaccggatacctgtccgcctttctcccttcgggaagcgtggcgctttctcatagctcacgctgtaggtatctcagttcggtgtaggtcgttcgctccaagctgggctgtgtgcacgaaccccccgttcagcccgaccgctgcgccttatccggtaactatcgtcttgagtccaacccggtaagacacgacttatcgccactggcagcagccactggtaacaggattagcagagcgaggtatgtaggcggtgctacagagttcttgaagtggtggcctaactacggctacactagaaggacagtatttggtatctgcgctctgctgaagccagttaccttcggaaaaagagttggtagctcttgatccggcaaacaaaccaccgctggtagcggtggtttttttgtttgcaagcagcagattacgcgcagaaaaaaaggatctcaagaagatcctttgatcttttctacggggtctgacgctcagtggaacgaaaactcacgttaagggattttggtcatgagattatcaaaaaggatcttcacctagatccttttaaattaaaaatgaagttttaaatcaatctaaagtatatatgagtaaacttggtctgacagttaccaatgcttaatcagtgaggcacctatctcagcgatctgtctatttcgttcatccatagttgcctgactccccgtcgtgtagataactacgatacgggagggcttaccatctggccccagtgctgcaatgataccgcgagacccacgctcaccggctccagatttatcagcaataaaccagccagccggaagggccgagcgcagaagtggtcctgcaactttatccgcctccatccagtctattaattgttgccgggaagctagagtaagtagttcgccagttaatagtttgcgcaacgttgttgccattgctgcaggcatcgtggtgtcacgctcgtcgtttggtatggcttcattcagctccggttcccaacgatcaaggcgagttacatgatcccccatgttgtgcaaaaaagcggttagctccttcggtcctccgatcgttgtcagaagtaagttggccgcagtgttatcactcatggttatggcagcactgcataattctcttactgtcatgccatccgtaagatgcttttctgtgactggtgagtactcaaccaagtcattctgagaatagtgtatgcggcgaccgagttgctcttgcccggcgtcaacacgggataataccgcgccacatagcagaactttaaaagtgctcatcattggaaaacgttcttcggggcgaaaactctcaaggatcttaccgctgttgagatccagttcgatgtaacccactcgtgcacccaactgatcttcagcatcttttactttcaccagcgtttctgggtgagcaaaaacaggaaggcaaaatgccgcaaaaaagggaataagggcgacacggaaatgttgaatactcatactcttcctttttcaatattattgaagcatttatcagggttattgtctcatgagcggatacatatttgaatgtatttagaaaaataaacaaataggggttccgcgcacatttccccgaaaagtgccacctgacgtctaagaaaccattattatcatgacattaacctataaaaataggcgtatcacgaggccctttcgtcttcaagaattctcatgtttgacagcttatcatcgataagctcac

SEQ ID NO: 30 - DNA, 50726 bp, synthetic construct
  misc_feature 1..50726: note = Chimeric construct 3
  source 1..50726: mol_type = other DNA
atgtggcccgggagacctgttttccaagagaaaacaggtttttttatgtctgtaataacgctttgtcgaaccttccaacaattagaagaatgatgcacaaaagaaaattagtccgattaaaaagtagtgtataagaccttatgtaaaacaatacttttatcactttatatccggaaatttgataaaaaaagaaacgaaaaataaagaaataatactatattcaaaaaaaatgttataaaaatttaatgttttttattgtactttaaaaaatatccgttaatatagtgcatatatggattatatagtcatataatttcttttattgtcatttttctgcttttttctacattttcttatcctcttattatgagaactggagggaatccgttgagcgaacatacttattctttaacccatgcccaaaggagagtgtggtttaccgaactgctggagccagataccagcatttgcaatcttacagcttgtgtgaaatttaaaggcaatattgagcttgatactctggagggagcactgaatcattccatctcccgcaacgacgccattagatttcagctgttagaaggagaagagcttgagcctcgattgcaccttactgaatataaatattatccacttagaataattgatttttcaaatgttgaaatgatagaaatagagcaatggattcaggatcaagcgagcattccatttaaactgttcaactcgcctctttttcaattttacctccttagaattgactctcatgaagtttggctatttgcgaaattccatcatatcataatggatggaatctctttaaatgtgatgggaaatcaaattatagatctttatcaaaaaatgaaaaagaaagatcctttacctgatcagccggaaccttcttacttgagctacatcgaaaaagagagtcaatatctacaatctccacggtttgcaaaggaccgtttattttggacgcaaacctttgagcacccgttggaataccactcgttagccgaccagacgtccttacaaaaacagagcacatctgcatccagagacaccatcattctttcacctgatctagagcaaacgattcgaatcttctgcgaagaacacaagatcaatatcatttccttatttatggcttcattttacatatgcatcagccgaatcacttctaaaaaagatcttgccattggcacctactatggcaacagaggttcaaaggctgaaaaagaaatgctcggcatgttcgttagttcccttccaatcagaataacggttgatcctgacacagattttctttcctttgtccgcacaataggcagggaacagctttctgttatgcgtcatcaacggtttccttataatttgcttgtaaatgaattaagaaatgaacagaaggatttacacaaccttatcggtatatctatgcagtatcagccacttcagtggcacaatgcagatgattttgactatgaaacagcgctttatttcagcggatacaccgcgaacgaactttcagttcaaatacaagaacggatagacaatggaaccattcaattaaatttcgactatcaaaataccttgttttctcttgaggatattaaacgaatacaatctcatctgcttaccatactggaaaacgcccttaaacatccgcacagctttataagagaattagatatgacgaatacaagagaaaagcaaaaattgttgtatgagtttaacaagacggccgtggcggcccctaaagctttcaccctgcatgggctgtttgagcgacaggcagctttcacaccggagcggctggccattcgcttttcaggcggttcgctgacatacgctgagcttgatatgtacgccagccggctggctgcgcaccttgcggcacgcggcgtcacaaacgaaagtatcgtcggtgtcctgtctgaacgctcacctgacatgctgatcgctgtccttgctgtattgaaggccggcggggcgtatttgccgcttgatcctgcgtatccaaaggagcggctgagctacatgctgaaagacagcggggcatcgctcttgctgacacagccgggatgctccgcaccaaacttttctggcgaaacgcttgaagtggacatgacatctcttgcgagcgaaaaagcagaaaaccatgagtttactcctgctgacggcggatctctcgcctatgtcatctatacatcgggctctaccgggcagccgaaaggagtggccgttgagcaccgtcaggctgtttcctttctgaccggcatgcagcaccagtttccgctttcggaagatgacattgtcatggtgaaaacctctttttcctttgatgcgtctgtgtggcagctgttttggtggtcgctttccggtgcttcggcgtatctgcttccgcccggctgggagaaagactccgcattgatcgtacaagccattcatcaggaaaacgtgacaacggctcattttattccggctatgctgaacagctttctcgatcaagcggaaatcgaaaggctgagtgacaggacaagcctaaagcgtgtattcgccggaggtgaaccgcttgcgccgcgtacggcagcccgttttgcttctgtattgccgcaggtatcattaatccatggttacgggccgacagaagcaacggtagacgcggcattttacgtattggatccagaacgggacagggatcgtttgcggattccgattgggaagcccgtacctggtgcgcgtttgtatgttttagatccgcatttagccgtacagccttccggtgtcgccggcgaactgtacattgccggagcgggtgttgccagaggttatttgaatcggccggcattaacggaggagcgttttcttgaagacccgttttacccgggggaacgcatgtacaaaaccggggatgtggcgcgctggctccctgacgggaatgttgaattcctcgggcgcacggatgatcaggtaaaaatccgcggctaccggattgagccgggagaaattgaagcggcactaagaagcatagaaggcgtaagagaggcggctgttaccgtacggacagacagcggggagccggaattatgcgcttatgtagaagggctccaaagaaacgaagtgcgtgcacagcttgagagactgttgccgggctacatggtcccagcctatatgatagagatggaacagtggccggttacgccaagcggaaagctcgaccgaaacgccctgccagctcctggcggagcggcagatgcggagacctacacggcgccgagaaacgtgactgagatgaagctttctcagctgtgggaggacgtgctgaaaaatggccctgtcgggattcacgacaacttttttgaccgcgggggacattccttaaaagcaacggcgcttgtctcacggatcgccaaagaattcgatgtacaggtgccgctaaaagatgtgtttgcccatccgacagtagaaggactggctaccgttatccgtgaaggaacggacagtccatatgaagcgattaagcccgctgaaaaacaggaaacctatccggtttcctctgcccaaaagcggatttatgtccttcagcagctggaggacggagggacaggctacaatatgccggctgtgttagagctcgaagggaagctcaaccctgaaaggatggagagagctttcaaagagctgatcaagcgccacgagtcgcttcggacctccttcgaacaggacgcaggaggcgatccggtgcagcgcatccatgacgaggtgccgtttacgttacagactacagttctcggcgaacgaaccgaacaggaggccgcagccgcatttatcaaaccgtttgatctcagccaagcgccgctgttccgtgcccaaatcgtaaagatatcagatgagcggcacctgttgctggttgatatgcatcacatcatttcagacggtgtttccgtcaacattctgattcgggaattcggcgagctgtacaataatcggaatcttccggcactgcgcattcaatataaagattatgccgtatggcgagaaggattcaaaacaggagacgcgtacaaaacgcaagaggcgtactggctgaagcagctcgagggcgagctgcctgtgctggatcttccggctgatcatgcccgcccgccggtgcgaagcttcgcgggtgacaaggtctcatttacgctggatcaagaggttgcatcaggccttcacaagctggcacgtgaaaacggaagcacactgtacatggtgcttcttgcggcttacaccgcgttcttgtcacgcttaagcggacaggaagatatcatcgtcggctcgccaattgccggccggccgcacaaggatcttgagccgatactcggcatgtttgtgaacacgctggcgcttcggacgcgcccggagggcgggaagccattcgtacagtatttgcaggaagtgcgtgagacagcattggaagcctttgagcaccaggattacccgttcgaagagcttgtcgataagcttgaattgacacgagatatgagccggaacccagtgtttgatgcgatgtttatccttcaaaatgtggaaaaacaagacatagatctgagagaaataaaagtccggcctgccaatttcgcacatcacatttccttatttgatatcacattaatagctacggaaataagtggatctatttgctgcgaaatggaatttagtacagaagtattcctgaaagctacgattgaacgctgggctgatcattttatcgaatttctgcatgaggcactttcaactcctgaaacaagccttgcacaaataaacatacttagtgataaagaaaaacaaaaaatagtctttgaatttaacaaaacggccgttgaggccgctcaaaaagatattccttttcatcgcatatttgaagcgaaagctgaagaaaatccagaacatatagctgttattgataacgaaacagagattagctatcgccttctaaatgaaagagccaatcgtctggcacgaacattgcaaaacagaaaaggaccgaagccaactgtggctgttttagccaagcggtccatcgatgcaattgttggagttctggcagtgatgaaagctggcggagtgtatatcccaatcgatgcacattatccaaaagctcgtattgaatacattcttcgtgatagcggggcagatattcttcttttacagagagagttgaagcatttgatttcgaactcgcctgaatctgagatgtctcacatcttccttgacgatgagggctcttttgaagaaagtaactgcaaccttaacttatctcctgctcctgaagagccggtatatatcatttatacgtcaggaacgacgggtgcgcctaaaggtgttattgtcacctatcagaactttactcatgctgctcttgcttggcgtcaaatttatgaactggatcggaagcctgtcagactgcttcaaatcgcgagcttttcattcgatgtcttctcaggagatttggcgagaacattgaccaacggcgggactctaatcgtttgcccagatgaaacacggctggaacctgctgaaatatataaaatcattaaatctcagagaatcacggtgatggagtcgacaccggctctcattatcccggtgatggagtatgtataccgtaaccagttcaagcttcctgacttagacatactgattcttggttccgacatggtgaaagctcaagatttcaaaacattgacagatcgctttggccaaagcatgcgcatcattaatagctatggtgtcacagaggcaaccattgattcgagtttctatgaaaccagtatgggtggagagtgtacgggagataacgtaccaatcggcagcccgctgccgaatgtacacatgtacgtactcagccagactgatcaaattcagccgatcggtgttgccggcgagctgtgcatcggcggggcaggtgttgcgaaaggctatcatcataaacctgacttaacgcaaatgaaatttacagaaaatccatttgtctctggagaaaggctgtacagaaccggtgatcgagcatgctggcttccaaacggaacgatccggcttcttggccgaatggattatcaagtaaagataaatggatacagaattgaaacagaagaaattgaaagtgttctgcttcaaacggggcttgtcagagaagctgctgttgccgttcagcatgataaaaatggacaggctggtttggcagcatatattgtgccttcagacgtcaatacgaatgctctccgtgctgctttaacaaaggaactgccagcgtatatgattcctgcatatctgattcctttagtaaacatgccgctgaccctaaacggaaagctggacagaaatgccttgccggctccaaataatgtgttatcgcgtccatataccgcaccagttaacgacttacaaaaaacgatggcgtatatatgggaagatgtactgagcatgtcacgagtcggcattcacgattccttttttgagcttggcggagactcaattaaagcattacaagtggcagcacgtctggcagctgaaggctggagcatgacaatacgcgacttattccgttattcaacgattcaggaactatgcggacatatcacaccattggcatctcaagcggaccagggacctgcggaaggtgaagctgaactcaccccgattcagcgaagatttttcggacaggtacatgcttttcactatcattacaaccagtccgtcatgcttttcagtgaaaaaggattcaatgctaacgcgcttcatctagcgctgcgtaaaataaccgagcatcatgatgccattcgcatgattttccaacgtgaccaaaacggccatgtcattcagtttaatcgcggaatcaatcacaaggatcatgaactgtttggcctttatatttcagattggacaaaagcatcgctggaaagggctcatcttgatgaaaaacttgccgctgaggaaaccgtcattcaaagcaaaatgaatgtagaaaaagggcccttactgcaagcaggtttgtttaaaacggcagaaggggatcatttgctgattgcacttcatcatcttgtgatagatggcgtttcttggagaattctgcttgaggatttagctgcagcatatcaacaggctttagaaaagaaagaaatccaattaccgccaaaaacggattcttatttatcctacgccgatggtcttacccaaatagctgaaagtaaacaattgctttcagagaaaacgtattggcaaacgattttagacgctcacactgcttttcttcctaaggacatagaaaatgtgccagacaaactccaaatgaacagcgacgcagcagcgtttgtactatccggggactggactgaaaaattgctgtttgaaacccagcaagcctatggtactgatgccaacgaacttttgcttacggctttaggaatggcgctttctgaatggactgggcatgaccaaatcgtgatcagcactgagggacacggtagagaagggcatgtgccaaacattgatatttcaaggacagttggatggtttacctccatttatcctattctgctagacatgggtattcccgagcctttcgaggatcagctcgcataccgaattaagacgacaaaagatatgctgagaagagtaccgaacaaaggaactggatacggattgttaacacacataggagaactgcggcataaagagcctgaggtcagctttaattatctcggtcaatttagcgaagagaaggaagttgaaacgtttcaattatcatattaccagccccgttacgaaatagcgggtgagagagaacgagagtatgagctggacatcaatgctctcattacggacggacggcttcacgtaaaagcggtatacacccaagtgttcagcaaacactcaattgagtgctttatggatcgttttcacaggcatcttatcgagacgattgagcattgttcgcagaaaaaagcacgcgaaaaaacattgagcgatttcagcaataaagaattaacgttgtctgcattatctagcatcgaagatctcgtgaaagatctttaacttttgaaaaggtgtgtggaattgatggcacaatcggcacaaattcaagatatttatccgttatcgcacatgcaggaaggaatgctgtttcattcactaatggatttcagctcgaaagcatatatcgaacagacctcgtttacgatcacagggaatctatgcgtcgactcgtttcaaaagagcttaaaccttcttgtttctagatatgatattttcagaacgattttcattaaagaagtaccagatcttacaggtccgcagcaggtagttctatcaaaccgtgaattgacagtatatagagaagatatttctcgcctggctgatcaagaacagcagacgctgattgatgcttttatgactaaggatcgggaaaaaggatttgatttgcaaaaagatcctttaatgcgtcttgccctttttgatagaggagacagccaatatacatgtgtctggacacatcaccatatcatcatggatgggtggtgtctcggcattattcttaaagagtttttcagcatgtatgattcgctcaaaaataactcacctgtacagcttggcagcacggtgccgtacagccgttatattgaatggctcggagaacaagatcaagaagagactgctgcctactggagcgaatatttgaaggagtacggcaatactgcttctattccccgaataaagcgccgcacggcagacgggaattataaagccgaccaggtcagcttttcattagcgccggatatggttgagaaactgacagaggctgcccaaaactggggagtgacattaaacacgctgtttatgagtatttggggcgtgctgctccatcgatataatgctgcagatgatgccgtttttggctccgtcatttcgggacgcccgtcagcgattgacgggattgaatcaatggtcggtttgtttatcaatactgttccagtgcgaatccgatctgcggaaggcataacattttcttcgctggtcaaagccgtgcaggaggatattttatcatctgaacagcatgggtattatccgctttatgagattcaaaaccatagtccattgaagcaagggttgatcgatcatatttttgtttttgaaaattaccctgtacagcttcatcaggcattaagcgtggagagtgaaaatgacgaaggcgctctgaagctgagtgacatttcaatgtcggaacaaaccaattacgactttaatatcgttatcgttccgggagaatcattttatatcaaattcagctacaacgcagacgtttacgagcgggaggagatgctgaggattcaggggcatctaaagcaagcactggattgcattttgacaaatcccgatgttgccgtcagtgacatcaatatcgtgccgccggaggagcaacaggttatccaattgtttaacgaaacggcccgtccggccgtgaacaaaacgataccccaattgtttgaggaacaagctcacaaaacacctgaagctgctgcattgaaaatgggaaacgagtgctggacctatcgccagttacaagtaagagccaatcagattgcgcacgccctgatagaaaaaggcgttggatctggggatatcgttgctgtaatgatgggccggtcaatggaaatgcctgcagctctgcttgggatttggaaagcaggcggcgcttatatgccgcttgatccacattttccagcagaacgtctttcttttcttctgaaggacagtcaagcggctcaattgctgatagaagaagaccttatttccttgatccctccgtcctatgaaggaaatacgataacgatagaacatacagaaagttaccaaacagaagcgccaaatatgccgccaggtgatctagcctacttgatctatacgtcgggaacgacggggcgccctaaaggggttttagttgatcatcacggtattgccaatacattgcaatggagacgggaagagtatagcatgaccgaacaggatatatccctccatttgttttcgtacgtgtttgacggctgtgtaacgagcttatttaccccgcttttatctggtgcgtgcgtactgctgacaacagatgacgaagcgaaggatgtgctggcccttaagcgaaaaatagcccgttataaggtcagccacatgatcattgttccttccctgtacagggtgttattggaagtgatgactgctgacgatgcaaaaagtcttcgtattgtgacatttgcgggtgaagcggtcacgcctgatctgcttgagttgaatcaaataatttgtccttctgctgaactggcaaatgaatacgggcccacagaaaacagtgtggcaacaacaatattgcggcatctgaataaaaaagagaggatcacgatcggacacccgatcagaaacacaaaagtatttgttttgcacggaaatcaaatgcagccgatcggcgcggcgggtgaactgtgtatttccggcgcgggtcttgcgagaggatactacaaacagcaagagctgacacagaaagcattctccgatcatccattccttgaaggggagcgtttataccgaacaggtgatgcaggccgctttttgcctgatggaacgattgaatatattggacgttttgatgatcaagtgaaaattaggggttatcgtattgaactgagagagattgaaacagttcttcgacaagcaccgggggtaaaagaagcagcggtactggcccgtgatgtttctgctgaggaaaaggagctcgttgcttatatcgttccggaaaagggaaacagcctcccagatttgtatcagcatcttgccgggacattgccgtcctatatgatcccagcaagtattatcaacatcagccagatgccattaacatccagcggcaagcttgacaggtttgcgcttcctgaaccagaaaacaatacgagtgtcacatatatggcgccccgaaccttaatcgaagctgatctcgcacatatttgggaagatgtgctgaataaacagcacatcggcattcgtgatgatttctttcagttaggcggacagtccttaaaagcggccgcactggtatcaagaatacataaaaagcttaatgtcgagctgccgctcagtgaggtgttttcttatccgacggttgaaagcatggcggtcaaattgatgagcttaaaagaacacgcttttacacagattgaacctgcggatcaaagagatgtctatccgctgtctttctcgcaaaaacgattatatgctcttcatcagctggcagatgacagcacaggctacaacatgccagctgtacttgaattacgcggaaatctgaatcgccagcggttgagaagcgttctcacagaacttgtgaatcggcatgaagcattacggactgtttttgtgcttgacagagacgagcctgtgcagatcatttatccagagatggcttttgatctaaaagagcttgaaatggaatcagaacaaatgcttgagtctgcaatcgagacctttatcaaaccgttttatctatcatccggtccgctttttagagcatgtgtcattacaatgggcaataatcgcggctttttgctgctcgatatgcaccatattattgccgacggtgtctcgatgagcactcttgtccaagaatttactgacttatattgcggaaaagagttgccagctttaaacctgcattataaggattttgctgtttggcagcaagagaagcacccgaaagagctatacaaaaaacaggaggcctactggctcggtcagcttggcgggagtcttcctacactagaattaccgcttgataaaacaaggccgcgtctccctgatttcaggggtggaacaattgaagtcaacattgataaagacatggctgatgaactgcaccgtttaatggctgaaacgggaacaacattgtatatgattcttctggctgtctattctattttgttatctaagctaagcgggcaagaggatattgttgtcggttcgcctgctgccggaagaccgcacgctgatctggagcgcgtcatcggaatgttcgtcaatacattggcgatgcgcagcaagcccgagggccacaaaacgttcagctcctatttgcatgacattcgccacctggctctgaccgcttacgagcatcaggattatccttttgaggagctggcagataagctcgatacaaatcgagaggtaaatcgcaacccgctgttcgatgcgatgcttgtgcttcaaagcagtgaagatttccggttcgaagtgcctggtctgtcgatttcgtctgtcactcctaaacatgatatatctaaattcgatttaacattacatgctgaggagcatctgagtggaatacgctgccgttttgaatacagcactgctctttttgaagaagaaaccattacgcagtgggcatcctattttattgaattggtaaaaggggtaacggcggatactgagatgagaatttcgaacatgcaattgcttcctgctgcagagcgtaggttactccttgaaaaaatggggcaggccgccctggccccgagaaatgaaaacatagtaagcttatttgaaaagcaagtagctcagtatccggagcatatcgcagtggtgtgcggccattctcagcttacgtatcgagacctgaatgaaaaagccgagcgggcagctgctatgctgatcaaacaaggggtcagaactggcgatatcgtcggtctgatgctcgatcggtcacctgatatgatcattggcgttttatcgattttaaaagctggcggggcctatttgccgattgatcctgaatatcccaaggagcgtattagctttatgctcaatgacagcggagcaaaactgctgctgacagagcgcggtctaaacaaacctgcagactacaccgggcatattttgtatatcgatgaatgtgaaaacaactcaattccggctgatgtaaacattgaagaaatagtaacggatcagcccgcatacgtgatatacacatctggaacgactggtcagccaaagggagtcattgtcgagcaccgcaatgtgatcagtctcttgaagcatcaaaacctgccttttgaatttaaccatgaagacgtctggacgttatttcattcttattgctttgatttctctgtatgggagatgttcggtgcgttattgaacggaagtacattagtcgtggtctctaaagaaacagcccgtgacccccaagcattccgattattgttaaaaaaagagcgcgtcactgtactcaatcagaccccgactgctttttacggcttgatgcttgaagaccaaaatcatacagatcatttaaacatccgctatgtgatttttggcggcgaagccttacagcccggattgcttcaaagctggaatgaaaaatatcctcatactgatttgattaatatgtacggtattacagaaacaacggtccatgtaacattcaaaaaattgtccgcagcagacattgcaaaaaataaaagcaatatcggccggcctctttctactctgcaggctcatgtgatggatgcccatatgaacctgcagccgaccggagttccaggggagctgtatataggcggcgaaggtgtggcacggggatatctcaacagagatgagctgaccgctgaccgttttgtatccaatccttatcttccgggagacagattataccgaacaggagatcttgctaagcgcctgtcaaatggcgagctggaatacttaggccgcattgatgagcaggtgaaagtcagagggcaccgtattgagttaggcgaaatccaagcggcacttcttcagtatccaatgattaaagaggcggctgtcattaccagagcagacgagcaagggcaaacagctatatatgcatatatggtgataaaagatcaacaggctgcgaatatatcagacatccgaacttacctaaaaaacgccttgcctgactttatgctgcctgcccgtatgatacaaattgacagcatcccggtgactgttaatggaaagctcgatcagaaagccctgccagagcctgaaaaacaagcttatacagctgatgatatcagtcctagaaatgagattgaaacggtgatggctgaaatttgggaagagcttcttaatgtagatgagctgggtgtaagcgccaatttctttaagcttggcggagactctattaaagcgctgcaggtttgtgccagactgaagcagcgcggatttgaaacgacagtacgtgagatgtttgaacatcagactcttggtgaactgtccgcccgggttcgaaaagacgtacgcgccattgaccaaggcccggtcgaaggcgagattacttggacacctatccagcagtggtttttctcgcaatctctggaaagccatcattttaaccaatccgttatgatctaccgggctgaacgatttgatgaggctgcgcttagaaaagtactaaaaagccttgtgactcatcatgatgcactgagaatcgtatgccggcatgaagatggcaggcaagtgcagataaacagagggatagatctttcagatgaggagctatatgcacttgaactgtttgatgtaaaggatagcctaacagaagcccggaacacgattgaggaagcagccagccggatgcaagaacatattcgtttggaaaccggccccttacttcacgctggattgtttagaaccgagaatggtgaccatttatttctaacgattcatcacttagttgttgatgcggtttcttggcgcattttgtttgaggatttttcaacagcttacaaacaggcagtctcaggagaatctattaaactgccgcaaaaaacagattcatatttaacgtattcacaaagaatagctgactactctataagccgccaggtgcagcgcgaagcagcgtactgggatgagtgcgagaaccgtcacatccagcctattccaaaagacaatgacgcagcatctaacacattcaaagatacagaagtgattgattttgagctatctcgccatcacacagaattactattaacggctgcacataaagcttacagcacggagatgaatgatatccttctgacagctttaggtcttgctttgcagaaatggacgggaaataaccaatttaaaatcagcatggagggccatggaagggaatcatatcttgaggacatcgatattagcagaactgttggctggttcacctccatttatcctgtgtggcttgatatgagagattccgatcataaggacaaagaagagcggctgggccaccttattaaacagacaaaagatatgctgcaccgtataccgcataaaggcgcgggctacggcgtgctgaaatatatcagcaaaagatggggctctcagaaaaacagcccagaaatcagctttaattatttaggccagtttgatcaggatattcaatcaaatgcctttgaggtgtctgacatcaagccaggaaatgagatcagcccgaactgggagcgtccttatgcactggatatcagcggcgccgtttcttcggggtgcctgaacatgcacatcatctataacaggtttcaatttgaggaaaaaacaatccaaacattttccaggcattttaaacagactctggaaaacatcattgagcattgtaccggcaaagaaaaccaagagtggagcgcatctgatttcactgatgaagacttaacgcttgatgaattgagtgagatcatgggagccgtcaacaaactataggagaggagattcactgatgccgcagcaacctgaaatacaggatatataccctttgtcatttatgcaggaagggatgctttttcactcactgtatgatgaacagtcgagagcttattttgaacaggcttcttttacgatccatggacagcttgacttggagcgtttccaaaaaagtatggatgctgtttttgacaggtacgatatctttcgaacagcattcatctataaaaatgtagccaaacctcgtcaagtcgtgctcaagcaacgtcattgccctattcatattgaagatatttcccatctcaatgaaagggataaagaacattgtaccgaggcattcaaagagcaggacaaatccaaaggctttgatctccaaacggatgtactgatgagaatatctattttaaaatgggcgcctgatcattatgtctgtatctggagccaccatcatattttaatggatggctggtgtttaggcatcgtcattaaagactttctccatatttatcaagcgctgggtaaaggccagcttcctgatttgcctcccgtacagccgtacgggacgtatattaaatggctgatgcagcaagatcgtgaagaagcagctgagtactggaaaaagaggcttcagcatttcgaaaaatctacacccctgccgaaaagaacagatcaaattccgaatgggacactacagcagatcacgtttgccattcccgaaaaagaaaccgccgaattacagaaaatcgcagcagcttctggtgcgacactaaacactgttttccaagctttatgggggattatgcttcaaaaggtcaatcgcagcagcgatgctgtgttcggttcagttatatcaggcagaccttctgagctaaaagatgtggaaaacatggtcgggctttttatcaataccattcctattcgagcccaaagtgattctctgtctttttctgacctagtcaggagaatgcaaaaggacatgaatgaggcagaagcctatagttactttcccttgtatgatattcaggcgcagagtgctctaaagcaagagttgatcgatcatattatcgtctttgaaaatacacctacccagcaagagatcgaagagctgaatcaagcggggtcatttgatttctccgtcaaagattttgagatggaagaggtgaccaattatagttgcagtgtcaaagtgatcccaggccgtaccttgtacgttcggattcattttcagaccagcgcttatcaaccaagcatgatgtccgaaataaaagattatttgctgcacatggtctctgacgtcatctctgatccatctcttcctgtgtcaaagatgacgttgctagatgaggacaaaacacggaaaatcgtttctcaaaataacaggacggccagtgtggcccctgaagccccaaccctgcatgggctgtttgaacgacaggcggcagtcacaccggagcggctggccattcgcttttcaggcggttcgctgacatacgctgagcttgatatgtacgccagccggctggctgcgcaccttgcggcacgcggcgtcacaaacgaaagtatcgtcggtgtcctgtctgaacgctcacctgacatgctgatcgctgtccttgctgtattgaaggccggaggggcgtatttgccgcttgatcctgcgtatccaaaggagcggctgagctacatgctgaaagacagcggggcatcgctcttgctgacacagccgggatgctccgcaccaaacttttctggcgaaacgcttgaagtggacatgacatctcttgagtgtgaagaagtaaaacgtcatgtgtctgcttctgttagcgacggatctctcgcctatgtcatctatacatcgggctctaccgggcagccgaaaggagtggccgttgagcaccgccaggctgtttcctttctgaccggcatgcagcaccagtttcggctttcggaagatgacattgtcatggtgaaaacctctttttcctttgatgcgtctgtgtggcagctgttttggtgggctctttccggtgcttcggcgtatctgcttccgcccggctgggaaaaagactccgcattgatcgtacaagccattcatcaggaaaacgtgacaacggctcattttattccggctatgctgaacagctttctcgatcaagcggaaatcgaaaggctgagtgacaggacaagcctaaagcgtgtattcgccggaggtgaaccgcttgcgccgcgtacggcagcccgttttgcttctgtattgccgcaggtatcattaatccatggctacgggccgacagaagccacggtagacgcggcattttacgtgttagatccagaacgggacagagaccgtttgcggattccgattgggaagcccgtacctggtgcgcgtttgtatgttttagatccgcatttagccgtacagccttccggtgtcgccggcgaactatacattgccggagcgggtgttgccagaggttatttgaatcggccggcattaacggaggagcgttttcttgaagacccgttttacctgggggaacgcatgtacaaaaccggggatgtggcgcgctggctccctgacgggaatgttgaattcctcgggcgcacggatgatcaggtgaaaatccgcggctaccggattgagccgggagagattgaagcggcactaagaagcatagaaggcgtaagggaggcggccgttaccgtacggacagacagcggcgagccggaattatgcgcttatgtagaagggctccaaagaaacgaagtgcgtgcacagcttcagagactgttgccgggctacatggtcccagcctatatgatagaaatggaacagtggccggttacaccaagcggaaagctcgaccgaaacgccctgccagctcctggcggagcggcagatgcggagacctacacggcgccgagaaacgtgactgagatgaagctttctcagctgtgggaggacgtgctgaaaaatggccctgtcgggattcacgacaacttttttgaccgcgggggacattccttaaaagcaacggcgcttgtctcacggatcgccaaagaattcgatgtacaggtgccgctaaaagatgtgtttgcccatccgacggtagaaggactggctaccgttatccgtgaaggaacggacagtccatatgaagcgattaagcccgctgaaaaacaggaaacctatccggtttcctctgcccaaaagcggatttatgtccttcagcagctggaggacggagggacaggctacaatatgccggctgtgttagagctcgaagggaagctcaaccttgaaaggatggacagagctttcaaagagctgatcaagcgccacgagtcgcttcggaccgccttcgaacaggacgcaggaggcgacccggtgcagcgcatccatgacgaggtgccgtttacgttacagactacagttctcggcgcacgaaccgaagaggaggccgcagccgcatttatcaaaccgtttgatctcagccaagcgccgctgttccgtgcccaaatcgtaaaggtatcagatgagcggcacctgttgctggttgatatgcatcacatcatttcagacggtgtttccgtcaacattctgattcgggaattcggcgaactgtacaataatcggaagcttccggcactgcgcattcaatataaagattatgccgtatggcaagaaggattcaaaacaggagacgcgtacaaaacgcagggggcgtactggctgaagcagctcgagggcgagctgcctgtgctggatcttccggctgatcatgcccgcccgccgatgcgaagcttcgcgggtgacaaggtctcatttacgctggatcaagaggttacatcaggcctttacaagctggcacgagaaaacggaagcacactgtacatggtgctccttgcagcttacaccgcgttcttgtcacgcttaagcggacaggaagatatcatcgtcggctcgccaattgccggccggccgcacaaggatcttgagccgatactcggcatgtttgtgaacacgctggcgcttcggacgcgcccggagggcgggaagccgtttgtacagtacttgcaggaagtgcgcgagacagcaatggaagcctttgagcaccaagattacccgttcgaagagcttgttgataagcttgaattgacacgagatatgagcagaaatccgctgtttgacgtaatgtttgttcttcaaaatatggatcaggaatcgttggagctggatgaactttgtctcaaacctgcagcaaacaatgggcatcaaacgtccaaatttgatttaaccctatatgcccaggaacagccccgcggtttgctgacgttccaaatggagtttagtactgacttatataagaaaaaaacgatagaaaagtggcttcaatacttcaacaatatgttactctccatcatcaaagacaacaaagccgctctcggaacaataaatatcctgaatgaggatgaggcccattaccttatccacgagctcaatcgtacggccatagaggccccaagaaatgaaaccatcagcagactctttgaaatgcaggcagaacaaacacctaatgctgtagcaattgtcagcgacacccaagtattcacttacgaggacctgaacagctgggcaaatcaaattgcctcagttctacagataaagggcgtagggcctgatagtgttgtagccttgttgacaggcagaacaccagaactcattgcaggaatgctgggcattctaaaagccgggggagcctatctgcctatcgattctaatctgcctgttgaacgcatagcttatatgctgtctgacagcagggcagcattactccttcaatctgaaaaaacagaaaaacggctattaggcattgaatgtgaacaaatcataatcgaagatattcaaaagcaaggagaggcgaagaacgttgaatcttcagcagggccccattcacttgcatatatcatttatacctctggatcaaccggtaaaccaaagggtgtcatgattgagcagcgaagtgtaattcgtcttgttaaaaacagcaattatattacatttacacctgaagaccgccttctgatgacatcatcaatcggtttcgacgttgggtcatttgaaattttcggaccgctgctaaatggtgccgctttgcatctgtccgatcaacaaacatttctcgattcccatcagcttaagaggtacatagaacatcaaggaatcacaacgatttggctgacatcttctctattcaatcatttgacagagcaaaatgaacaaacattttcacagctgaaacatttgattattggcggagaagctttgtcgccgagccacgtcaatcgaatcagaaatgtctgccctgaagtatctatatggaatggatatggccctaccgaaaatacaactttttcgacatgccttcacattcaaaaaacatatgaactttccattccgatcgggcggccggttggtaattccaccgcttttatcttaaatcaatggggagtgctgcagccggtcggagctgtcggtgaactttgtgtcggcggagatggcgtcgccagaggatatttgggccgtcctgatttaacgaaagagaaatttgtcccacatccatttgcacctggcgatcgactgtatcgcacaggtgatctggcgcgctggctttccgatggcacaattgagtacgttggccgtattgatgatcaagtaaaagtcagaggctatcgggtggagctgggtgaaatcgaaacagcacttcgtcaaatagacggggtcaaagaagccgcagtgttagcacgtacagcccagaccgggagcaaagagctgtttggctatatcagcgtaaaagcaggcacgaatgctgaacaagtgcgttctcttctcgcgcgttcgctgccaaactatatgatcccggcgtatatcattgaaatggagactcttccgctcacatcaaacggcaaattgaaccggaaagcactgcctgaaccagatgtcgcatctaaacaaacatacatcccgccacgcaacgaacttgaagagcagctggcattgatctggcaggaggttctaggcatccagaggatcggaatagaggattcgttttttgaattgggcggagattcaatcaaagcccttcaagtttctgcacgccttgggcgctatggactaagcttgcaggtaagtgatttattccgtcatccaaagataaaggacttatcaccatttatccgtaagtcagagagaatcatagagcaaggacccattcagggtgacgttccttggacgcctgttcagcaatggtttttttcacaagatattgaagaaagacaccatttcaatcagtctgtcatgctattccattctggacgtttgtctgaaaacgcccttagaccagccttgaaaaaactggcggagcatcatgatgcgcttcggatggtttatcgcaacgatgacaggcgatggattcaaatcaaccaaggcattcatgagtcacagctatacagcttaagaatctctgatctttcacagtcagaaagcggctgggagacgaaaatcaaacaagaagttgccgatcttcagcaaagcatcaatttgcaggaaggaccattgttgcacgccgctttgtttaaaacactgaccggagattacttgttccttgcgatccatcaccttgtcgttgatggtgtctcatggcggattttgctggaggatttgtcagccggatatcaacaagctgctgcaggccagacgatccagcttccgcctaaaacggattcctaccaggaatacgcaagacgcatacaggaatatgcccaaagcagtaagctgattcgcgaagaggcgtattggcgaagtgtagaagaacagcaagccgcagaactgccctatgaaataccgcatcatgtgaacatcgacttcagcaaaagggactcattaagcttttcactgactgaagcagacaccgccgtcttgctgcaaaacgtcaatcacgcctatggcacagatacacaagatattctgttaaccgcagcatccttggcgatttgtgaatggacaggaggaagcaagctccgtatcgctatggaaggacacgggagagaacacattctgccagagttagatataagcaggacggtcggctggtttacatccatgtacccggccctcataagctttgaaaatcatagggatgagctcggaacctcagtaaaaaccgttaaagatacactgggccggataccaaacaaaggggtaggttacggtatgctgaaataccttacacaccctgaaaataaaagcattacgttttcaaaaacacctgaaatcagctttaactatttgggccagttcaacgacatcgaaagacaggacaccttccgcccatcaagccttggtagcggaaaggatatcactcatacatggaagcgcgagcaaatcatcgagatgagtgcaatggcagcagacaaaaagctccatttcaatcttagttatccgccagcccgctttcacagaaacacaatggaacagcttattaacaggattgaacactttttgctggacattatgaaacactgcgccggtcaacagaaagcagaaaagacactgagcgatttcagcagtcaatcattaacggcagaggacttggacagcatatccagcttggtggaagaattgtagaaaatcgtgacaggagacatgaacatgacaaaagcgaattcaattcaggatatttatccgctgtcttacatgcaggaagggatgcttttccattccctcctgcaaaaagattcacaggcgtatgttgagcaagcttcttttacaatagaaggaaaagtcaacccgcagttttttcaaaacagcatcaacgctcttgtagaaagacatgatattttcagaacgatttttatcagccaaaatgtttcctccccccagcaggttgttctgagagaacgaaatgtcatcgtactggaagaagacattactcatttaaacgaggcggagcaatcacagtttatcgagcaatggaaagaaaaggaccgggaccgggggtttcatttgcaaaaggatgtgctcatgcgcatcgctctgattcaaacaggagagagccagtactcttgcatttggacctttcatcatatcatgatggacggttggtgcctcagcattgtgctaaaggagtttctgcatatttacgcatcttatgtaaatgcatccccaataacattggagccggtccagccatacggaaagtatatcaaatggctgatggagcaagacaaagagcaggcggtttcttattgggatcattatctttccggccacgaacagcaaaccgtgctcccgaagcagaaaaaaacaaagggaaaaagcaggcaggaacacgttacattttcattctctaaggaagaaagcagcaggctttcagagcttgctgctagagaagaagtgacactcagtacgatttttcataccatttggggcattctgctgcaaaaatataataataacgatgacgccgtattcggttctgtcatttcaggaagacccgcagaaatcgaaggcattgaacatatggtaggtcttttcattaatacgatgccggttcgggtgcagggggcaaaaacgccttttcttcaacttataaaagatatgcaaaaagaccgtcttgccgctgaagcgtacagctaccaccctttatatgagattcaatcccgctcagctgttaagcaagggctgattgatcatattctcgtatttgaaaactatccggtgcagcaagagattcaaatgctgaacaaacaggaacatgcttctgatctttttcagattcataatttcactgtcgcagatgaaaccaactacagcttttatcttatggtggcgccaggggaagaaattcatatcaaaatgaactatgatgcggagcagcacgatcggtcttttgtgctctctgtcaaagagcatcttctgaatgctgtatcacaaatcttaaataatccgaatcttccacctgaagaaatcgatatcacgacagatactgaaaagcggcagctgattggagaaatcacagatcaggccccagaggcccctgaaggaatggctgttcaccaagtgtttgaagagcaagcgaaacggacgccggcgagcaccgccgtcgtatatgaaggaaccaagctgacgtaccgcgagctgaatgcagcggctaaccgtctggcgagaaagcttgtcgaacatgggcttcaaaaaggggaaacagcagcgattatgaacgaccgctcagtagaaaccgttgtcggcatgctggctgttttaaaagcaggcgccgcatatgtgccgcttgatccagcgcttcctggggatcgtcttcgtttcatggcagaggacagctccgttcgaatggttttgatcggaaattcttatacagggcaggcacatcagctgcaagtgccggttcttacactggacataggctttgaagagagtgaagcggctgacaatctcaacctgccatccgccccgtctgatttggcgtacatcatgtacacatccggttcaacgggcaaaccgaaaggcgtcatgatcgaacataaaagcattctgcgcctcgtcaaaaatgccgggtacgttcctgttactgaagaagaccgcatggcgcaaacgggagctgtcagctttgatgccggaacgtttgaggtattcggcgcactgctgaatggcgcagcactttatccggtcaaaaaagagacactgcttgatgcgaaacaatttgctgcattcctgcgtgagcaaagcatcacaactatgtggctgacatcacctttattcaaccagcttgctgcaaaggatgcgggtatgttcggcacactgcgccatttaatcatcggcggagatgcccttgtcccgcatattgtcagcaaagtaaaacaggcatcgccgtcgctttcattgtggaacggatacggcccgacagaaaacacgacgttttcaaccagttttctgatcgaccgcgagtatggcggctctatcccaatcgggaagccgatcggaaattccactgcctatattatggatgagcagcaatgcctgcagccaatcggcgcgcctggtgagctttgcgtaggcggaatcggtgtagcgcgtgggtatgtcaatctccctgagctgacggagaagcaatttctggaagacccgttcagaccgggtgagagaatttaccgcactggtgacttggcaagatggctgccggacggcaatatcgaatttttaggcagaatcgacaaccaagtgaaggtgcgcggcttccgaattgagcttggcgaaattgaaacaaaactgaacatggctgagcatgtgacagaagccgcggtgatcatacgcaagaacaaagcagacgaaaatgaaatttgcgcgtacttcacggcggatcgtgaagtggctgtgagtgagctgagaaaaacactgtctcagtctttgcctgactatatggtccctgcccacctgattcaaatggacagcctgccgctcacgccaaacgggaaaatcaacaaaaaggaactgcctgcaccgcaatcagaagccgtgcagccggaatacgcagcaccaaaaacagagagtgaaaagaaattagcggagatctgggaaggaatactcggcgtcaaagcaggcgttaccgataacttctttatgatcggcggccattctttgaaagcgatgatgatgacggcgaaaattcaagagcattttcataaggaagttccgataaaagtgctttttgaaaagccgactattcaagaactggcactgtatttggaagagaacgaaagcaaagaagagcagacgttcgaaccgatcaggcaagcatcttatcagcagcattatcctgtatccccggcccagcggagaatgtatatcctcaatcagcttggacaagcaaacacaagctacaacgtccccgctgtacttctgctggagggagaagtagataaagaccggcttgaaaacgcgattcagcaattaatcaaccggcacgaaatcctccgtacatcgtttgacatgatcgacggagaggttgtgcaaaccgttcataaaaacatatcgttccagctggaggctgccaagggacgggaagaagacgcggaagagataatcaaagcatttgttcagccgtttgaattaaaccgcgcgccgctcgtccgttcgaagctgtccagcttggaagaaaaacgccacctgctgctcattgatatgcatcatattattactgacggaagttcaacaggcattctaatcggtgatcttgccaaaatatatcaaggcgcagatctggaactgccacaaattcactataaagattacgcagtttggcacaaagaacaaactaattatcaaaaagatgaggaatactggctcgatgtctttaaaggcgaactgccaatactggatcttcccgcggatttcgagcggccagctgaacggagctttgcgggagagcgcgtgatgtttgggcttgataagcaaatcacggctcaaatcaaatcgctcatggcagaaacagatacgacaatgtacatgtttttgctggcggcgttcaatgtactcctttccaagtacgcgtcacaggatgatatcattgtcggctcgccgacagctggcagaacacatcctgatctgcaaggtgtgccgggtatgtttgtcaacacggtggcactcagaacggcaccagcgggagataaaaccttcgcgcaattccttgaagaggtcaaaacagccagccttcaagcattcgagcaccagagctatccgcttgaggagctgattgaaaagcttccgcttacaagggatacaagcagaagtccgctgttcagcgtgatgttcaacatgcagaatatggagattccttcattaagattaggagatttgaagatttcctcgtattccatgcttcatcatgttgcgaaatttgatctttccttggaagcggtcgagcgtgaagaggatatcggcctaagctttgactatgcgactgccttgtttaaggacgagacgatccgccgctggagccgccactttgtcaatatcatcaaagcggccgcggctaatccgaacgttcggctgtctgatgtagatctgctttcatctgcagaaacggctgctttgctagaagaaagacatatgacggccatgacggccgcaacctttgcagcactttttgaaaaacaggcccagcaaacacctgaccattctgcggtgaaggctggcggaaatctgttgacctatcgcgagcttgatgaacaggcgaaccagctggcgcatcatcttcgtgcccaaggggcaggaaatgaagacatcgtcgcgattgttatggaccggtcagctgaagtcatggtatccattctcggtgtcatgaaggcgggggcagctttccttccgattgatcctgatacacctgaagaacgaatccgttattcattagaggacagcggagcaaaatttgcggtcgtgaatgaaagaaacatgacggctattgggcaatatgaagggataattgtcagccttgatgacggtaaatggagaaatgaaagcaaggagcgcccatcatccatttccgggtctcgcaatcttgcatacgtcatttatacgtccggtacgaccggaaagccaaagggcgtgcagattgagcatcgtaatctgacaaactatgtctcttggtttagtgaagaggcgggcctgacggaaaatgataagactgtattgctttcatcttacgcatttgaccttggctatacgagcatgttccctgtacttctgggcgggggcgagctccatatcgtccagaaggaaacctatacggcgccggatgaaatagcgcactatatcaaggagcatgggatcacttatatcaagctgacaccgtctctgttccatacaatagtgaacaccgccagttttgcaaaagatgcgaactttgaatccttgcgcttgatcgtcttgggaggagaaaaaatcatcccgactgatgttatcgccttccgtaagatgtatggacataccgaatttatcaatcactacggcccgacagaagcaacgatcggcgccatcgccgggcgggttgatctgtatgagccggatgcatttgcgaaacgcccgacaatcggacgcccgattgcgaatgccggtgcgcttgtcttaaatgaagcattgaagcttgtgccgcctggagcgagcggacagctctatatcacgggacaggggctcgcgagagggtatctcaacaggcctcagctgacagccgagagatttgtagaaaatccatattcgccgggaagcctcatgtacaaaaccggagatgtcgtacgaagactttctgacggtacgcttgcatttatcggccgggctgatgatcaggtgaaaatccgaggctaccgcattgagccgaaagaaattgaaacggtcatgctcagcctcagcggaattcaagaagcggttgtactagcggtttccgagggcggtcttcaagagctttgcgcgtattatacgtcggatcaagatattgaaaaagcagagctccggtaccagctttccctaacactgccgtctcatatgattcctgctttctttgtgcaggttgacgcgattccgctgacggcaaacggaaaaaccgacagaaacgctctgccgaagcctaacgcggcacaatccggaggcaaggccttggccgcaccggagacagcgcttgaagaaagtttatgccgcatttggcagaaaacgcttggcatagaagccatcggcattgatgacaattttttcgatttaggcggccattcattaaaagggatgatgctgattgccaacattcaggcggaattggagaaaagcgtaccgcttaaagcactgttcgagcagccgacagttcgccagctggcggcttatatggaggcgtctgctgtttcaggcggccatcaagtactcaaaccggctgacaagcaggatatgtatccattgtcatccgcacagaaacgaatgtacgtgctcaatcagcttgaccgccagacgataagctacaacatgccatctgttcttctaatggaaggagagcttgatatttcgcgcctgcgcgactcactcaatcagcttgtgaaccgtcacgaatcattgcggacgtcatttatggaagctaatggtgagcctgttcagcgcatcattgagaaggcggaggttgatcttcatgtgtttgaagccaaagaagacgaagcggaccaaaagattaaggaatttatccggccattcgacttaaacgacgcaccgctcattcgcgcagctttgcttcgaatagaagcgaaaaaacatttgctgcttttagatatgcatcatatcatcgcagacggcgtctcaagaggcatctttgtaaaagaattggcgctgctttacaaaggagagcagcttccggagccgacgcttcattataaagatttcgccgtttggcaaaatgaagctgagcaaaaagaacggatgaaggagcatgaggcgtactggatgtcagttctttcaggcgagctgccagagcttgatctcccgctcgattatgcccgtccgcctgtgcaaagctttaaaggagatacgatccgtttccgtacgggaagtgagacggcaaaggcggtagaaaaactgcttgccgaaaccggaacgaccttgcacatggtgctccatgctgttttccacgtctttttaagcaaaatttccggacagcgggatatcgtcatcggctccgttactgccggccggacgaatgctgatgttcaggacatgccgggaatgttcgtcaatacacttgccctgagaatggaagcgaaagaacagcaaacatttgcggagcttttggagctagcaaagcagacgaacctgtcagcccttgagcatcaggagtatccgtttgaagatctggttaatcagcttgatctccctcgggatatgagccgaaacccattgtttaatgtgatggtgacgacagaaaaccctgataaagaacagcttacattgcaaaatctgagcatttcaccttatgaggctcatcagggaacttctaagtttgatctgacactgggcggatttactgatgaaaatggcattggcttgcagctcgaatatgcgacagatctgttcgcaaaagaaacagctgaaaaatggagcgaatacgttctgcggctactaaaggctgttgcggataacccgaaccagccgctttccagtctgttactggtcaccgagacagaaaagcaagcgcttcttgaggcatggaagggcaaggccccgaaggcctacggagttcaaacaatcagtcaattgtttgagcagcaagctgcacgaacaccaaaagcttctgcacttgtcagcggagacaaaacactcacttatcaggagcttgacgagtggtccaatggaatcgcacgtgcattgcgcagccgaggtgttaagccggacacaccagtaggcatcatgatgcatcgttcgttcagtatgatagcatccatacttggtgtgtggaaagccggaggctgttacgttcccattgatcctgaatacccgaaagaacggaaacgctatatcctcagcgacagcggaacgaaactgctgatgacaataaatgaagcggatctgggagtacttgctgactttgaaggagagatcttgacgatagaaagcgtagaggaagacgacaaatcgccgctgccgcaaatgtcgtctgcccatcatttggcttatatcatttatacttcaggaacgacgggccgtccaaaaggggtaatggtcgagcataaagggattgctaacactcttcagtggcggcgaaacgcttatgcattcaacgagacagataccattctgcagctcttttctttctcatttgacggctttataactagtatgtttacaccgcttttgtcaggtgcaaaagccgttttgcttcatgaagaggaagcgaaggatattctggccattaagcatcagctgtctcgtcaacggattacacatatgattattgtgcctgttttatatcgagcgcttttggacgtagtgcagccggaagatgtaaagacgcttagagtcgtcacactggcgggagaagcggctgaccgcgaattgatcgcccgcagcttagctatatgtccgcataccgaactcgccaacgaatatggaccgacagaaaacagcgtggcgactaccgtcatgagacatatggaaaagcaggcatacgtaagcatcggccagccgattgacggaactcaagtgctgattttaaatagcaatcatcagcttcagccaatcggtgttgcgggagagctttgtatagcaggaacagggcttgcaagagggtacgttaatcttccagaactgacagagagagcattcacgcagaatccatttaaacccgaagcacgaatgtaccgaacaggagacgccgccagatggatggccgacggtacactcgaatatctcggaagaatcgatgatcaagtcaaaatcagaggataccgtgtagaaacgaaagaaattgaatcggtcatccggtgtataaagggtgtaaaagacgccgcagtagttgctcatgtaacagcgtcaggacaaaccgaattaagcgcttatgtggtgacaaaaccagggttgagcacaaatgctgtacgctcagaattacaaaacaagctgccggtgtttatgcaccctgcgtttattgaaaaactggactcacttccattgtcaccaaacggcaagctggatcgcggagcacttccaaaacctgtatacaaccacgaaggtgaacgtccattcctcccgccatccagcaaaatggaacaaatactggcagatatatggaaagaagtactgggggcagaaaagatcggaacagctgattcgttctttgaacttggcggagattcaatcaaagcgttacaggtatctgcgcggcttcaccggataggcaagcaaatggcagtgaaagatttgtttagccatccgaccattcaagaattggcagcttatatccgtgattcagatacaagttccagccaagctgcggttgagggagacgtacaatggtcgcctgttcaaaaatggtttctttctcaagatataaaagaaaaacaccattttaatcagtccgtaatgctgcatcgaagcacctctgtacaagaagacgcactgcgaaaaacgttaaaagcaataacgtgtcatcatgatgcgctgcgaatggtgtttacacagaatgaacaaggaaagtgggatcaatataatcggccgctcagtcattcggacgacgcgttgtacggccttcagatgattgatttgtcagctccggacggcactgatggaaatagaccgtatgaacctcttatcaagcgccatgtacttgatattcagcagaaaatggatttgaagaatggtccgctgctgcaagccggtcttttccacacaattgacggtgatttcttatttttatctgctcatcacctcgtcgttgacggcatctcatggcgggttctgcttgaagatttggctttagggtatcgccaagctgctggcggggaggatatcaaactgccgcctaaaacaagctcgtttaaagcgtatgcgaaaaagctctctgactacgctgaaagccagcagctaatgaaacagctcaagtattggcgcgaagccgaagagtatcaaacagaggcattgccttttgatcaaatcgatggaactagagcacacgagggacaacggtccacaatttcgtttaccttaaacgataaagagacagcagcactcttaaaagacgccaacagcgcatataacactgatacgcaggacatgctgctcgcttctgtcattcttgcgctgcgccattggaccaatcaatccgccttcaaactatcattagagggccacgggcgagaggatgtattaaaaggaatagatgtgagccggacgattggatggtttaccgccatttatccgttattgattaaactgaacgcagacttgccagattcggaagaaagcatggttcatgtgctaaaaacaacaaaagatacactgagacgtgtacctgacaaaggattcggctacggtgtcatcaaatatttgactccgcctggcaaaaaagacatcaatttcacaggtgcaccagaaatcagctttaattatcttggtcaatttgaaagcggccgcacagctgaagtacctgaggaggacgccttctcattctctccgctgggtgccggaggtgatatcagcacaacatggaaccgtgaacagtcgctggatatcagcgcaatcgctgcagaaggaaaattgactgtcaatatgacttatgacaatgcccgctttcagcgcaaaaccatcgaacagcttagcgaaacatgccgtcaatttttattacagctgatcgaacactgccagaacaaaagcgaaacagaaaagacgatcagtgattttgatgatcaagaactgaccgaggacgccctgcaagagatcgctgatatgctcagttttcactaatgaatccgtgaagaaaggtgcagacactatgaataccattaaaaaaatcaagaacatttatcctctgagtcatatgcaggaagggatgctgtttcattccttcctccgtaaagaggagggggcgtatgttgagcagtcgctcttcaccattaaaggaagcctcagctatgactggttccagcgcagcattcaagccattatcgaccgccatgatattttcagaaccgtgtttttgccgcacgtcccgcatttgtcgggacctcggcaagtcgtgatgacagaacgtgaattccatttgaacagcgaagacatttctcatctgccgacaaacgaccagaatgagtatattgaacgctttaaagagaaggacaagcaaaaaggctttgatctgcaaaaagacatgctgatgcggatttctctattcaaaacagctaaagatgagcatgtctgtatctggagtcaccatcacattttaatggacggatggtgcctaggtatcgttatgcaggaatttatgcaaatttatcaatcgattcatgcaggaaaaccgctttcattagaccctgtccgtccgtacagcacctatatttcatggctgacaaaccgagacaaagaaaaagcagcggcctactgggatacctatttaaaaaactacagcgctccatcacctctgcctcgtgtgtctgataaagaaacaaaagaaagttatcaccgtgaagatttgatattttcattaaataaaccactgacagacaagctgaaagagactgccaaacaacacggcgtcacgctcgctacccttattcaggcagtctggggtgtgatgctgcagcaatataaccgcacagacgacgttgtgtttggcgcagttgtatcaggaagaccgtcagaaatcccaggcgtggagcaaatgatagggttgtttatcaataccataccgattcgaattaaaacacaccaagacgaaacgtttcacgagctgctcatacgctgccagaaagaaatgctggaagctgagccgtttacctgccagcctttatttgatattcaggcaaacaccgcattaaaacaggaactgattgatcacattatcgtctttgaaaactatccgttacagcagaaaatcgccgattccgctgatcaaaccgattcaccgctgcaaatcgatcaagttcaagtatccgagcaatcaggatataactttaatcttgtcgttgctcctggcgaagagcttgtcatcaagttcagctataatgcattcgtttacgatgctgcctggatcagctgtatcaagaggcaatttacgcaagcgcttagcacagctgcacagcaccctcatatgccaattgctgatttttcttttcttgatgcaacagaaaaagagcagattgtcacacagttcaacaatacggccacggaggccccaaagaatcatacaattatcgatttatttcgcgaacaagcagaaaagacgccagaccataccgcacttgtgtatggcaatatgtctatttcgtataaagagcttgataaacgctctaatgcgctcgccagagagttaattcaaaagggatttcggaaaaacgagacagccggaatattggctgcacattctcccgaattcatgatcagtgtgcttgccgtattaaaagcagggggagcatacctcccgcttgatgcggagcttccgcctgaacgagtcagctttatgcttgaggaaacgcaggcaaaaatgctgattgttcaaaagggattggagcaaaacgctgcgttctcaggaacatgtatcatttcagatgcgcagggattgatggaagagaacgatatccctattaatatcagctccagcccggatgatcttgcgtacatcatgtatacctcaggatcaacaggccggccgaaaggggtcatgatcacgaatcgcaatgtcgtgtcccttgtcagaaacagcaattacacgtctgcgtccggtgatgaccggtttattatgactggatctatcagctttgacgccgtcacctttgaaatgttcggggcacttttaaatggcgcaagccttcatatcattgataaatcgacaatgctgacacctgatcggtttggagcgtatttgcttgaaaatgacattacagtgctatttttaacgacagctctttttaatcagctggcacaggtacgagctgacatgtttcgcggactccatacgttatatgtcggaggagaagcactctctcctgccctgatgaatgccgtcagacacgcctgtccagatctcgcgcttcataatatttacgggccaacggaaaacacgactttttcaaccttttttgaaatgaagagagactatgcggggccgattccgattggaaaaccaatcagtaatagcaccgcttacatcttagatacaaaaggacgtcttttgccaataggcgttcccggcgagctttgtgttggcggtgatggagtcgctaaaggctatttgaacagagtagatctgacaaatgctgtgttttctcctcatcctttcttgcctggagaaagaatataccgtactggtgatttggcgcgctggctgcctgatggaaacttagaatacatcagcagaattgacaggcaaatgaaaatccgcggaaaacgaattgagcctgccgaaatagaagcgcgcctgttagaaatggaaggcgttcaagaagcagcagtgacattgagagaaaaagatggagaggcgcagctgtacactcattacgtcggtgatcacaaaaaaacagatacggattttcgcgccgatttggcgcgtgtgcttccagactatatgatcccgcagcactgggtgcgtgtggagcggatgccgcttaccggaaacggaaaaatagaccgcagcgcgctgcctattccagaaaataagcctgccaaacgacagaacatcatattgccaagaaacttggttgaagaagaattggcgaacatttggaagcaagtcctcggtgttaacacaatcagtattgatgatgacttctttgctattggcggacattcactaagagcactgcaagtcatacatacactaaaacatcagcagaacattgacataccgattgatttcttgttcgaacatccgacaatcgctcagcttgccgaaaaactttattctaaacagctgacagcagcaaatgaacagcatgtgatcaaactgaaccagcacggcgcgcaaaatcttttctgcttcccgccgatatcgggatttggcatttattttaaagaccttgctttattgctgaatgagaaggcagccgtatacgggtttcactttattgaacaagacacccgcattgaacaatatgttaattgcatgacggacatacagcctgagggcccatacgttttattaggctactctgcaggcggaaacctggcttttgaagtggcacaggctatggagcgcaaaggattagaagtcagcgacttcattatcgtggacgcttatctaaaagaacagcctttgcctatcgataccggtaatgacgaatctgcagcatatctgcctgaagcagtcagagaaaaggtgatgaagaaaaaaagaaactatcaggaatattgggcacaattgctgaatgaaggccacatcaaagcaagcattcatttcatcgaagctggaatccaccccgaaaccagcgggcatacaggcttaacgaaatgggaaggcgcctgcggaaactatagtgagtacacgggttttggcgctcataaagacatgctggaaggaacatatgctgaaaagaatgccgacatcatcctcgacattttagaaaagatcacttcaaatcaagtaatactgcacaaacgataaagcggattagcggacagaggccattctctgtccgtctttctttttgtatggccgtctgtgagctttaatgcggtagtttatcacagttaaattgctaacgcagtcaggcaccgtgtatgaaatctaacaatgcgctcatcgtcatcctcggcaccgtcaccctggatgctgtaggcataggcttggttatgccggtactgccgggcctcttgcgggatatcgtccattccgacagcatcgccagtcactatggcgtgctgctagcgctatatgcgttgatgcaatttctatgcgcacccgttctcggagcactgtccgaccgctttggccgccgcccagtcctgctcgcttcgctacttggagccactatcgactacgcgatcatggcgaccacacccgtcctgtggatcctctacgccggacgcatcgtggccggcatcaccggcgccacaggtgcggttgctggcgcctatatcgccgacatcaccgatggggaagatcgggctcgccacttcgggctcatgagcgcttgtttcggcgtgggtatggtggcaggccccgtggccgggggactgttgggcgccatctccttgcatgcaccattccttgcggcggcggtgctcaacggcctcaacctactactgggctgcttcctaatgcaggagtcgcataagggagagcgtcgaccgatgcccttgagagccttcaacccagtcagctccttccggtgggcgcggggcatgactatcgtcgccgcacttatgactgtcttctttatcatgcaactcgtaggacaggtgccggcagcgctctgggtcattttcggcgaggaccgctttcgctggagcgcgacgatgatcggcctgtcgcttgcggtattcggaatcttgcacgccctcgctcaagccttcgtcactggtcccgccaccaaacgtttcggcgagaagcaggccattatcgccggcatggcggccgacgcgctgggctacgtcttgctggcgttcgcgacgcgaggctggatggccttccccattatgattcttctcgcttccggcggcatcgggatgcccgcgttgcaggccatgctgtccaggcaggtagatgacgaccatcagggacagcttcaaggatcgctcgcggctcttaccagcctaacttcgatcattggaccgctgatcgtcacggcgatttatgccgcctcggcgagcacatggaacgggttggcatggattgtaggcgccgccctataccttgtctgcctccccgcgttgcgtcgcggtgcatggagccgggccacctcgacctgaatggaagccggcggcacctcgctaacggattcaccactccaagaattggagccaatcaattcttgcggagaactgtgaatgcgcaaaccaacccttggcagaacatatccatcgcgtccgccatctccagcagccgcacgcggcgcatctcgggcagcgttgggtcctggccacgggtgcgcatgatcgtgctcctgtcgttgaggacccggctaggctggcggggttgccttactggttagcagaatgaatcaccgatacgcgagcgaacgtgaagcgactgctgctgcaaaacgtctgcgacctgagcaacaacatgaatggtcttcggtttccgtgtttcgtaaagtctggaaacgcggaagtcagcgccctgcaccattatgttccggatctgcatcgcaggatgctgctggctaccctgtggaacacctacatctgtattaacgaagcgctggcattgaccctgagtgatttttctctggtcccgccgcatccataccgccagttgtttaccctcacaacgttccagtaaccgggcatgttcatcatcagtaacccgtatcgtgagcatcctctctcgtttcatcggtatcattacccccatgaacagaaatcccccttacacggaggcatcagtgaccaaacaggaaaaaaccgcccttaacatggcccgctttatcagaagccagacattaacgcttctggagaaactcaacgagctggacgcggatgaacaggcagacatctgtgaatcgcttcacgaccacgctgatgagctttaccgcagaattcgcccttcccggtcgatatgaacagcttatttacataattcacgttattggtagttataaatgaaattcctaatatcggttatgaagtgaaattgaatttctacttgatctttctctctatttttgtaaaataaaattaagaatatttaaatattcaatgattcatttttgcagaaatcggaggaagaagaatatatgaaaacatttaacatttctcaacaagatccccccatattgttgtataagtgatgaaatactgaatttaaaacttagtttatatgtggtaaaatgttttaatcaagtttaggaggaattaattatgaagtgtaatgaataatgaatgtaacagggttcaattaaaagagggaagcgtatcattaaccctataaactacgtctgccctcattattggagggtgaaatgtgaatacatcctattcacaatcgaatttacgacacaaccaaattttaatttggctttgcattttatctttttttagcgtattaaatgaaatggttttgaacgtctcattacctgatattgcaaatgattttaataaaccacctgcgagtacaaactgggtgaacacagcctttatgttaaccttttccattggaacagctgtatatggaaagctatctgatcaattaggcatcaaaaggttactcctatttggaattataataaattgtttcgggtcggtaattgggtttgttggccattctttcttttccttacttattatggctcgttttattcaaggggctggtgcagctgcatttccagcactcgtaatggttgtagttgcgcgctatattccaaaggaaaataggggtaaagcatttggtcttattggatcgatagtagccatgggagaaggagtcggtccagcgattggtggaatgatagcccattatattcattggtcctatcttctactcattcctatgataacaattatcactgttccgtttcttatgaaattattaaagaaagaagtaaggataaaaggtcattttgatatcaaaggaattatactaatgtctgtaggcattgtattttttatgttgtttacaacatcatatagcatttcttttcttatcgttagcgtgctgtcattcctgatatttgtaaaacatatcaggaaagtaacagatccttttgttgatcccggattagggaaaaatataccttttatgattggagttctttgtgggggaattatatttggaacagtagcagggtttgtctctatggttccttatatgatgaaagatgttcaccagctaagtactgccgaaatcggaagtgtaattattttccctggaacaatgagtgtcattattttcggctacattggtgggatacttgttgatagaagaggtcctttatacgtgttaaacatcggagttacatttctttctgttagctttttaactgcttcctttcttttagaaacaacatcatggttcatgacaattataatcgtatttgttttaggtgggctttcgttcaccaaaacagttatatcaacaattgtttcaagtagcttgaaacagcaggaagctggtgctggaatgagtttgcttaactttaccagctttttatcagagggaacaggtattgcaattgtaggtggtttattatccatacccttacttgatcaaaggttgttacctatggaagttgatcagtcaacttatctgtatagtaatttgttattacttttttcaggaatcattgtcattagttggctggttaccttgaatgtatataaacattctcaaagggatttctaaatcgttaagggatcaactttgggagagagttcaaaattgatcctttttttataacaggaattgggcatcaaataaaacgaaaggctcagtcgaaagactgggcctttcgttttatctgttgtttgtcggtgaacgctctcctgagtaggacaaatccgccgggagcggatttgaacgttgcgaagcaacggcccggagggtggcgggcaggacgcccgccataaactgccaggcatcaaattaagcagaaggccatcctgacggatggcctttttgcgtttctacaaactcttcctgtcgtcatatctacaattctacacagcccagtccagactattcggcactgaaattatgggtgaagtggtcaagacctcactaggcaccttaaaaatagcgcaccctgaagaagatttatttgaggtagcccttgcctacctagcttccaagaaagatatcctaacagcacaagagcggaaagatgttttgttctacatccagaacaacctctgctaaaattcctgaaaaattttgcaaaaagttgttgactttatctacaaggtgtggcataatgtgtggaattgtgagcggataacaattaagctaattctatggtaaaagcattcctgaacccaatatccttatttttagtggacaaggccttgttctcatatggttgcttgagccagtgccttacaaggctcttccgctttggcaggctgttcaaaattatttattagagcaactcaaggaactaggcggagatccaaaagcaaccgatgcagcacgtgtttttcggattgctgggagcgtcaatagtaagaatggagcggaagtaagagcggaatatcggcacgattacagatatgagttaaggcagattcaatttgattaccttccagaactcaatgaggttattaatcccgctccacaaaagaaaaaacgggggcgtaaaaagaaagtagttcagttattcaatacctacaaactccattacgctcgcctattggatatagtgaaattggtggaactacgaaattatgaggtaactggatacagggaaatcatttgctttttataccgttattggttgtgctgttacacgaacgaccctgtagaggctttaaatcaaacacagacacttaatttacagttcactgagcctttacccttaaaagaggttgaaagggctacacggagcgcagaaaaggcgtgggaagcacgaaataacgaagaggctaaccggattgcaatcgaaaaaggatatcccagtgctggatacaatattagcaataaaaagttgattgaatggctagatatcacaccagaagaacagaagcatttacagacgattatagacgctaatgagaaacggagaagaaagcgggaaagggataggatttatcaagaacaaaaacgtcgtgagcggggagatatgacccgacaggagtatattaagcaacaacaggataaaacagatgataaattatttaaattgcaggagttattagaacagaatcccaaaatctcaaaaattaaattagcaaaaatacttggtgtagataaatcgcacttatacagactgctgaaacaactataactggaaaaaattagtgtctcatggttcgtcgcccttatattatgggcgttagcctgcttgctaattggataggtgttattgtcatttcaacgtcggacgttttggtagatgaacgtcggacgttatttgcttcaatagattgttgatgtattaagggttgcagtgaatcgacaagcaaaaagttatgacgttgtgaaaaaattgaatagaaaattggaaattacgtcggacgttctaacttaaaaaccctgttatatcaatgatttaaaaggaaattaacgtcataaaagacctttctgcaacaaaagtttttctggaagagttgaggttattttataggtattatggacttttgtagactttttgtgtactttttgtggactccacactcgctggtatcgtgttattttttaattgagatatgaatatggaaattaaacgttttaggcgttggtttggtgatgacaaaaaaataagagtacccgctcacaacggatactctttcgagaaatgtacgaaacgctataaataaaaaataactagatacatttacattgtatcacgtttcgtacatttctccaataacaaattgattggaggaatgcaaagtgaataatgaaccagtaaaacgtggtaagaagaacagatgggaattaaacctacctataatgacttatgtagtagctgatgattggattgataaactaggacacgaaacgtttactttatggttgaggttccatacttgggtagatagagaagatgaactccgagattatgatcgcatacctagaagttttgagaacatatataaaaagacactaggaatctcaaaaagtaagttttatagattgataaaacctttatgggaatatggattaatagacatcatagaatacgaagaatctaaccgtaattctactaaacctaaaaatataattgtttatgagtatcctttacacgaaatagaaagaaagtataaaccactagaaaaattaagagattgggataaagactataattccgtttctaaagaattaggtaaaacaggtggtagaccaaggaaaaaagatagtgaagaagaacccgaaaagaaacccgaagaagtaactaaaaagaaacgtaaatataagttaaaaagagttatccacaacggtttcaaaaatgaaacggtggagggtttcaaaaatgaaacggtggagggtttcaaaaatgaaacggtgaccgtttcaaaaataaaacccaataattattcaaatatctttaataacttatcaaatatttctactaatgtttcaaataatttattaattgatgatgatgaggaaatcgaaaatgaaccaactggtcgtacaataaataggtcattacttttttcacaagaagatattaaacaggcctatcaatttattaatagattttcagttatacagttacgtgaaaactttagctttgataaacactttgaagaacggttggtatgttatttatggaaagcagggatttctactttttacacgcacgaaatcagtaaaatgataaaaaaaatagcagactatgaaaaatctaaaaaaggtagattaaacccaatacgtgaccgagccttatatatggtaaatggtcttgtaatgaatagagcttcttcccaaagtgaacatgctacttataaactaaaccaatataaaaaacagaaggaacaggaaaaacaacaacaggagcaacaaagatcaagagtaccgttctataattggttggaggaaagagaagaacaaaccgaaggtcaactacccaccacttaaagcctaacggcttttgaagtggggcttgtaaaaagccctagttgactaccccaagtctttcgaggactacgttggaaaggtcatgacacctacaaatgctcctctagttcgtagccactgtcgttgatggttaaaagtcctgatgggtagggacggtgctgtcaacatcacaagcccttccaacatgggggaagaggaagaacactccgagaaaggagggggctgtcgtacacgccttgttcgtgtacgtgatttttaacacttttatctctaatataatctctccttgagttagcagagactaagaataaaacacattaggattttttatctacataaggaggttcaatacatgcctactatttcgtttaagggaaagtcttttgtacaaaatcatcacttgactgtaaaatatcatgaattgatcccagaaccagaaaaaagtctgaccgataaagttagtcttcatgacaatcttatcattcatggggacaatttaaaggcgttgaaagctctactacctacatatgctggtaagatagattgcatctatattgacccaccatacaatactggaactgaaaaatggatttataatgataatgtcaactccccaatgattagggaatggcttggaaaagtggtagacaaagaagacttatcccgacatgataagtggctttgtatgatgatgccgaggttaaaactgttgaaagagttgttgtcagaagacggagtgatatttgtaagcattgactacaatgaaatacaccatcttacgtgccttatgaacgaaatattcggtgaggagaattttcgtgacgctattatcattcgtagaggagtaaaaaatgttcaagcgcaatttgacacaattgattctctttcaaatggttatgagtctattttggtttacactaaacagccatctcgacgatttaataaggtttatgaagatgtagaagaaaagcctggtagttggaataatcattggagaggtacagaccgtaaaactatgagatatgaattatttggggttactccgacagaaggtcaatggagatgggggaaagaacgtagtctccaggctattgaaaactatcaaatgatgttagatgaacttagacaaaaaggcattactaatccaactcaagaggatattgataaatggtatcttgaatatgtagaaaataatggggaagatattgacttgttacgacaaaatgataatggcacgattgagcactttgttccaccgactagcaaaaagttgttaagtaatgcctggtttgacttaaaacccaacggttctagtcaattaaagaagatatttggaaggaaggttttcgataaccctaaatcaattgatttggtaaaaagactaatacaatttgcgactgaaaacaaagaagcgattgtacttgactcatttgcagggagtggcactactgctcatgcagtattatcgcttaacaaacaagatggagggaatcgtcgtttcatccttattgagatggaagaatatgcacatgagattaccgcagaacgcggatctttatcgatttgcatgcaagctaattcggtggaaacgaggtcatcatttccttccgaaaaaacggttgcatttaaatcttacatatgtaatactttcaaagactacatttgtaagatttgatgtttgagtcggctgaaagatcgtacgtaccaattattgtttcgtgattgttcaagccataacactgtagggatagtggaaagagtgcttcatctggttacgatcaatcaaatattcaaacggagggagacgattttgatgaaaccagtaacgttatacgatgtcgcagagtatgccggtgtctcttatcagaccgtttcccgcgtggtgaaccaggccagccacgtttctgcgaaaacgcgggaaaaagtggaagcggcgatggcggagctgaattacattcccaaccgcgtggcacaacaactggcgggcaaacagtcgttgctgattggcgttgccacctccagtctggccctgcacgcgccgtcgcaaattgtcgcggcgattaaatctcgcgccgatcaactgggtgccagcgtggtggtgtcgatggtagaacgaagcggcgtcgaagcctgtaaaacggcggtgcacaatcttctcgcgcaacgcgtcagtgggctgatcattaactatccgctggatgaccaggatgccattgctgtggaagctgcctgcactaatgttccggcgttatttcttgatgtctctgaccagacacccatcaacagtattattttctcccatgaagacggtacgcgactgggcgtggagcatctggtcgcattgggtcaccagcaaatcgcgctgttagcgggcccattaagttctgtctcggcgcgtctgcgtctggctggctggcataaatatctcactcgcaatcaaattcagccgatagcggaacgggaaggcgactggagtgccatgtccggttttcaacaaaccatgcaaatgctgaatgagggcatcgttcccactgcgatgctggttgccaacgatcagatggcgctgggcgcaatgcgcgccattaccgagtccgggctgcgcgttggtgcggatatctcggtagtgggatacgacgataccgaagacagctcatgttatatcccgccgttaaccaccatcaaacaggattttcgcctgctggggcaaaccagcgtggaccgcttgctgcaactctctcagggccaggcggtgaagggcaatcagctgttgcccgtctcactggtgaaaagaaaaaccaccctggcgcccaatacgcaaaccgcctctccccgcgcgttggccgattcattaatgcagctggcacgacaggtttcccgactggaaagcgggcagtgagcgcaacgcaattaatgtgagttaggatcctgcctcgcgcgtttcggtgatgacggtgaaaacctctgacacatgcagctcccggagacggtcacagcttgtctgtaagcggatgccgggagcagacaagcccgtcagggcgcgtcagcgggtgttggcgggtgtcggggcgcagccatgacccagtcacgtagcgatagcggagtgtatactggcttaactatgcggcatcagagcagattgtactgagagtgcaccatatgcggtgtgaaataccgcacagatgcgtaaggagaaaataccgcatcaggcgctcttccgcttcctcgctcactgactcgctgcgctcggtcgttcggctgcggcgagcggtatcagctcactcaaaggcggtaatacggttatccacagaatcaggggataacgcaggaaagaacatgtgagcaaaaggccagcaaaaggccaggaaccgtaaaaaggccgcgttgctggcgtttttccataggctccgcccccctgacgagcatcacaaaaatcgacgctcaagtcagaggtggcgaaacccgacaggactataaagataccaggcgtttccccctggaagctccctcgtgcgctctcctgttccgaccctgccgcttaccggatacctgtccgcctttctcccttcgggaagcgtggcgctttctcatagctcacgctgtaggtatctcagttcggtgtaggtcgttcgctccaagctgggctgtgtgcacgaaccccccgttcagcccgaccgctgcgccttatccggtaactatcgtcttgagtccaacccggtaagacacgacttatcgccactggcagcagccactggtaacaggattagcagagcgaggtatgtaggcggtgctacagagttcttgaagtggtggcctaactacggctacactagaaggacagtatttggtatctgcgctctgctgaagccagttaccttcggaaaaagagttggtagctcttgatccggcaaacaaaccaccgctggtagcggtggtttttttgtttgcaagcagcagattacgcgcagaaaaaaaggatctcaagaagatcctttgatcttttctacggggtctgacgctcagtggaacgaaaactcacgttaagggattttggtcatgagattatcaaaaaggatcttcacctagatccttttaaattaaaaatgaagttttaaatcaatctaaagtatatatgagtaaacttggtctgacagttaccaatgcttaatcagtgaggcacctatctcagcgatctgtctatttcgttcatccatagttgcctgactccccgtcgtgtagataactacgatacgggagggcttaccatctggccccagtgctgcaatgataccgcgagacccacgctcaccggctccagatttatcagcaataaaccagccagccggaagggccgagcgcagaagtggtcctgcaactttatccgcctccatccagtctattaattgttgccgggaagctagagtaagtagttcgccagttaatagtttgcgcaacgttgttgccattgctgcaggcatcgtggtgtcacgctcgtcgtttggtatggcttcattcagctccggttcccaacgatcaaggcgagttacatgatcccccatgttgtgcaaaaaagcggttagctccttcggtcctccgatcgttgtcagaagtaagttggccgcagtgttatcactcatggttatggcagcactgcataattctcttactgtcatgccatccgtaagatgcttttctgtgactggtgagtactcaaccaagtcattctgagaatagtgtatgcggcgaccgagttgctcttgcccggcgtcaacacgggataataccgcgccacatagcagaactttaaaagtgctcatcattggaaaacgttcttcggggcgaaaactctcaaggatcttaccgctgttgagatccagttcgatgtaacccactcgtgcacccaactgatcttcagcatcttttactttcaccagcgtttctgggtgagcaaaaacaggaaggcaaaatgccgcaaaaaagggaataagggcgacacggaaatgttgaatactcatactcttcctttttcaatattattgaagcatttatcagggttattgtctcatgagcggatacatatttgaatgtatttagaaaaataaacaaataggggttccgcgcacatttccccgaaaagtgccacctgacgtctaagaaaccattattatcatgacattaacctataaaaataggcgtatcacgaggccctttcgtcttcaagaattctcatgtttgacagcttatcatcgataagctcac

SEQ ID NO: 31 - DNA, 51 bp, synthetic construct
  misc_feature 1..51: note = primer srf00-F
  source 1..51: mol_type = other DNA
tagggccgatgtggcccaaaaatgtcatgaaagaatcgttgtaagacgctc

SEQ ID NO: 32 - DNA, 35 bp, synthetic construct
  misc_feature 1..35: note = primer srf00-R
  source 1..35: mol_type = other DNA
cttacgggcccccacggccttaccgccggccctcg

SEQ ID NO: 33 - DNA, 43 bp, synthetic construct
  misc_feature 1..43: note = primer srf04-F
  source 1..43: mol_type = other DNA
cggtaaggccgtgggggcccgtaaggacatgacgataccagag

SEQ ID NO: 34 - DNA, 43 bp, synthetic construct
  misc_feature 1..43: note = primer srf04-R
  source 1..43: mol_type = other DNA
tttcggggccgcactggcccccgggttaaactgctgaatttgc

SEQ ID NO: 35 - DNA, 52 bp, synthetic construct
  misc_feature 1..52: note = primer srf05-F
  source 1..52: mol_type = other DNA
cccgggggccagtgcggccccgaaagataaaacaattgttcagctgtttgag

SEQ ID NO: 36 - DNA, 42 bp, synthetic construct
  misc_feature 1..42: note = primer srf05-R
  source 1..42: mol_type = other DNA
tgtcggggccgctagggccttgcccttccaagcctcaagaag

SEQ ID NO: 37 - DNA, 44 bp, synthetic construct
  misc_feature 1..44: note = primer srf06-F
  source 1..44: mol_type = other DNA
gggcaaggccctagcggccccgacagacaaaacggttcatcagc

SEQ ID NO: 38 - DNA, 45 bp, synthetic construct
  misc_feature 1..45: note = primer srf06-R
  source 1..45: mol_type = other DNA
ttcaggggcctctgcggccgtgctgttaaacacctcgacaatttg

SEQ ID NO: 39 - DNA, 43 bp, synthetic construct
  misc_feature 1..43: note = primer srf09-F
  source 1..43: mol_type = other DNA
gggcaaggccccgacggccccgacagacaaaacggttcatcag

SEQ ID NO: 40 - DNA, 33 bp, synthetic construct
  misc_feature 1..33: note = primer srf09-R
  source 1..33: mol_type = other DNA
tgtttcggccgccggggccggcgggtttaagcc

SEQ ID NO: 41 - DNA, 43 bp, synthetic construct
  misc_feature 1..43: note = primer srf10-F
  source 1..43: mol_type = other DNA
cccgccggccccggcggccgaaacaaagcctctgacgtattgg

SEQ ID NO: 42 - DNA, 54 bp, synthetic construct
  misc_feature 1..54: note = primer srf10-R
  source 1..54: mol_type = other DNA
tagggccaagaaggccttatgaaaccgttacggtttgtgtattaagaaattcga

SEQ ID NO: 43 - DNA, 38504 bp, synthetic construct
  misc_feature 1..38504: note = linked construct srfAA-AC
  source 1..38504: mol_type = other DNA
atgtggcccaaaaatgtcatgaaagaatcgttgtaagacgctcttcgcaagggtgtctttttttgcctttttttcggtttttgcgcggtacacatagtcatgtaaagattgtaaattgcattcagcaataaaaaaagattgaacgcagcagtttggtttaaaaatttttatttttctgtaaataatgtttagtggaaatgattgcggcatcccgcaaaaaatattgctgtaaataaactggaatctttcggcatcccgcatgaaacttttcacccatttttcggtgataaaaacatttttttcatttaaactgaacggtagaaagataaaaaatattgaaaacaatgaataaatagccaaaattggtttcttattagggtggggtcttgcggtctttatccgcttatgttaaacgccgcaatgctgactgacggcagcctgctttaatagcggccatctgttttttgattggaagcactgctttttaagtgtagtactttgggctatttcggctgttagttcataagaattaaaagctgatatggataagaaagagaaaatgcgttgcacatgttcactgcttataaagattaggggaggtatgacaatatggaaataactttttaccctttaacggatgcacaaaaacgaatttggtacacagaaaaattttatcctcacacgagcatttcaaatcttgcggggattggtaagctggtttcagctgatgcgattgattatgtgcttgttgagcaggcgattcaagagtttattcgcagaaatgacgccatgcgccttcggttgcggctagatgaaaacggggagcctgttcaatatattagcgagtatcggcctgttgatataaaacatactgacactactgaagatccgaatgcgatagagtttatttcacaatggagccgggaggaaacgaagaaacctttgccgctatacgattgtgatttgttccgtttttccttgttcaccataaaggaaaatgaagtgtggttttacgcaaatgttcatcacgtgatttctgatggtatctccatgaatattctcgggaatgcgatcatgcacatttatttagaattagccagcggctcagagacaaaagaaggaatctcgcattcatttatcgatcatgttttatctgaacaggaatatgctcaatcgaagcggtttgaaaaggacaaggcgttttggaacaaacaatttgaatcggtgcctgaacttgtttccttgaaacggaatgcatccgcagggggaagtttagatgctgagaggttctctaaagatgtgcctgaagcgcttcatcagcagattctgtcgttttgtgaggcgaataaagtcagtgttctttcggtatttcaatcgctgctcgccgcctatttgtacagggtcagcggccagaatgatgttgtgacgggaacatttatgggcaaccggacaaatgcgaaagagaagcagatgcttggcatgtttgtttctacggttccgcttcggacaaacattgacggcgggcaggcgttttcagaatttgtcaaagaccggatgaaggatctgatgaagacacttcgccaccaaaagtatccgtataatctcctaatcaacgatttgcgtgaaacaaagagctctctgaccaagctgttcacggtttctcttgaatatcaagtgatgcagtggcagaaagaagaggatcttgcctttttgactgagccgattttcagcggcagcggattaaatgatgtctcaattcatgtaaaggatcgatgggatactgggaaactcaccatagattttgattaccgcactgatttattttcacgtgaagaaatcaacatgatttgtgagcgcatgattaccatgctggagaacgcgttaacgcatccagaacatacaattgatgaattaacactgatttctgatgcggagaaagagaagctgcttgcgagggccggcggtaaggccgtgggggcccgtaaggacatgacgataccagagctgttccaagaaaaggctgaactgctttctgatcatccagcggttgtatttgaagatcgcacattgtcctatcgaacgttacatgagcaatctgcacgcatcgccaatgtgctgaaacagaaaggggttggcccggacagtcctgtcgcggttttgattgaacgctctgaacggatgattacagctatcatgggaattttaaaagccggcggagcctatgtgccgattgatccgggttttcctgctgagcgcattcaatatattttggaggactgcggggcggatttcatcctgactgaatcgaaggttgcggcgcctgaagccgatgctgagctgattgacttagatcaggcgattgaggaaggtgcagaagaaagcctgaatgcagatgtgaacgctcggaaccttgcctacattatttacacatcgggaacaaccggacgcccgaaaggcgttatgatcgagcatcgccaggttcatcatttggttgaatctctgcagcagacgatttatcaaagcggcagccaaaccctgcggatggcattgcttgcgccgttccactttgatgcgtcagtgaagcagatcttcgcgtcgcttcttttgggccaaaccctttatatcgtaccgaagaaaacagtgacgaacggggccgcccttactgcatattatcggaagaacagcattgaggcgacggacggaacaccggctcatttgcaaatgctggcagcagcaggcgattttgaaggcctaaaactgaagcacatgctgatcggaggagaaggcctgtcatctgttgttgcggacaagctgctgaagctgtttaaagaagccggcacagcgccgcgtttgactaatgtgtacgggccgactgaaacgtgcgttgacgcgtctgttcatccggttatccctgagaatgcagttcaatcagcgtatgtgccgatcgggaaagcgctggggaataaccgcttatatattttggatcaaaaaggccggctgcagcctgaaggcgtggcgggtgagctttatatcgcgggagacggtgtgggccgaggctatttacatttgcctgaattaacggaagagaagtttttacaagatccattcgtgccgggcgatcgcatgtaccggaccggggacgtggtgcgctggcttccagatggaacaatcgaatatttaggcagagaggatgaccaggtcaaagtccgcggataccggattgagcttggggaaattgaagccgtgattcagcaggcgccagacgttgcaaaagccgttgttttggcacgccctgacgaacagggaaatcttgaggtttgcgcatatgttgtgcagaagcctggaagcgaatttgcgccagccggtttgagggagcatgcggccagacagcttcctgactatatggtgccggcttactttacagaagtgacagaaattccgcttacaccaagcggcaaagtcgaccgccgcaagctgtttgcactagaggtgaaggctgtcagcggcactgcctatacagcgccgcgaaatgagactgaaaaagcaatcgcagccatttggcaggacgtgctgaacgttgagaaggcggggatctttgacaatttctttgaaactggcggacattcattaaaagccatgacccttttaacaaagattcataaggaaacaggcattgagattccgcttcaatttttgtttgagcatccgacgattacggctcttgcagaggaagctgatcacagagaaagcaaagcttttgcggtgattgaacctgctgaaaaacaggagcattacccgctttcattggcacagcagcgaacatatatcgtcagccagttcgaggatgcgggagtcggctataacatgccagcagcagcaattctggaagggcctttagatattcaaaagctggagcgcgcatttcagggattaatccgacgccacgagtcattgagaacatcatttgttcttgaaaacagcacgccgagacagaaaattcacgatagcgttgatttcaacatcgaaatgattgaaagaggcggccgctcagatgaggcaattatggcttcattcgttcggacatttgatttggcgaaagctccgctgttcagaatcggtttgctggggcttgaagagaaccgtcatatgctgctgtttgacatgcaccatttgatttctgacggtgtatccattggcattatgctggaggagttagcacgcatttataaaggcgaacagcttcctgatcttcgtctccagtataaggactacgctgtatggcaaagcagacaggctgctgaagggtacaagaaggaccaggcttattggaaggaagtctttgcaggcgagctcccggtgcttcagcttctgtccgattacccaagaccacctgttcaaagctttgaaggggatcgggtgtcaatcaagctggatgcgggggtaaaggatcgcctcaatcgtttggctgaacaaaacggcgccactttatatatggtgatgctttccgcttactatacgcttttgtcaaagtatacggggcaggatgacatcattgtcgggacaccgtcagcgggcagaaatcactccgatacagagggcattatcgggatgttcgtcaatacgcttgcgattcgcagtgaggtgaagcagaatgagacgtttacccaattgatctcgcgtgtccgcaaacgggtgctggatgccttttctcatcaggactatccgtttgagtggcttgttgaagatttgaacatcccgcgtgatgttagcaggcatccgctgtttgacacgatgttcagccttcaaaacgcgacagagggcattccggctgtcggcgatctttccttgtctgttcaagagaccaatttcaagattgccaaatttgatttgacggtgcaggcgagagaaaccgatgaaggcattgagattgatgtggattacagcacaaagctgtttaaacaaagcacggcagacaggctgcttacgcattttgcgcgtttgcttgaagatgctgcggctgatccagagaagccgatttctgagtataagcttctttctgaagaggaggctgcttcgcaaattcagcagtttaacccgggggccagtgcggccccgaaagataaaacaattgttcagctgtttgaggagcaagcggcgaatacgccagaccacactgcgcttcaatatgaaggcgaatcactcacttatcgtgaactgaatgaacgggccaatcgtttagcccgcggcattctttctcttggagctggcgaaggcagaactgcggctgtcttatgcgagcggtcaatggatatgattgtgtcgatcttggcagtattaaaatcaggttcggcttatgttccgatcgatccggaacatccgattcagcggatgcagcatttcttccgtgacagcggagcaaaggtgcttctcactcagaggaaattaaaggctttggcggaagaagcggaatttaagggcgttatcgtgctagccgatgaggaagaaagctatcatgccgatgcgcgaaatctcgcactgcctcttgattctgcagcaatggccaacctgacgtatacttccggaacgactggaacacctaaggggaatatcgtgacacatgccaatattctccgcacggtgaaggaaacgaattatctcagcattacagaacaggatacgattctcggtctttccaattacgtgtttgacgcgtttatgttcgatatgttcggctctttgttaaacggagccaagctggtgctgataccgaaggaaaccgttttggacatggctcgcctgtcccgcgtcattgaacgggagaacatcagcattctcatgattacaaccgctttgttccacttgcttgtggacttgaatccggcatgcttgtcaacgcttcgcaagattatgtttggcggggaacgggcttcggttgagcatgtcagaaaagctttgcaaacggttggaaagggcaagctccttcatatgtatggaccgtctgaaagcacggttttcgcgacgtatcatccggttgatgaattggaggagcacacgctgtctgttccgattggaaaaccggtcagcaatacggaagtatacattcttgaccgtacgggacacgtgcagcctgccgggattgccggagagctttgcgtcagcggcgaaggactcgtgaaaggctattacaaccgtccagaactgactgaggagaaatttgttccccatccgtttacatccggcgaacgcatgtataaaacgggagaccttgcgagatggctgccgaatggcgacatcgaatttatcgggcgaatcgaccatcaggtgaagattcgcggacagcgcatcgagcttggagaaatcgaacatcagctgcaaacccatgatcgtgttcaggaaagtgttgtgcttgccgttgatcaaggagcgggagataaactgttgtgtgcttactatgtcggagaaggagacatctcatcacaagagatgagagagcatgctgcgaaggacttgccggcatatatggttcctgcggtgtttatccaaatggacgagctgccgctgacagggaacggaaaaattgaccggagagcgctgccgattcctgatgccaacgtttcaagaggtgtttcatatgttgcgccacgcaatggaacggaacaaaaagtcgcggacatttgggcacaggtacttcaggcagaacaagtcggcgcttatgaccacttctttgacattggcggacattcattagcaggcatgaagatgcttgccttggttcatcaggaactgggcgttgagctgtcactcaaggatctcttccagtcaccgacggttgagggcttggcacaggtgattgcctctgctgaaaaagggacagccgcaagtatcagcccggcagagaaacaagatacgtatcctgtttcttcaccgcaaaaacggatgtacgtgcttcagcagcttgaggatgcgcaaacgagctataacatgccggcggttctgcgcctgacaggtgagcttgatgttgaaaggcttaacagcgtcatgcagcagttaatgcagcgtcatgaagccttgagaaccacgtttgaaataaaagatggagaaacggtgcagcggatctgggaagaggctgagtgcgagatagcctatttcgaagccccggaagaagagacagagcggatcgtttctgagtttattaagcctttcaaaatcgaccaacttccactgttcagaatagggcttatcaagcattcagacactgagcatgtgctgctgttcgatatgcatcatattatttctgatggtgcatctgtcggtgtgctgattgaggagctttcaaagctgtacgacggagaaacccttgagccgctccgtattcaatataaggattatgccgtgtggcagcagcagttcattcagtctgagctttacaagaagcaagaagagcattggctgaaggagctggacggagagctgccggtgctgacgcttccgactgattacagtcggcctgccgttcaaacatttgagggagaccgcattgcattttcattagaagcaggcaaagctgatgctctgcgcaggcttgcaaaagaaacggattccacgctttacatggtgcttctggcttcatacagtgcgtttttatcaaaaattagcgggcaagacgatatcatcgtcggttcacctgtggccggacgatctcaagcggacgtcagccgcgtcatcggaatgttcgtcaatacattggcgctgcgcacgtatccgaagggtgaaaagacgtttgctgactatcttaacgaagtgaaagaaacggcactcagcgcttttgatgcgcaggattacccacttgaggatttgatcggaaatgttcaggttcagcgtgacacaagcagaaatccgttattcgatgcagttttttcaatgcaaaatgcgaatataaaggatttaacaatgaaagggattcagcttgagccgcatccgtttgaacggaaaacagccaagtttgacctcacgctgacggctgacgaaaccgacggagggcttacattcgtactcgaatacaatacagctctgtttaagcaggaaacgattgaacgatggaagcaatattggatggagcttttagatgcagttactgggaacccgaaccagccgctttccagcctgtcactggtcaccgagacagaaaagcaagcgcttcttgaggcatggaagggcaaggccctagcggccccgacagacaaaacggttcatcagctattcgaagagactgcccagcgccacaaagaccgcccggctgtcacatacaacggccagtcttggacgtacggcgagctgaatgcgaaggcaaaccgtctcgcgcggattctgatggactgcggcatcagcccggatgaccgcgtcggcgttctcacgaagccgtcgcttgaaatgtccgccgcggtgctcggcgtcttgaaagccggagcggcgtttgtgccgattgatcctgactatccggatcagcggattgagtatattttacaggacagcggcgcgaagcttctcttgaaacaggaaggcatttcagtgccggacagctatacgggagatgtcattcttctcgacggaagccgcacgattctaagcctgccgcttgatgaaaacgacgaggaaaatccagaaaccgctgtaaccgcggagaacttggcgtacatgatttacacgtctggaacgaccggacagccgaagggtgtcatggtcgagcaccatgcgcttgtgaacctgtgcttctggcaccacgacgcgttcagcatgacagcggaggaccgcagtgcgaagtacgcgggctttgggttcgacgcttccatttgggagatgttcccgacctggacgatcggtgccgaacttcacgtcattgaggaagcgatccgcctcgatatcgtccgcctgaacgattattttgaaacgaacggcgtaacgatcacgttcctgccgacacagcttgcggaacagttcatggagcttgagaacacatcacttcgcgtattgcttactggaggagacaagctgaagcgcgcagtgaaaaagccgtacacactcgtcaataactacgggccgacagagaatacggtcgttgccacaagcgcagaaatccatccggaggaaggctcgctttccatcggaagggccattgccaatacgagagtatacattctcggcgagggcaatcaggtgcagccggaaggcgtagccggagagctttgcgtggcggggcgcggactggcacgcggctatctgaatcgagaagacgaaaccgcgaagcggtttgtcgctgatccgtttgtgccgggtgagcgcatgtaccgcaccggcgatttggtgaaatggacgggcggcggcatcgaatacatcggccggatcgaccagcaggtcaaggtccgcggctaccggatcgagctctcagaaattgaagtccagctcgcccagctttctgaggtgcaggatgcggcggtgacagctgtcaaagataaaggcggcaacacagcgatcgcggcgtatgtcacaccggaatcagctgacatagaagcactgaaatcagcactgaaggaaaccctgccggattacatgatcccggcgttctgggtgacgctgaacgagcttccggttacggcaaacggcaaagtggaccgcaaagccttgcctgagccggacatcgaagcgggaagcggagaatacaaagcgccgacgaccgacatggaagagctgcttgccggcatctggcaggacgtgcttggaatgtctgaagtcggtgtcaccgacaatttcttctcgcttggcggagattccatcaaaggaattcaaatggcgagccgcttgaaccagcacggctggaagctggaaatgaaagatctcttccagcacccgacgatcgaagagctcacccagtacgtagagcgtgccgaaggcaaacaggcagaccaaggcccggtggagggcgaagtcatcctgacgccgatccagcgctggttctttgaaaagaacttcacgaacaagcaccactggaaccaatctgtgatgcttcacgccaagaagggctttgatcctgaacgggtggagaaaacattgcaggcgctgatcgagcatcatgacgcgctccgcatggtctatcgtgagggacaggaagacgtcattcaatacaacagaggtcttgaagctgcttcagctcaattggaggtcatccagattgagggccaagctgcagattacgaagaccgaatagagagagaagcggagcgtttgcaaagcagcatcgacttgcaggaaggcggcttgttaaaagcaggcttgttccaagcggaagacggagatcacttgcttcttgccattcaccacttagtggttgacggcgtgtcgtggcggattttactggaggatttcgccgcggtatatacacagcttgagcaaggcaatgaaccggttctcccgcagaaaacacattcatttgcagagtatgcagagagattgcaagacttcgcgaactccaaagcctttttgaaagaaaaagagtattggagacagcttgaagaacaagctgttgcggcaaagcttccgaaagaccgcgaatctggtgatcagcgaatgaaacatacaaagacaattgaattctcgctgactgctgaagagacagaacagctcaccacaaaggtgcatgaggcatatcacacagaaatgaatgatattttgctgacggcattcggattggcaatgaaggagtggacgggtcaagatcgagtaagtgttcatttagaggggcatggacgtgaagaaatcatagaagacctgaccatttctcgcacagtcggctggtttacaagtatgtacccaatggtgctcgatatgaagcatgcggatgatctgggctaccagctgaagcaaatgaaagaagatatcagacatgtgccgaataagggagtcggatacggcattctgcgctatctgacggcaccggaacataaagaagatgtggcgttctcgattcagccggatgtcagcttcaactatttaggtcagtttgacgaaatgtcggatgcaggtttgtttacgagatcagagctgccatcaggacagtcattaagccctgaaacagaaaaaccgaatgcgctggatgttgtcggatatatcgaaaacggaaaactgacgatgtcactggcctatcattctcttgaatttcatgaaaaaacagtacaaacattcagtgacagctttaaagcgcatcttctcagaatcattgaacattgcctatctcaagatggtacggaactgaccccgagtgatcttggtgacgacgatttgacgctggatgagctggataaattaatggaaattttctaatagaggtggcatatgagcaaaaaatcgattcaaaaggtgtacgcactgacaccaatgcaggagggaatgctgtatcatgcgatgcttgatccgcattcttcctcgtacttcacacaattagagcttgggattcacggcgcttttgatcttgaaatctttgagaaaagcgtcaatgaactgattcggtcatacgatattctccgtacggtatttgtgcatcagcagctgcaaaaaccgcgtcaggtcgtgttagcggaacgcaaaacaaaagtgcattatgaggatatcagtcatgcagacgaaaaccgccagaaagagcacattgagcgttacaaacaagacgttcagcgccaaggctttaacctggcaaaagacatattgttcaaggtagcggttttccgccttgctgcagatcagctgtatcttgtctggagcaatcatcatattatgatggacggctggagcatgggcgtcctcatgaaaagcctgttccaaaactatgaagcgctcagagcaggcaggacaccggcaaacggtcagggcaagccttattccgattacatcaagtggcttggaaaacaggacaatgaagaagcggagagctactggagcgagcgcttggcgggttttgaacagccaagcgtgctcccgggccgcctgcctgtgaaaaaagacgaatacgtcaataaagaatattcatttacatgggacgaaacactggttgcccgtattcagcaaaccgcaaatctccatcaagtgacagggcctaacctatttcaggccgtttggggcattgttctcagcaaatacaactttacggatgatgtgatcttcggaacggtcgtctcgggacgaccgtctgaaatcaacggaatcgaaacgatggcggggctgtttatcaacaccattccagtgcgggtgaaagttgaacgagatgctgcattcgctgatattttcacagctgttcagcagcatgcagtagaggcagagcgttacgattacgtgccgctctatgagattcaaaaacgctcagctcttgatggcaatctcttaaaccatctggtcgcgtttgaaaattatccgcttgatcaagagcttgaaaacggcagcatggaagaccgcctcgggttttcgattaaggtagaaagcgcatttgaacaaacgagcttcgatttcaacctgattgtgtatccgggcaaaacgtggaccgtcaaaattaaatataacggagccgcctttgattccgcttttatcgaacggacagcggagcaccttacccgcatgatggaagcagctgtcgatcagccggccgcttttgtgcgtgagtacgggcttgtgggagacgaagagcagcggcaaattgtcgaggtgtttaacagcacggccgcagaggcccctgaaggaatggctgttcaccaagtgtttgaagagcaagcgaaacggacgccggcgagcaccgccgtcgtatatgaaggaaccaagctgacgtaccgcgagctgaatgcagcggctaaccgtctggcgagaaagcttgtcgaacatgggcttcaaaaaggggaaacagcagcgattatgaacgaccgctcagtagaaaccgttgtcggcatgctggctgttttaaaagcaggcgccgcatatgtgccgcttgatccagcgcttcctggggatcgtcttcgtttcatggcagaggacagctccgttcgaatggttttgatcggaaattcttatacagggcaggcacatcagctgcaagtgccggttcttacactggacataggctttgaagagagtgaagcggctgacaatctcaacctgccatccgccccgtctgatttggcgtacatcatgtacacatccggttcaacgggcaaaccgaaaggcgtcatgatcgaacataaaagcattctgcgcctcgtcaaaaatgccgggtacgttcctgttactgaagaagaccgcatggcgcaaacgggagctgtcagctttgatgccggaacgtttgaggtattcggcgcactgctgaatggcgcagcactttatccggtcaaaaaagagacactgcttgatgcgaaacaatttgctgcattcctgcgtgagcaaagcatcacaactatgtggctgacatcacctttattcaaccagcttgctgcaaaggatgcgggtatgttcggcacactgcgccatttaatcatcggcggagatgcccttgtcccgcatattgtcagcaaagtaaaacaggcatcgccgtcgctttcattgtggaacggatacggcccgacagaaaacacgacgttttcaaccagttttctgatcgaccgcgagtatggcggctctatcccaatcgggaagccgatcggaaattccactgcctatattatggatgagcagcaatgcctgcagccaatcggcgcgcctggtgagctttgcgtaggcggaatcggtgtagcgcgtgggtatgtcaatctccctgagctgacggagaagcaatttctggaagacccgttcagaccgggtgagagaatttaccgcactggtgacttggcaagatggctgccggacggcaatatcgaatttttaggcagaatcgacaaccaagtgaaggtgcgcggcttccgaattgagcttggcgaaattgaaacaaaactgaacatggctgagcatgtgacagaagccgcggtgatcatacgcaagaacaaagcagacgaaaatgaaatttgcgcgtacttcacggcggatcgtgaagtggctgtgagtgagctgagaaaaacactgtctcagtctttgcctgactatatggtccctgcccacctgattcaaatggacagcctgccgctcacgccaaacgggaaaatcaacaaaaaggaactgcctgcaccgcaatcagaagccgtgcagccggaatacgcagcaccaaaaacagagagtgaaaagaaattagcggagatctgggaaggaatactcggcgtcaaagcaggcgttaccgataacttctttatgatcggcggccattctttgaaagcgatgatgatgacggcgaaaattcaagagcattttcataaggaagttccgataaaagtgctttttgaaaagccgactattcaagaactggcactgtatttggaagagaacgaaagcaaggaggagcagacgtttgaaccgatcaggcaagcatcttatcagcagcattatcctgtatccccggcccagcggagaatgtatatcctcaatcagcttggacaagcaaacacaagctacaacgtccccgctgtacttctgctggagggagaagtagataaagaccggcttgaaaacgcgattcagcaattaatcaaccggcacgaaatcctccgtacatcgtttgacatgatcgacggagaggttgtgcaaaccgttcataaaaacatatcgttccagctggaggctgccaagggacgggaagaagacgcggaagagataatcaaagcatttgttcagccgtttgaattaaaccgcgcgccgctcgtccgttcgaagcttgtccagctggaagaaaaacgccacctgctgctcattgatatgcatcatattattactgacggaagttcaacaggcattctaatcggtgatcttgccaaaatatatcaaggcgcagatctggaactgccacaaattcactataaagattacgcagtttggcacaaagaacaaactaattatcaaaaagatgaggaatactggctcgatgtctttaaaggcgaactgccaatactggatcttcccgcggatttcgagcggccagctgaacggagctttgcgggagagcgcgtgatgtttgggcttgataagcaaatcacggctcaaatcaaatcgctcatggcagaaacagatacgacaatgtacatgtttttgctggcggcgttcaatgtactcctttccaagtacgcgtcacaggatgatatcattgtcggctcgccgacagctggcagaacacatcctgatctgcaaggtgtgccgggtatgtttgtcaacacggtggcactcagaacggcaccagcgggagataaaaccttcgcgcaattccttgaagaggtcaaaacagccagccttcaagcattcgagcaccagagctatccgcttgaggagctgattgaaaagcttccgcttacaagggatacaagcagaagtccgctgttcagcgtgatgttcaacatgcagaatatggagattccttcattaagattaggagatttgaagatttcctcgtattccatgcttcatcatgttgcgaaatttgatctttccttggaagcggtcgagcgtgaagaggatatcggcctaagctttgactatgcgactgccttgtttaaggacgagacgatccgccgctggagccgccactttgtcaatatcatcaaagcggccgcggctaatccgaacgttcggctgtctgatgtagatctgctttcatctgcagaaacggctgctttgctagaagaaagacatatgacggccatgacggccgcaacctttgcagcactttttgaaaaacaggcccagcaaacacctgaccattctgcggtgaaggctggcggaaatctgttgacctatcgcgagcttgatgaacaggcgaaccagctggcgcatcatcttcgtgcccaaggggcaggaaatgaagacatcgtcgcgattgttatggaccggtcagctgaagtcatggtatccattctcggtgtcatgaaggcgggggcagctttccttccgattgatcctgatacacctgaagaacgaatccgttattcattagaggacagcggagcaaaatttgcggtcgtgaatgaaagaaacatgacggctattgggcaatatgaagggataattgtcagccttgatgacggtaaatggagaaatgaaagcaaggagcgcccatcatccatttccgggtctcgcaatcttgcatacgtcatttatacgtccggtacgaccggaaagccaaagggcgtgcagattgagcatcgtaatctgacaaactatgtctcttggtttagtgaagaggcgggcctgacggaaaatgataagactgtattgctttcatcttacgcatttgaccttggctatacgagcatgttccctgtacttctgggcgggggcgagctccatatcgtccagaaggaaacctatacggcgccggatgaaatagcgcactatatcaaggagcatgggatcacttatatcaagctgacaccgtctctgttccatacaatagtgaacaccgccagttttgcaaaagatgcgaactttgaatccttgcgcttgatcgtcttgggaggagaaaaaatcatcccgactgatgttatcgccttccgtaagatgtatggacataccgaatttatcaatcactacggcccgacagaagcaacgatcggcgccatcgccgggcgggttgatctgtatgagccggatgcatttgcgaaacgcccgacaatcggacgcccgattgcgaatgccggtgcgcttgtcttaaatgaagcattgaagcttgtgccgcctggagcgagcggacagctctatatcacgggacaggggctcgcgagagggtatctcaacaggcctcagctgacagccgagagatttgtagaaaatccatattcgccgggaagcctcatgtacaaaaccggagatgtcgtacgaagactttctgacggtacgcttgcatttatcggccgggctgatgatcaggtgaaaatccgaggctaccgcattgagccgaaagaaattgaaacggtcatgctcagcctcagcggaattcaagaagcggttgtactagcggtttccgagggcggtcttcaagagctttgcgcgtattatacgtcggatcaagatattgaaaaagcagagctccggtaccagctttccctaacactgccgtctcatatgattcctgctttctttgtgcaggttgacgcgattccgctgacggcaaacggaaaaaccgacagaaacgctctgccgaagcctaacgcggcacaatccggaggcaaggccttggccgcaccggagacagcgcttgaagaaagtttatgccgcatttggcagaaaacgcttggcatagaagccatcggcattgatgacaattttttcgatttaggcggccattcattaaaagggatgatgctgattgccaacattcaggcggaattggagaaaagcgtaccgcttaaagcactgttcgagcagccgacagttcgccagctggcggcttatatggaggcgtctgctgtttcaggcggccatcaagtactcaaaccggctgacaagcaggatatgtatccattgtcatccgcacagaaacgaatgtacgtgctcaatcagcttgaccgccagacgataagctacaacatgccatctgttcttctaatggaaggagagcttgatatttcgcgcctgcgcgactcactcaatcagcttgtgaaccgtcacgaatcattgcggacgtcatttatggaagctaatggtgagcctgttcagcgcatcattgagaaggcggaggttgatcttcatgtgtttgaagccaaagaagacgaagcggaccaaaagattaaggaatttatccggccattcgacttaaacgacgcaccgctcattcgcgcagctttgcttcgaatagaagcgaaaaaacatttgctgcttttagatatgcatcatatcatcgcagacggcgtctcaagaggcatctttgtaaaagaattggcgctgctttacaaaggagagcagcttccggagccgacgcttcattataaagatttcgccgtttggcaaaatgaagctgagcaaaaagaacggatgaaggagcatgaggcgtactggatgtcagttctttcaggcgagctgccagagcttgatctcccgctcgattatgcccgtccgcctgtgcaaagctttaaaggagatacgatccgtttccgtacgggaagtgagacggcaaaggcggtagaaaaactgcttgccgaaaccggaacgaccttgcacatggtgctccatgctgttttccacgtctttttaagcaaaatttccggacagcgggatatcgtcatcggctccgttactgccggccggacgaatgctgatgttcaggacatgccgggaatgttcgtcaatacacttgccctgagaatggaagcgaaagaacagcaaacatttgcggagcttttggagctagcaaagcagacgaacctgtcagcccttgagcatcaggagtatccgtttgaagatctggttaatcagcttgatctccctcgggatatgagccgaaacccattgtttaatgtgatggtgacgacagaaaaccctgataaagaacagcttacattgcaaaatctgagcatttcaccttatgaggctcatcagggaacttctaagtttgatctgacactgggcggatttactgatgaaaatggcattggcttgcagctcgaatatgcgacagatctgttcgcaaaagaaacagctgaaaaatggagcgaatacgttctgcggctactaaaggctgttgcggataacccgaaccagccgctttccagtctgttactggtcaccgagacagaaaagcaagcgcttcttgaggcatggaagggcaaggccccgacggccccgacagacaaaacggttcatcagctattcgaagagactgtccagcgccacaaagaccgcccggctgtcacatacaacggccaatcttggacgtacggcgagctgaacgcgaaggcaaaccgcctcgcccggattctgatggactgcggcatcagcccggatgaccgcgtcggcgttctcacgaagccgtcgcttgaaatgtccgccgcggtgctcggcgtcttgaaagccggagcggcgtttgtgccgattgatcctgactacccggatcagcggattgagtatattttacaggacagcggcgcgaagcttctcttgaaacaggaaggcatttcagtgccggacagctatacgggagatgtcattcttctcgacggaagccgcacgattctaagcctgccgcttgatgaaaacgacgagggaaatccagaaaccgctgtaaccgcggagaacttggcgtacatgatttacacgtctggaacgaccggacagccgaagggtgtcatggtcgagcaccatgcgcttgtgaacctgtgcttctggcaccacgacgcgttcagcatgacagcggaggaccgcagtgcgaagtacgcgggcttcgggttcgacgcttccatttgggagatgttcccgacctggacgatcggcgctgaacttcacgtcattgatgaagcgatccgcctcgatatcgtccgcctgaacgattattttgaaacgaacggcgtaacgatcacgttcctgccgacacagcttgcggaacagttcatggagcttgagaacacatcacttcgcgtcctcttgaccggaggagacaagctgaagcgggcagtgaaaaagccgtacacactcgtcaacaactacgggccgacagaaaatacggtcgttgccacaagcgcagaaatccatccggaggaaggctcgctttccatcggacgggccattgccaatacgagagtatacattctcggcgagggcaatcaggtgcagccggaaggcgtagccggagagctttgcgtggcggggcgcggactggcacgaggctatctgaatcgagaagacgaaaccgcgaagcggtttgtcgctgatccgtttgtgccgggtgaacgcatgtaccgcaccggcgacttggtgaagtgggtgaacggcggcatcgaatacatcggccggatcgaccagcaggtcaaggtccgcggctaccggatcgagctctcagaaattgaagtccagctcgcccagctttctgaggtgcaggatgcggcggtgacagctgtcaaagataaaggcggcaatacagcgatcgcggcgtatgtcacaccggaaacagctgacatagaagcactaaaatcaacactaaaggaaaccctgccggattacatgatcccggcgttctgggtgacgctgaacgagcttccggttacggcaaacggcaaagtcgaccgcaaagccttgcctgagccggacatcgaagcgggaagcggagaatacaaagcgccgacgaccgacatggaagagctgcttgccggcatctggcaggacgtgcttggaatgtctgaagtcggtgtcaccgacaatttcttctcgcttggcggagattccatcaaaggaattcaaatggcgagccgcttgaatcagcacggctggaagctggaaatgaaagatctcttccagcatccgacgatcgaagagctcacccagtacgtagagcgtgccgaaggcaaacaggcagaccaaggcccggtggagggcgaagtcatcctgacgccgatccagcgctggttctttgaaaagaacttcacgaacaagcaccactggaaccaatcggtgatgcttcacgccaaaaagggctttgatcctgaacgggtggagaaaacattgcaggcgctgatcgagcatcatgacgcgctccgcatggtctaccgcgaggaaaacggggacatcgttcaggtgtataaaccgatcggtgagagcaaggtcagcttcgaaatcgtggatctgtacggctccgatgaagagatgctgagaagccagattaagcttctcgcgaacaagctgcaaagcagtctcgatctgcgaaacgggccgcttttaaaggcggagcaatatcgcacagaagctggggatcacctgctcattgctgtacaccatctcgtggtcgacggtgtgtcatggcggattttgcttgaagactttgcttcaggctacatgcaggctgagaaagaagagagccttgtcttcccgcaaaaaacaaactccttcaaggattgggcggaagaactggcggcattcagccaatcagcgcatcttttacagcaggctgaatactggtcgcaaattgccgctgaacaggtttctcctttacctaaggattgtgaaacagagcagcggatcgtcaaggatacatcatctgtcctatgtgaattaacggcagaagacactaagcatcttttaacagatgttcatcagccatatggaactgaaatcaacgatattcttctcagcgcgctcggtttgacaatgaaagaatggacaaagggggccaaaattggcattaaccttgagggacacggccgggaggacattatcccgaatgtgaatatctccagaacggtcggctggtttacggcacaataccctgttgtgctcgacatatctgacgcagatgcctcagctgtgatcaaaacagtcaaagaaaacctgcgccgcattccggacaaaggtgttggctacggcattcttcgttatttcacagaaacagcggaaacaaagggcttcacaccggagatcagcttcaactatttgggccaattcgacagtgaagtcaaaaccgatttctttgaaccgtccgctttcgatatggggcgccaagtaagcggagaatcagaggcgctgtacgcattaagcttcagcggcatgatcagaaacggccggtttgtgctttcctgctcctacaatgagaaggagtttgaaagagctacagtcgaggagcaaatggaacggtttaaagaaaacctcctgatgctaatccgccattgcacggaaaaagaagacaaggaattcacaccaagcgacttcagcgccgaagaccttgaaatggacgagatgggagatatctttgacatgcttgaggagaatttaaaataaaacgcaagggaattacagaaggcgggagcgaaacatatgagtcaatttagcaaggatcaggttcaagatatgtattacctatcgccgatgcaggaagggatgctttttcatgccatcctgaatcccggccaaagcttttaccttgaacaaatcacgatgaaagtaaaaggcagcttgaatatcaaatgtcttgaagaaagcatgaatgtgatcatggaccggtacgatgtatttcgtaccgtgttcattcacgaaaaagtaaaaaggcctgtccaagtcgtattgaaaaaacggcagttccatatagaagaaatcgatctgacacacttaacgggcagcgagcaaacagccaaaatcaatgagtacaaagaacaggataagatcaggggttttgatttgacgcgggatattccgatgcgggcagccattttcaagaaagctgaagaaagctttgaatgggtgtggagctaccaccacattattttggacggatggtgcttcggcatcgtcgtacaggatctatttaaggtatacaatgctctgcgcgaacaaaagccgtacagcctgccgcccgtcaaaccgtataaagactacatcaagtggcttgaaaagcaggataaacaagcatcactgcgttactggcgcgaatatttagagggctttgaaggacaaacgacgtttgcggagcaaagaaagaaacaaaaggacggctatgagccgaaagagctgctcttttcactgtcggaggcggaaacaaaggcctttaccgagcttgcaaaatcgcagcataccactttgagtacggcgctgcaggcagtctggagcgtattgatcagccgctatcagcagtctggcgatttggccttcggtacagttgtttcagggcgtcccgcggaaatcaaaggcgttgaacatatggtcgggctgtttatcaacgttgtcccgagacgtgtgaagctgtctgagggtatcacatttaacggcttgctcaagcggctgcaggagcaatcgctgcagtccgagccgcatcaatatgtgccgctttatgacatccaaagccaggccgatcagccgaaactgattgaccacatcattgtttttgagaactatccgcttcaggatgcgaaaaatgaagaaagcagtgaaaacggctttgatatggtggatgttcatgtttttgagaagtcgaattatgatctcaacctgatggcttccccgggagatgagatgctgattaagcttgcctataatgagaatgtgtttgatgaggcgtttatcctgcgcttgaaatctcagcttcttacagcaattcagcagctcatccagaatcctgatcagcctgtcagcacgatcaacctcgttgacgacagggagagagaatttttgctaaccggcttaaacccgccggccccggcggccgaaacaaagcctctgacgtattggttcaaggaagcagtgaacgccaatccggatgcaccggcgcttacgtattccggccagaccctgtcttatcgcgaattagatgaggaagcgaaccgcattgcacgccggctgcaaaaacacggtgcgggcaaaggctctgttgtagcgctgtacacgaagcgctcacttgaactggtgatcggcattctcggtgtattaaaggcgggagcagcctatctgccggttgatccgaagctgccagaggaccgaatctcgtatatgctggctgacagtgcggcagcctgtcttctgacgcatcaggagatgaaagaacaagcggctgagctgccgtatacaggcacaacgctcttcattgatgatcaaacacggtttgaagaacaggcaagcgatcctgcaaccgcgattgatcctaatgatccggcatatatcatgtacacgtccggcacaaccggaaagccaaagggcaatatcaccactcatgccaatattcaaggattggtcaagcatgtagactacatggcattttctgatcaggatacgttcttgtctgtttcgaattacgcctttgatgcatttacctttgatttctatgcttctatgctgaatgcggcacggctcattatcgcagatgaacatacgctgcttgatacagaacggctcacagatctgatcctgcaagagaatgtcaatgtcatgtttgcgacaaccgcactatttaatcttctcacagatgcgggagaggattggatgaaggggcttcgctgtatattattcggcggagagcgcgcgtcagtgcctcatgtcagaaaagcgctgcggatcatggggccgggcaagctgattaactgctacgggccgactgagggaacagtgtttgcgacagctcacgtcgtgcatgatctgccggattccatctcctcattgccgatcggaaagccgatcagcaatgccagtgtttatattctgaatgagcaaagccagctccagccattcggggcggtcggtgaactgtgcatcagcggaatgggcgtgtcaaaagggtatgtaaatcgtgctgacctcacgaaggaaaagtttatcgagaacccgttcaagccgggagaaacgctttaccgtacaggggatttagcgcgctggctgccggatggaacgattgaatacgccggccgtattgacgaccaggtcaaaatacgcggacaccggattgagcttgaagaaatcgaaaagcagctgcaggaatacccaggtgtgaaagatgcggtcgttgtggcggaccgccatgagtctggcgatgcatcaatcaatgcctaccttgtgaaccgaacgcagctttcagctgaagacgtgaaggcgcacctgaaaaaacagcttcctgcttacatggtgccgcaaacctttaccttcttggatgagcttcctttaacgacgaacgggaaagtcaataaacggctgctcccaaaacctgatcaggatcagctggcggaagaatggattggaccgcggaacgagatggaagaaacaatcgcacaaatatggtctgaggttctcggcagaaagcaaattggcattcatgacgatttctttgcgctcggagggcattccttgaaggccatgaccgccgcgtcccgcatcaagaaagagctcgggattgatcttccagtgaagcttttgtttgaagcgccgacgatcgccggcatttcagcgtatttgaaaaacgggggctctgatggcttgcaggatgtaacgataatgaatcaggatcaggagcagatcattttcgcatttccgccggttctgggctatggccttatgtaccaaaatctgtccagccgcttgccgtcatacaagctatgcgcctttgattttattgaggaggaagaccggcttgaccgctatgcggatttgatccagaagctgcagccggaagggcctttaacattgtttggatattcagcgggatgcagcctggcgtttgaagctgcgaaaaagcttgaggaacaaggccgtattgttcagcggatcatcatggtggattcctataaaaaacaaggtgtcagtgatctggacggacgcacggttgaaagtgatgtcgaagcgttgatgaatgtcaatcgggacaatgaagcgctcaacagcgaagccgtcaaacacggcctcaagcaaaaaacacatgccttttactcatactacgtcaacctgatcagcacaggccaggtgaaagcagatattgatctgttgacttccggcgctgattttgacatgccggaatggcttgcatcatgggaagaagctacaacaggtgtttaccgtgtgaaaagaggcttcggaacacacgcagaaatgctgcagggcgaaacgctagataggaatgcggagattttgctcgaatttcttaatacacaaaccgtaacggtttcataaggccttctgtgagctttaatgcggtagtttatcacagttaaattgctaacgcagtcaggcaccgtgtatgaaatctaacaatgcgctcatcgtcatcctcggcaccgtcaccctggatgctgtaggcataggcttggttatgccggtactgccgggcctcttgcgggatatcgtccattccgacagcatcgccagtcactatggcgtgctgctagcgctatatgcgttgatgcaatttctatgcgcacccgttctcggagcactgtccgaccgctttggccgccgcccagtcctgctcgcttcgctacttggagccactatcgactacgcgatcatggcgaccacacccgtcctgtggatcctctacgccggacgcatcgtggccggcatcaccggcgccacaggtgcggttgctggcgcctatatcgccgacatcaccgatggggaagatcgggctcgccacttcgggctcatgagcgcttgtttcggcgtgggtatggtggcaggccccgtggccgggggactgttgggcgccatctccttgcatgcaccattccttgcggcggcggtgctcaacggcctcaacctactactgggctgcttcctaatgcaggagtcgcataagggagagcgtcgaccgatgcccttgagagccttcaacccagtcagctccttccggtgggcgcggggcatgactatcgtcgccgcacttatgactgtcttctttatcatgcaactcgtaggacaggtgccggcagcgctctgggtcattttcggcgaggaccgctttcgctggagcgcgacgatgatcggcctgtcgcttgcggtattcggaatcttgcacgccctcgctcaagccttcgtcactggtcccgccaccaaacgtttcggcgagaagcaggccattatcgccggcatggcggccgacgcgctgggctacgtcttgctggcgttcgcgacgcgaggctggatggccttccccattatgattcttctcgcttccggcggcatcgggatgcccgcgttgcaggccatgctgtccaggcaggtagatgacgaccatcagggacagcttcaaggatcgctcgcggctcttaccagcctaacttcgatcattggaccgctgatcgtcacggcgatttatgccgcctcggcgagcacatggaacgggttggcatggattgtaggcgccgccctataccttgtctgcctccccgcgttgcgtcgcggtgcatggagccgggccacctcgacctgaatggaagccggcggcacctcgctaacggattcaccactccaagaattggagccaatcaattcttgcggagaactgtgaatgcgcaaaccaacccttggcagaacatatccatcgcgtccgccatctccagcagccgcacgcggcgcatctcgggcagcgttgggtcctggccacgggtgcgcatgatcgtgctcctgtcgttgaggacccggctaggctggcggggttgccttactggttagcagaatgaatcaccgatacgcgagcgaacgtgaagcgactgctgctgcaaaacgtctgcgacctgagcaacaacatgaatggtcttcggtttccgtgtttcgtaaagtctggaaacgcggaagtcagcgccctgcaccattatgttccggatctgcatcgcaggatgctgctggctaccctgtggaacacctacatctgtattaacgaagcgctggcattgaccctgagtgatttttctctggtcccgccgcatccataccgccagttgtttaccctcacaacgttccagtaaccgggcatgttcatcatcagtaacccgtatcgtgagcatcctctctcgtttcatcggtatcattacccccatgaacagaaatcccccttacacggaggcatcagtgaccaaacaggaaaaaaccgcccttaacatggcccgctttatcagaagccagacattaacgcttctggagaaactcaacgagctggacgcggatgaacaggcagacatctgtgaatcgcttcacgaccacgctgatgagctttaccgcagaattcgcccttcccggtcgatatgaacagcttatttacataattcacgttattggtagttataaatgaaattcctaatatcggttatgaagtgaaattgaatttctacttgatctttctctctatttttgtaaaataaaattaagaatatttaaatattcaatgattcatttttgcagaaatcggaggaagaagaatatatgaaaacatttaacatttctcaacaagatccccccatattgttgtataagtgatgaaatactgaatttaaaacttagtttatatgtggtaaaatgttttaatcaagtttaggaggaattaattatgaagtgtaatgaataatgaatgtaacagggttcaattaaaagagggaagcgtatcattaaccctataaactacgtctgccctcattattggagggtgaaatgtgaatacatcctattcacaatcgaatttacgacacaaccaaattttaatttggctttgcattttatctttttttagcgtattaaatgaaatggttttgaacgtctcattacctgatattgcaaatgattttaataaaccacctgcgagtacaaactgggtgaacacagcctttatgttaaccttttccattggaacagctgtatatggaaagctatctgatcaattaggcatcaaaaggttactcctatttggaattataataaattgtttcgggtcggtaattgggtttgttggccattctttcttttccttacttattatggctcgttttattcaaggggctggtgcagctgcatttccagcactcgtaatggttgtagttgcgcgctatattccaaaggaaaataggggtaaagcatttggtcttattggatcgatagtagccatgggagaaggagtcggtccagcgattggtggaatgatagcccattatattcattggtcctatcttctactcattcctatgataacaattatcactgttccgtttcttatgaaattattaaagaaagaagtaaggataaaaggtcattttgatatcaaaggaattatactaatgtctgtaggcattgtattttttatgttgtttacaacatcatatagcatttcttttcttatcgttagcgtgctgtcattcctgatatttgtaaaacatatcaggaaagtaacagatccttttgttgatcccggattagggaaaaatataccttttatgattggagttctttgtgggggaattatatttggaacagtagcagggtttgtctctatggttccttatatgatgaaagatgttcaccagctaagtactgccgaaatcggaagtgtaattattttccctggaacaatgagtgtcattattttcggctacattggtgggatacttgttgatagaagaggtcctttatacgtgttaaacatcggagttacatttctttctgttagctttttaactgcttcctttcttttagaaacaacatcatggttcatgacaattataatcgtatttgttttaggtgggctttcgttcaccaaaacagttatatcaacaattgtttcaagtagcttgaaacagcaggaagctggtgctggaatgagtttgcttaactttaccagctttttatcagagggaacaggtattgcaattgtaggtggtttattatccatacccttacttgatcaaaggttgttacctatggaagttgatcagtcaacttatctgtatagtaatttgttattacttttttcaggaatcattgtcattagttggctggttaccttgaatgtatataaacattctcaaagggatttctaaatcgttaagggatcaactttgggagagagttcaaaattgatcctttttttataacaggaattgggcatcaaataaaacgaaaggctcagtcgaaagactgggcctttcgttttatctgttgtttgtcggtgaacgctctcctgagtaggacaaatccgccgggagcggatttgaacgttgcgaagcaacggcccggagggtggcgggcaggacgcccgccataaactgccaggcatcaaattaagcagaaggccatcctgacggatggcctttttgcgtttctacaaactcttcctgtcgtcatatctacaattctacacagcccagtccagactattcggcactgaaattatgggtgaagtggtcaagacctcactaggcaccttaaaaatagcgcaccctgaagaagatttatttgaggtagcccttgcctacctagcttccaagaaagatatcctaacagcacaagagcggaaagatgttttgttctacatccagaacaacctctgctaaaattcctgaaaaattttgcaaaaagttgttgactttatctacaaggtgtggcataatgtgtggaattgtgagcggataacaattaagctaattctatggtaaaagcattcctgaacccaatatccttatttttagtggacaaggccttgttctcatatggttgcttgagccagtgccttacaaggctcttccgctttggcaggctgttcaaaattatttattagagcaactcaaggaactaggcggagatccaaaagcaaccgatgcagcacgtgtttttcggattgctgggagcgtcaatagtaagaatggagcggaagtaagagcggaatatcggcacgattacagatatgagttaaggcagattcaatttgattaccttccagaactcaatgaggttattaatcccgctccacaaaagaaaaaacgggggcgtaaaaagaaagtagttcagttattcaatacctacaaactccattacgctcgcctattggatatagtgaaattggtggaactacgaaattatgaggtaactggatacagggaaatcatttgctttttataccgttattggttgtgctgttacacgaacgaccctgtagaggctttaaatcaaacacagacacttaatttacagttcactgagcctttacccttaaaagaggttgaaagggctacacggagcgcagaaaaggcgtgggaagcacgaaataacgaagaggctaaccggattgcaatcgaaaaaggatatcccagtgctggatacaatattagcaataaaaagttgattgaatggctagatatcacaccagaagaacagaagcatttacagacgattatagacgctaatgagaaacggagaagaaagcgggaaagggataggatttatcaagaacaaaaacgtcgtgagcggggagatatgacccgacaggagtatattaagcaacaacaggataaaacagatgataaattatttaaattgcaggagttattagaacagaatcccaaaatctcaaaaattaaattagcaaaaatacttggtgtagataaatcgcacttatacagactgctgaaacaactataactggaaaaaattagtgtctcatggttcgtcgcccttatattatgggcgttagcctgcttgctaattggataggtgttattgtcatttcaacgtcggacgttttggtagatgaacgtcggacgttatttgcttcaatagattgttgatgtattaagggttgcagtgaatcgacaagcaaaaagttatgacgttgtgaaaaaattgaatagaaaattggaaattacgtcggacgttctaacttaaaaaccctgttatatcaatgatttaaaaggaaattaacgtcataaaagacctttctgcaacaaaagtttttctggaagagttgaggttattttataggtattatggacttttgtagactttttgtgtactttttgtggactccacactcgctggtatcgtgttattttttaattgagatatgaatatggaaattaaacgttttaggcgttggtttggtgatgacaaaaaaataagagtacccgctcacaacggatactctttcgagaaatgtacgaaacgctataaataaaaaataactagatacatttacattgtatcacgtttcgtacatttctccaataacaaattgattggaggaatgcaaagtgaataatgaaccagtaaaacgtggtaagaagaacagatgggaattaaacctacctataatgacttatgtagtagctgatgattggattgataaactaggacacgaaacgtttactttatggttgaggttccatacttgggtagatagagaagatgaactccgagattatgatcgcatacctagaagttttgagaacatatataaaaagacactaggaatctcaaaaagtaagttttatagattgataaaacctttatgggaatatggattaatagacatcatagaatacgaagaatctaaccgtaattctactaaacctaaaaatataattgtttatgagtatcctttacacgaaatagaaagaaagtataaaccactagaaaaattaagagattgggataaagactataattccgtttctaaagaattaggtaaaacaggtggtagaccaaggaaaaaagatagtgaagaagaacccgaaaagaaacccgaagaagtaactaaaaagaaacgtaaatataagttaaaaagagttatccacaacggtttcaaaaatgaaacggtggagggtttcaaaaatgaaacggtggagggtttcaaaaatgaaacggtgaccgtttcaaaaataaaacccaataattattcaaatatctttaataacttatcaaatatttctactaatgtttcaaataatttattaattgatgatgatgaggaaatcgaaaatgaaccaactggtcgtacaataaataggtcattacttttttcacaagaagatattaaacaggcctatcaatttattaatagattttcagttatacagttacgtgaaaactttagctttgataaacactttgaagaacggttggtatgttatttatggaaagcagggatttctactttttacacgcacgaaatcagtaaaatgataaaaaaaatagcagactatgaaaaatctaaaaaaggtagattaaacccaatacgtgaccgagccttatatatggtaaatggtcttgtaatgaatagagcttcttcccaaagtgaacatgctacttataaactaaaccaatataaaaaacagaaggaacaggaaaaacaacaacaggagcaacaaagatcaagagtaccgttctataattggttggaggaaagagaagaacaaaccgaaggtcaactacccaccacttaaagcctaacggcttttgaagtggggcttgtaaaaagccctagttgactaccccaagtctttcgaggactacgttggaaaggtcatgacacctacaaatgctcctctagttcgtagccactgtcgttgatggttaaaagtcctgatgggtagggacggtgctgtcaacatcacaagcccttccaacatgggggaagaggaagaacactccgagaaaggagggggctgtcgtacacgccttgttcgtgtacgtgatttttaacacttttatctctaatataatctctccttgagttagcagagactaagaataaaacacattaggattttttatctacataaggaggttcaatacatgcctactatttcgtttaagggaaagtcttttgtacaaaatcatcacttgactgtaaaatatcatgaattgatcccagaaccagaaaaaagtctgaccgataaagttagtcttcatgacaatcttatcattcatggggacaatttaaaggcgttgaaagctctactacctacatatgctggtaagatagattgcatctatattgacccaccatacaatactggaactgaaaaatggatttataatgataatgtcaactccccaatgattagggaatggcttggaaaagtggtagacaaagaagacttatcccgacatgataagtggctttgtatgatgatgccgaggttaaaactgttgaaagagttgttgtcagaagacggagtgatatttgtaagcattgactacaatgaaatacaccatcttacgtgccttatgaacgaaatattcggtgaggagaattttcgtgacgctattatcattcgtagaggagtaaaaaatgttcaagcgcaatttgacacaattgattctctttcaaatggttatgagtctattttggtttacactaaacagccatctcgacgatttaataaggtttatgaagatgtagaagaaaagcctggtagttggaataatcattggagaggtacagaccgtaaaactatgagatatgaattatttggggttactccgacagaaggtcaatggagatgggggaaagaacgtagtctccaggctattgaaaactatcaaatgatgttagatgaacttagacaaaaaggcattactaatccaactcaagaggatattgataaatggtatcttgaatatgtagaaaataatggggaagatattgacttgttacgacaaaatgataatggcacgattgagcactttgttccaccgactagcaaaaagttgttaagtaatgcctggtttgacttaaaacccaacggttctagtcaattaaagaagatatttggaaggaaggttttcgataaccctaaatcaattgatttggtaaaaagactaatacaatttgcgactgaaaacaaagaagcgattgtacttgactcatttgcagggagtggcactactgctcatgcagtattatcgcttaacaaacaagatggagggaatcgtcgtttcatccttattgagatggaagaatatgcacatgagattaccgcagaacgcggatctttatcgatttgcatgcaagctaattcggtggaaacgaggtcatcatttccttccgaaaaaacggttgcatttaaatcttacatatgtaatactttcaaagactacatttgtaagatttgatgtttgagtcggctgaaagatcgtacgtaccaattattgtttcgtgattgttcaagccataacactgtagggatagtggaaagagtgcttcatctggttacgatcaatcaaatattcaaacggagggagacgattttgatgaaaccagtaacgttatacgatgtcgcagagtatgccggtgtctcttatcagaccgtttcccgcgtggtgaaccaggccagccacgtttctgcgaaaacgcgggaaaaagtggaagcggcgatggcggagctgaattacattcccaaccgcgtggcacaacaactggcgggcaaacagtcgttgctgattggcgttgccacctccagtctggccctgcacgcgccgtcgcaaattgtcgcggcgattaaatctcgcgccgatcaactgggtgccagcgtggtggtgtcgatggtagaacgaagcggcgtcgaagcctgtaaaacggcggtgcacaatcttctcgcgcaacgcgtcagtgggctgatcattaactatccgctggatgaccaggatgccattgctgtggaagctgcctgcactaatgttccggcgttatttcttgatgtctctgaccagacacccatcaacagtattattttctcccatgaagacggtacgcgactgggcgtggagcatctggtcgcattgggtcaccagcaaatcgcgctgttagcgggcccattaagttctgtctcggcgcgtctgcgtctggctggctggcataaatatctcactcgcaatcaaattcagccgatagcggaacgggaaggcgactggagtgccatgtccggttttcaacaaaccatgcaaatgctgaatgagggcatcgttcccactgcgatgctggttgccaacgatcagatggcgctgggcgcaatgcgcgccattaccgagtccgggctgcgcgttggtgcggatatctcggtagtgggatacgacgataccgaagacagctcatgttatatcccgccgttaaccaccatcaaacaggattttcgcctgctggggcaaaccagcgtggaccgcttgctgcaactctctcagggccaggcggtgaagggcaatcagctgttgcccgtctcactggtgaaaagaaaaaccaccctggcgcccaatacgcaaaccgcctctccccgcgcgttggccgattcattaatgcagctggcacgacaggtttcccgactggaaagcgggcagtgagcgcaacgcaattaatgtgagttaggatcctgcctcgcgcgtttcggtgatgacggtgaaaacctctgacacatgcagctcccggagacggtcacagcttgtctgtaagcggatgccgggagcagacaagcccgtcagggcgcgtcagcgggtgttggcgggtgtcggggcgcagccatgacccagtcacgtagcgatagcggagtgtatactggcttaactatgcggcatcagagcagattgtactgagagtgcaccatatgcggtgtgaaataccgcacagatgcgtaaggagaaaataccgcatcaggcgctcttccgcttcctcgctcactgactcgctgcgctcggtcgttcggctgcggcgagcggtatcagctcactcaaaggcggtaatacggttatccacagaatcaggggataacgcaggaaagaacatgtgagcaaaaggccagcaaaaggccaggaaccgtaaaaaggccgcgttgctggcgtttttccataggctccgcccccctgacgagcatcacaaaaatcgacgctcaagtcagaggtggcgaaacccgacaggactataaagataccaggcgtttccccctggaagctccctcgtgcgctctcctgttccgaccctgccgcttaccggatacctgtccgcctttctcccttcgggaagcgtggcgctttctcatagctcacgctgtaggtatctcagttcggtgtaggtcgttcgctccaagctgggctgtgtgcacgaaccccccgttcagcccgaccgctgcgccttatccggtaactatcgtcttgagtccaacccggtaagacacgacttatcgccactggcagcagccactggtaacaggattagcagagcgaggtatgtaggcggtgctacagagttcttgaagtggtggcctaactacggctacactagaaggacagtatttggtatctgcgctctgctgaagccagttaccttcggaaaaagagttggtagctcttgatccggcaaacaaaccaccgctggtagcggtggtttttttgtttgcaagcagcagattacgcgcagaaaaaaaggatctcaagaagatcctttgatcttttctacggggtctgacgctcagtggaacgaaaactcacgttaagggattttggtcatgagattatcaaaaaggatcttcacctagatccttttaaattaaaaatgaagttttaaatcaatctaaagtatatatgagtaaacttggtctgacagttaccaatgcttaatcagtgaggcacctatctcagcgatctgtctatttcgttcatccatagttgcctgactccccgtcgtgtagataactacgatacgggagggcttaccatctggccccagtgctgcaatgataccgcgagacccacgctcaccggctccagatttatcagcaataaaccagccagccggaagggccgagcgcagaagtggtcctgcaactttatccgcctccatccagtctattaattgttgccgggaagctagagtaagtagttcgccagttaatagtttgcgcaacgttgttgccattgctgcaggcatcgtggtgtcacgctcgtcgtttggtatggcttcattcagctccggttcccaacgatcaaggcgagttacatgatcccccatgttgtgcaaaaaagcggttagctccttcggtcctccgatcgttgtcagaagtaagttggccgcagtgttatcactcatggttatggcagcactgcataattctcttactgtcatgccatccgtaagatgcttttctgtgactggtgagtactcaaccaagtcattctgagaatagtgtatgcggcgaccgagttgctcttgcccggcgtcaacacgggataataccgcgccacatagcagaactttaaaagtgctcatcattggaaaacgttcttcggggcgaaaactctcaaggatcttaccgctgttgagatccagttcgatgtaacccactcgtgcacccaactgatcttcagcatcttttactttcaccagcgtttctgggtgagcaaaaacaggaaggcaaaatgccgcaaaaaagggaataagggcgacacggaaatgttgaatactcatactcttcctttttcaatattattgaagcatttatcagggttattgtctcatgagcggatacatatttgaatgtatttagaaaaataaacaaataggggttccgcgcacatttccccgaaaagtgccacctgacgtctaagaaaccattattatcatgacattaacctataaaaataggcgtatcacgaggccctttcgtcttcaagaattctcatgtttgacagcttatcatcgataagctcac

SEQ ID NO: 44 - protein, 6 aa, synthetic construct
  REGION 1..6: note = A1 core motif sequence
  SITE 2: note = misc_feature - Xaa can be Thr or Ser
  SITE 4: note = misc_feature - Xaa can be any of naturally occurring amino acid
LXYXEL

SEQ ID NO: 45 - protein, 12 aa, synthetic construct
  REGION 1..12: note = A2 core motif sequence
  SITE 5: note = misc_feature - Xaa can be any of naturally occurring amino acid
  SITE 9: note = misc_feature - Xaa can be Val or Leu
  SITE 11: note = misc_feature - Xaa can be Leu or Ile
LKAGXAYLXPXD

SEQ ID NO: 46 - protein, 16 aa, synthetic construct
  REGION 1..16: note = A3 core motif sequence
  SITE 4: note = misc_feature - Xaa can be any of naturally occurring amino acid
  SITE 5: note = misc_feature - Xaa can be any of naturally occurring amino acid
  SITE 10: note = misc_feature - Xaa can be Val or Leu
  SITE 13: note = misc_feature - Xaa can be any of naturally occurring amino acid
LAYXXYTSGXTGXPKG

SEQ ID NO: 47 - protein, 7 aa, synthetic construct
  REGION 1..7: note = A5 core motif sequence
  SITE 2: note = misc_feature - Xaa can be any of naturally occurring amino acid
NXYGPTE

SEQ ID NO: 48 - protein, 15 aa, synthetic construct
  REGION 1..15: note = A6 core motif sequence
  SITE 4: note = misc_feature - Xaa can be any of naturally occurring amino acid
  SITE 6: note = misc_feature - Xaa can be any of naturally occurring amino acid
  SITE 8: note = misc_feature - Xaa can be any of naturally occurring amino acid
  SITE 10: note = misc_feature - Xaa can be Val or Leu
GELXIXGXGXARGYL

SEQ ID NO: 49 - protein, 6 aa, synthetic construct
  REGION 1..6: note = A7 core motif sequence
  SITE 2: note = misc_feature - Xaa can be Arg or Lys
YXTGDL

SEQ ID NO: 50 - protein, 20 aa, synthetic construct
  REGION 1..20: note = A8 core motif sequence
  SITE 3: note = misc_feature - Xaa can be any of naturally occurring amino acid
  SITE 5: note = misc_feature - Xaa can be any of naturally occurring amino acid
  SITE 12: note = misc_feature - Xaa can be any of naturally occurring amino acid
GRXDXQVKIRGXRIELGEIE

SEQ ID NO: 51 - protein, 7 aa, synthetic construct
  REGION 1..7: note = A9 core motif sequence
  SITE 3: note = misc_feature - Xaa can be any of naturally occurring amino acid
  SITE 6: note = misc_feature - Xaa can be Ile or Val
LPXYMXP

SEQ ID NO: 52 - protein, 6 aa, synthetic construct
  REGION 1..6: note = A10 core motif sequence
  SITE 4: note = misc_feature - Xaa can be Val or Leu
NGKXDR

SEQ ID NO: 53 - protein, 12 aa, synthetic construct
  REGION 1..12: note = T core motif sequence
  SITE 2: note = misc_feature - Xaa can be any of naturally occurring amino acid
  SITE 5: note = misc_feature - Xaa can be any of naturally occurring amino acid
  SITE 6: note = misc_feature - Xaa can be any of naturally occurring amino acid
  SITE 10: note = misc_feature - Xaa can be His or Asp
  SITE 12: note = misc_feature - Xaa can be Leu or Ile
DXFFXXLGGXSX

SEQ ID NO: 54 - protein, 10 aa, synthetic construct
  REGION 1..10: note = C1 core motif sequence
  SITE 2: note = misc_feature - Xaa can be any of naturally occurring amino acid
  SITE 5: note = misc_feature - Xaa can be any of naturally occurring amino acid
  SITE 7: note = misc_feature - Xaa can be Leu or Met
  SITE 8: note = misc_feature - Xaa can be Trp or Tyr
  SITE 9: note = misc_feature - Xaa can be any of naturally occurring amino acid
SXAQXRXXXL

SEQ ID NO: 55 - protein, 9 aa, synthetic construct
  REGION 1..9: note = C2 core motif sequence
  SITE 4: note = misc_feature - Xaa can be any of naturally occurring amino acid
  SITE 8: note = misc_feature - Xaa can be any of naturally occurring amino acid
RHEXLRTXF

SEQ ID NO: 56 - protein, 10 aa, synthetic construct
  REGION 1..10: note = C3 core motif sequence
  SITE 4: note = misc_feature - Xaa can be any of naturally occurring amino acid
  SITE 9: note = misc_feature - Xaa can be Trp or Val
MHHXISDGXS

SEQ ID NO: 57 - protein, 7 aa, synthetic construct
  REGION 1..7: note = C4 core motif sequence
  SITE 2: note = misc_feature - Xaa can be any of naturally occurring amino acid
  SITE 4: note = misc_feature - Xaa can be Phe or Tyr
YXDXAVW

SEQ ID NO: 58 - protein, 11 aa, synthetic construct
  REGION 1..11: note = C5 core motif sequence
  SITE 1: note = misc_feature - Xaa can be Ile or Val
  SITE 3: note = misc_feature - Xaa can be any of naturally occurring amino acid
  SITE 8: note = misc_feature - Xaa can be Gln or Leu
  SITE 9: note = misc_feature - Xaa can be Cys or Ala
  SITE 10: note = misc_feature - Xaa can be any of naturally occurring amino acid
XGXFVNTXXXR

SEQ ID NO: 59 - protein, 7 aa, synthetic construct
  REGION 1..7: note = C6 core motif sequence
  SITE 1: note = misc_feature - Xaa can be His or Asn
  SITE 4: note = misc_feature - Xaa can be Tyr Val
XQDXPFE

SEQ ID NO: 60 - protein, 8 aa, synthetic construct
  REGION 1..8: note = C7 core motif sequence
  SITE 3: note = misc_feature - Xaa can be any of naturally occurring amino acid
RDXSRNPL

SEQ ID NO: 61 - protein, 7 aa, synthetic construct
  REGION 1..7: note = mutant sequence
  LIPID 1: note = N-beta-hydroxyl aliphatic acyl
ELLVQYI

SEQ ID NO: 62 - protein, 7 aa, synthetic construct
  REGION 1..7: note = mutant sequence
  LIPID 1: note = N-beta-hydroxyl aliphatic acyl
ELLVDYI

SEQ ID NO: 63 - protein, 10 aa, synthetic construct
  REGION 1..10: note = mutant sequence
  LIPID 1: note = N-beta-hydroxyl aliphatic acyl
  MOD_RES 2: note = Orn
EXYTEVVQYI

SEQ ID NO: 64 - protein, 10 aa, synthetic construct
  REGION 1..10: note = mutant sequence
  LIPID 1: note = N-beta-hydroxyl aliphatic acyl
  MOD_RES 2: note = Orn
EXYTEVPDYI

SEQ ID NO: 65 - protein, 10 aa, synthetic construct
  REGION 1..10: note = mutant sequence
  LIPID 1: note = N-beta-hydroxyl aliphatic acyl
  MOD_RES 2: note = Orn
EXYTEVVDYI